European Patent Application EP 4 556 561 A1, published May 21, 2025. Title: Expression of biomolecules with improved promoter and TIR. Applicant: CysBio ApS. Application EP. The sequence listing filed with the application follows.

SEQUENCE LISTING (176 sequences)

SEQ ID NO: 1 - DNA, 35 bp, synthetic construct
  source 1..35: mol_type = other DNA
ttgacagctagctcagtcctaggtactgtgctagc

SEQ ID NO: 2 - DNA, 35 bp, synthetic construct
  source 1..35: mol_type = other DNA
ttgacagctagctcagtcctaggtattgtgctagc

SEQ ID NO: 3 - DNA, 35 bp, synthetic construct
  source 1..35: mol_type = other DNA
tttacggctagctcagtcctaggtatagtgctagc

SEQ ID NO: 4 - DNA, 35 bp, synthetic construct
  source 1..35: mol_type = other DNA
tttacggctagctcagccctaggtattatgctagc

SEQ ID NO: 5 - DNA, 35 bp, synthetic construct
  source 1..35: mol_type = other DNA
ctgacagctagctcagtcctaggtataatgctagc

SEQ ID NO: 6 - DNA, 35 bp, synthetic construct
  source 1..35: mol_type = other DNA
tttatagctagctcagcccttggtacaatgctagc

SEQ ID NO: 7 - DNA, 35 bp, synthetic construct
  source 1..35: mol_type = other DNA
ttgacagctagctcagtcctagggactatgctagc

SEQ ID NO: 8 - DNA, 35 bp, synthetic construct
  source 1..35: mol_type = other DNA
ttgacagctagctcagtcctaggtataatgctagc

SEQ ID NO: 9 - DNA, 47 bp, synthetic construct
  source 1..47: mol_type = other DNA
aaaaagagtattgacttaaagtctaacctataggtataatgtgtgga

SEQ ID NO: 10 - DNA, 36 bp, synthetic construct
  source 1..36: mol_type = other DNA
ttgacaattaatcatccggctcttagtgtttgtgga

SEQ ID NO: 11 - DNA, 36 bp, synthetic construct
  source 1..36: mol_type = other DNA
ttgacaattaatcatccggctcgtataatgtgtgga

SEQ ID NO: 12 - DNA, 46 bp, synthetic construct
  source 1..46: mol_type = other DNA
aaaaagagtattgacttcgcatctttttgtacctataatgtgtgga

SEQ ID NO: 13 - DNA, 36 bp, synthetic construct
  source 1..36: mol_type = other DNA
ttgacaattaatcatccggctcgtaatttatgtgga

SEQ ID NO: 14 - DNA, 36 bp, synthetic construct
  source 1..36: mol_type = other DNA
ttgacaattaatcatccggctcgtaatgtttgtgga

SEQ ID NO: 15 - DNA, 47 bp, synthetic construct
  source 1..47: mol_type = other DNA
aaaaaatttatttgctttcgcatctttttgtacctataatgtgtgga

SEQ ID NO: 16 - DNA, 35 bp, synthetic construct
  source 1..35: mol_type = other DNA
ttgcctcttaatcatcggctcgtataatgtgtgga

SEQ ID NO: 17 - DNA, 6799 bp, synthetic construct
  source 1..6799: mol_type = other DNA
gctgaggtcgcctcagcggccggcccctgcaggcgccggcgactagtcttggactcctgttgatagatccagtaatgacctcagaactccatctggatttgttcagaacgctcggttgccgccgggcgttttttattggtgagaatccaggggtccccaataattacgatttaaatttgtgtctcaaaatctctgatgttacattgcacaagataaaaatatatcatcatgaacaataaaactgtctgcttacataaacagtaatacaaggggtgttatgagccatattcagcgtgaaacgagctgtagccgtccgcgtctgaacagcaacatggatgcggatctgtatggctataaatgggcgcgtgataacgtgggtcagagcggcgcgaccatttatcgtctgtatggcaaaccggatgcgccggaactgtttctgaaacatggcaaaggcagcgtggcgaacgatgtgaccgatgaaatggtgcgtctgaactggctgaccgaatttatgccgctgccgaccattaaacattttattcgcaccccggatgatgcgtggctgctgaccaccgcgattccgggcaaaaccgcgtttcaggtgctggaagaatatccggatagcggcgaaaacattgtggatgcgctggccgtgtttctgcgtcgtctgcatagcattccggtgtgcaactgcccgtttaacagcgatcgtgtgtttcgtctggcccaggcgcagagccgtatgaacaacggcctggtggatgcgagcgattttgatgatgaacgtaacggctggccggtggaacaggtgtggaaagaaatgcataaactgctgccgtttagcccggatagcgtggtgacccacggcgattttagcctggataacctgattttcgatgaaggcaaactgattggctgcattgatgtgggccgtgtgggcattgcggatcgttatcaggatctggccattctgtggaactgcctgggcgaatttagcccgagcctgcaaaaacgtctgtttcagaaatatggcattgataatccggatatgaacaaactgcaatttcatctgatgctggatgaatttttctaataattaattggaccgttgtccttttccgctgcataaccctgcttcggggtcattatagcgattttttcggtatatccatcctttttcgcacgatatacaggattttgccaaagggttcgtgtagactttccttggtgtatccaacggcgtcagccgggcaggataggtgaagtaggcccacccgcgagcgggtgttccttcttcactgtcccttattcgcacctggcggtgctcaacgggaatcctgctctgcgaggctggccgtaggccggcctcagatccttccgtatttagccagtatgttctctagtgtggttcgttgtttttgcgtgagccatgagaacgaaccattgagatcatacttactttgcatgtcactcaaaaattttgcctcaaaactggtgagctgaatttttgcagttaaagcatcgtgtagtgtttttcttagtccgttatgtaggtaggaatctgatgtaatggttgttggtattttgtcaccattcatttttatctggttgttctcaagttcggttacgagatccatttgtctatctagttcaacttggaaaatcaacgtatcagtcgggcggcctcgcttatcaaccaccaatttcatattgctgtaagtgtttaaatctttacttattggtttcaaaacccattggttaagccttttaaactcatggtagttattttcaagcattaacatgaacttaaattcatcaaggctaatctctatatttgccttgtgagttttcttttgtgttagttcttttaataaccactcataaatcctcatagagtatttgttttcaaaagacttaacatgttccagattatattttatgaatttttttaactggaaaagataaggcaatatctcttcactaaaaactaattctaatttttcgcttgagaacttggcatagtttgtccactggaaaatctcaaagcctttaaccaaaggattcctgatttccacagttctcgtcatcagctctctggttgctttagctaatacaccataagcattttccctactgatgttcatcatctgagcgtattggttataagtgaacgataccgtccgttctttccttgtagggttttcaatcgtggggttgagtagtgccacacagcataaaattagcttggtttcatgctccgttaagtcatagcgactaatcgctagttcatttgctttgaaaacaactaattcagacatacatctcaattggtctaggtgattttaatcactataccaattgagatgggctagtcaatgataattacatgtccttttcctttgagttgtgggtatctgtaaattctgctagacctttgctggaaaacttgtaaattctgctagaccctctgtaaattccgctagacctttgtgtgttttttttgtttatattcaagtggttataatttatagaataaagaaagaataaaaaaagataaaaagaatagatcccagccctgtgtataactcactactttagtcagttccgcagtattacaaaaggatgtcgcaaacgctgtttgctcctctacaaaacagaccttaaaaccctaaaggcttaagtagcaccctcgcaagctcgggcaaatcgctgaatattccttttgtctccgaccatcaggcacctgagtcgctgtctttttcgtgacattcagttcgctgcgctcacggctctggcagtgaatgggggtaaatggcactacaggcgcggcgcgcccagctgtctagggcggcggatttgtcctactcaggagagcgttcaccgacaaacaacagataaaacgaaaggcccagtctttcgactgagcctttcgttttatttgatgcctttaattaagcggccgcggcgcgcccgtcgacgcgcgcgcggctgaggatacctcagctaatacgactcactataggggaattgtgagcggataacaattcccctctagaataattttgtttaactttaagaaggagaccagtttatgagccagaatggccgtccggtagtcctcatcgccgataagcttgcgcagtccactgttgacgcgcttggagatgcagtagaagtccgttgggttgacggacctaaccgcccagaactgcttgatgcagttaaggaagcggacgcactgctcgtgcgttctgctaccactgtcgatgctgaagtcatcgccgctgcccctaacttgaagatcgtcggtcgtgccggcgtgggcttggacaacgttgacatccctgctgccactgaagctggcgtcatggttgctaacgcaccgacctctaatattcactccgcttgtgagcacgcaatttctttgctgctgtctactgctcgccagatccctgctgctgatgcgacgctgcgtgagggcgagtggaagcggtcttctttcaacggtgtggaaattttcggaaaaactgtcggtatcgtcggttttggccacattggtcagttgtttgctcagcgtcttgctgcgtttgagaccaccattgttgcttacgatccttacgctaaccctgctcgtgcggctcagctgaacgttgagttggttgagttggatgagctgatgagccgttctgactttgtcaccattcaccttcctaagaccaaggaaactgctggcatgtttgatgcgcagctccttgctaagtccaagaagggccagatcatcatcaacgctgctcgtggtggccttgttgatgagcaggctttggctgatgcgattgagtccggtcacattcgtggcgctggtttcgatgtgtactccaccgagccttgcactgattctcctttgttcaagttgcctcaggttgttgtgactcctcacttgggtgggtctactgaagaggctcaggatcgtgcgggtactgacgttgctgattctgtgctcaaggcgctggctggcgagttcgtggcggatgctgtgaacgtttccggtggtcgcgtgggcgaagaggttgctgtgtggatggatctggctcgcaagcttggtcttcttgctggcaagcttgtcgacgccgccccagtctccattgaggttgaggctcgaggcgagctttcttccgagcaggtcgatgcacttggtttgtccgctgttcgtggtttgttctccggaattatcgaagagtccgttactttcgtcaacgctcctcgcattgctgaagagcgtggcctggacatctccgtgaagaccaactctgagtctgttactcaccgttccgtcctgcaggtcaaggtcattactggcagcggcgcgagcgcaactgttgttggtgccctgactggtcttgagcgcgttgagaagatcacccgcatcaatggccgtggcctggatctgcgcgcagagggtctgaacctcttcctgcaggccactgacgctcctggtgcactgggtaccgttggtaccaagctgggtgctgctggcatcaacatcgaggctgctgcgttgactcaggctgagaagggtgacggcgctgtcctgatcctgcgtgttgagtccgctgtctctgaagagctggaagctgaaatcaacgctgagttgggtgctacttccttccaggttgatcttgactaataaagcttggttgataaaagaaggagaccagtttatggctcaaatcttcaattttagttctggtccggcaatgctaccggcagaggtgcttaaacaggctcaacaggaactgcgcgactggaacggtcttggtacgtcggtgatggaagtgagtcaccgtggcaaagagttcattcaggttgcagaggaagccgagaaggattttcgcgatcttcttaatgtcccctccaactacaaggtattattctgccatggcggtggtcgcggtcagtttgctgcggtaccgctgaatattctcggtgataaaaccaccgcagattatgttgatgccggttactgggcggcaagtgccattaaagaagcgaaaaaatactgcacgcctaatgtctttgacgccaaagtgactgttgatggtctgcgcgcggttaagccaatgcgtgaatggcaactctctgataatgctgcttatatgcattattgcccgaatgaaaccatcgatggtatcgccatcgacgaaacgccagacttcggcgcagatgtggtggtcgccgctgacttctcttcaaccattctttcccgtccgattgacgtcagccgttatggtgtaatttacgctggcgcgcagaaaaatatcggcccggctggcctgacaatcgtcatcgttcgtgaagatttgctgggcaaagcgaatatcgcgtgtccgtcgattctggattattccatcctcaacgataacggctccatgtttaacacgccgccgacatttgcctggtatctatctggtctggtctttaaatggctgaaagcgaacggcggtgtagctgaaatggataaaatcaatcagcaaaaagcagaactgctatatggggtgattgataacagcgatttctaccgcaatgacgtggcgaaagctaaccgttcgcggatgaacgtgccgttccagttggcggacagtgcgcttgacaaattgttccttgaagagtcttttgctgctggccttcatgcactgaaaggtcaccgtgtggtcggcggaatgcgcgcttctatttataacgccatgccgctggaaggcgttaaagcgctgacagacttcatggttgagttcgaacgccgtcacggttgataaaagaaggagaccagtttatgcctaacattacctggtgcgacctgcctgaagatgtctctttatggccgggtctgcctctttcattaagtggtgatgaagtgatgccactggattaccacgcaggtcgtagcggctggctgctgtatggtcgtgggctggataaacaacgtctgacccaataccagagcaaactgggtgcggcgatggtgattgttgccgcctggtgcgtggaagattatcaggtgattcgtctggcaggttcactcaccgcacgggctacacgcctggcccacgaagcgcagctggatgtcgccccgctggggaaaatcccgcacctgcgcacgccgggtttgctggtgatggatatggactccaccgccatccagattgaatgtattgatgaaattgccaaactggccggaacgggcgagatggtggcggaagtaaccgaacgggcgatgcgcggcgaactcgattttaccgccagcctgcgcagccgtgtggcgacgctgaaaggcgctgacgccaatattctgcaacaggtgcgtgaaaatctgccgctgatgccaggcttaacgcaactggtgctcaagctggaaacgctgggctggaaagtggcgattgcctccggcggctttactttctttgctgaatacctgcgcgacaagctgcgcctgaccgccgtggtagccaatgaactggagatcatggacggtaaatttaccggcaatgtgatcggcgacatcgtagacgcgcagtacaaagcgaaaactctgactcgcctcgcgcaggagtatgaaatcccgctggcgcagaccgtggcgattggcgatggagccaatgacctgccgatgatcaaagcggcagggctggggattgcctaccatgccaagccaaaagtgaatgaaaaggcggaagtcaccatccgtcacgctgacctgatgggggtattctgcatcctctcaggcagcctgaatcagaagtgataa

SEQ ID NO: 18 - DNA, 6784 bp, synthetic construct
  source 1..6784: mol_type = other DNA
tattcgcacctggcggtgctcaacgggaatcctgctctgcgaggctggccgtaggccggcctcagatccttccgtatttagccagtatgttctctagtgtggttcgttgtttttgcgtgagccatgagaacgaaccattgagatcatacttactttgcatgtcactcaaaaattttgcctcaaaactggtgagctgaatttttgcagttaaagcatcgtgtagtgtttttcttagtccgttatgtaggtaggaatctgatgtaatggttgttggtattttgtcaccattcatttttatctggttgttctcaagttcggttacgagatccatttgtctatctagttcaacttggaaaatcaacgtatcagtcgggcggcctcgcttatcaaccaccaatttcatattgctgtaagtgtttaaatctttacttattggtttcaaaacccattggttaagccttttaaactcatggtagttattttcaagcattaacatgaacttaaattcatcaaggctaatctctatatttgccttgtgagttttcttttgtgttagttcttttaataaccactcataaatcctcatagagtatttgttttcaaaagacttaacatgttccagattatattttatgaatttttttaactggaaaagataaggcaatatctcttcactaaaaactaattctaatttttcgcttgagaacttggcatagtttgtccactggaaaatctcaaagcctttaaccaaaggattcctgatttccacagttctcgtcatcagctctctggttgctttagctaatacaccataagcattttccctactgatgttcatcatctgagcgtattggttataagtgaacgataccgtccgttctttccttgtagggttttcaatcgtggggttgagtagtgccacacagcataaaattagcttggtttcatgctccgttaagtcatagcgactaatcgctagttcatttgctttgaaaacaactaattcagacatacatctcaattggtctaggtgattttaatcactataccaattgagatgggctagtcaatgataattacatgtccttttcctttgagttgtgggtatctgtaaattctgctagacctttgctggaaaacttgtaaattctgctagaccctctgtaaattccgctagacctttgtgtgttttttttgtttatattcaagtggttataatttatagaataaagaaagaataaaaaaagataaaaagaatagatcccagccctgtgtataactcactactttagtcagttccgcagtattacaaaaggatgtcgcaaacgctgtttgctcctctacaaaacagaccttaaaaccctaaaggcttaagtagcaccctcgcaagctcgggcaaatcgctgaatattccttttgtctccgaccatcaggcacctgagtcgctgtctttttcgtgacattcagttcgctgcgctcacggctctggcagtgaatgggggtaaatggcactacaggcgcggcgcgcccagctgtctagggcggcggatttgtcctactcaggagagcgttcaccgacaaacaacagataaaacgaaaggcccagtctttcgactgagcctttcgttttatttgatgcctttaattaagcggccgcggcgcgcccgtcgacgcgcgcgcggctgaggatacctcagcataggcctttgacagctagctcagtcctaggtataatgctagctcttaatcatgctaaggaggattaactttatgagccagaatggccgtccggtagtcctcatcgccgataagcttgcgcagtccactgttgacgcgcttggagatgcagtagaagtccgttgggttgacggacctaaccgcccagaactgcttgatgcagttaaggaagcggacgcactgctcgtgcgttctgctaccactgtcgatgctgaagtcatcgccgctgcccctaacttgaagatcgtcggtcgtgccggcgtgggcttggacaacgttgacatccctgctgccactgaagctggcgtcatggttgctaacgcaccgacctctaatattcactccgcttgtgagcacgcaatttctttgctgctgtctactgctcgccagatccctgctgctgatgcgacgctgcgtgagggcgagtggaagcggtcttctttcaacggtgtggaaattttcggaaaaactgtcggtatcgtcggttttggccacattggtcagttgtttgctcagcgtcttgctgcgtttgagaccaccattgttgcttacgatccttacgctaaccctgctcgtgcggctcagctgaacgttgagttggttgagttggatgagctgatgagccgttctgactttgtcaccattcaccttcctaagaccaaggaaactgctggcatgtttgatgcgcagctccttgctaagtccaagaagggccagatcatcatcaacgctgctcgtggtggccttgttgatgagcaggctttggctgatgcgattgagtccggtcacattcgtggcgctggtttcgatgtgtactccaccgagccttgcactgattctcctttgttcaagttgcctcaggttgttgtgactcctcacttgggtgggtctactgaagaggctcaggatcgtgcgggtactgacgttgctgattctgtgctcaaggcgctggctggcgagttcgtggcggatgctgtgaacgtttccggtggtcgcgtgggcgaagaggttgctgtgtggatggatctggctcgcaagcttggtcttcttgctggcaagcttgtcgacgccgccccagtctccattgaggttgaggctcgaggcgagctttcttccgagcaggtcgatgcacttggtttgtccgctgttcgtggtttgttctccggaattatcgaagagtccgttactttcgtcaacgctcctcgcattgctgaagagcgtggcctggacatctccgtgaagaccaactctgagtctgttactcaccgttccgtcctgcaggtcaaggtcattactggcagcggcgcgagcgcaactgttgttggtgccctgactggtcttgagcgcgttgagaagatcacccgcatcaatggccgtggcctggatctgcgcgcagagggtctgaacctcttcctgcaggccactgacgctcctggtgcactgggtaccgttggtaccaagctgggtgctgctggcatcaacatcgaggctgctgcgttgactcaggctgagaagggtgacggcgctgtcctgatcctgcgtgttgagtccgctgtctctgaagagctggaagctgaaatcaacgctgagttgggtgctacttccttccaggttgatcttgactaataaagcttggttgataaaagaaggagaccagtttatggctcaaatcttcaattttagttctggtccggcaatgctaccggcagaggtgcttaaacaggctcaacaggaactgcgcgactggaacggtcttggtacgtcggtgatggaagtgagtcaccgtggcaaagagttcattcaggttgcagaggaagccgagaaggattttcgcgatcttcttaatgtcccctccaactacaaggtattattctgccatggcggtggtcgcggtcagtttgctgcggtaccgctgaatattctcggtgataaaaccaccgcagattatgttgatgccggttactgggcggcaagtgccattaaagaagcgaaaaaatactgcacgcctaatgtctttgacgccaaagtgactgttgatggtctgcgcgcggttaagccaatgcgtgaatggcaactctctgataatgctgcttatatgcattattgcccgaatgaaaccatcgatggtatcgccatcgacgaaacgccagacttcggcgcagatgtggtggtcgccgctgacttctcttcaaccattctttcccgtccgattgacgtcagccgttatggtgtaatttacgctggcgcgcagaaaaatatcggcccggctggcctgacaatcgtcatcgttcgtgaagatttgctgggcaaagcgaatatcgcgtgtccgtcgattctggattattccatcctcaacgataacggctccatgtttaacacgccgccgacatttgcctggtatctatctggtctggtctttaaatggctgaaagcgaacggcggtgtagctgaaatggataaaatcaatcagcaaaaagcagaactgctatatggggtgattgataacagcgatttctaccgcaatgacgtggcgaaagctaaccgttcgcggatgaacgtgccgttccagttggcggacagtgcgcttgacaaattgttccttgaagagtcttttgctgctggccttcatgcactgaaaggtcaccgtgtggtcggcggaatgcgcgcttctatttataacgccatgccgctggaaggcgttaaagcgctgacagacttcatggttgagttcgaacgccgtcacggttgataaaagaaggagaccagtttatgcctaacattacctggtgcgacctgcctgaagatgtctctttatggccgggtctgcctctttcattaagtggtgatgaagtgatgccactggattaccacgcaggtcgtagcggctggctgctgtatggtcgtgggctggataaacaacgtctgacccaataccagagcaaactgggtgcggcgatggtgattgttgccgcctggtgcgtggaagattatcaggtgattcgtctggcaggttcactcaccgcacgggctacacgcctggcccacgaagcgcagctggatgtcgccccgctggggaaaatcccgcacctgcgcacgccgggtttgctggtgatggatatggactccaccgccatccagattgaatgtattgatgaaattgccaaactggccggaacgggcgagatggtggcggaagtaaccgaacgggcgatgcgcggcgaactcgattttaccgccagcctgcgcagccgtgtggcgacgctgaaaggcgctgacgccaatattctgcaacaggtgcgtgaaaatctgccgctgatgccaggcttaacgcaactggtgctcaagctggaaacgctgggctggaaagtggcgattgcctccggcggctttactttctttgctgaatacctgcgcgacaagctgcgcctgaccgccgtggtagccaatgaactggagatcatggacggtaaatttaccggcaatgtgatcggcgacatcgtagacgcgcagtacaaagcgaaaactctgactcgcctcgcgcaggagtatgaaatcccgctggcgcagaccgtggcgattggcgatggagccaatgacctgccgatgatcaaagcggcagggctggggattgcctaccatgccaagccaaaagtgaatgaaaaggcggaagtcaccatccgtcacgctgacctgatgggggtattctgcatcctctcaggcagcctgaatcagaagtgataagctgaggtcgcctcagcggccggcccctgcaggcgccggcgactagtcttggactcctgttgatagatccagtaatgacctcagaactccatctggatttgttcagaacgctcggttgccgccgggcgttttttattggtgagaatccaggggtccccaataattacgatttaaatttgtgtctcaaaatctctgatgttacattgcacaagataaaaatatatcatcatgaacaataaaactgtctgcttacataaacagtaatacaaggggtgttatgagccatattcagcgtgaaacgagctgtagccgtccgcgtctgaacagcaacatggatgcggatctgtatggctataaatgggcgcgtgataacgtgggtcagagcggcgcgaccatttatcgtctgtatggcaaaccggatgcgccggaactgtttctgaaacatggcaaaggcagcgtggcgaacgatgtgaccgatgaaatggtgcgtctgaactggctgaccgaatttatgccgctgccgaccattaaacattttattcgcaccccggatgatgcgtggctgctgaccaccgcgattccgggcaaaaccgcgtttcaggtgctggaagaatatccggatagcggcgaaaacattgtggatgcgctggccgtgtttctgcgtcgtctgcatagcattccggtgtgcaactgcccgtttaacagcgatcgtgtgtttcgtctggcccaggcgcagagccgtatgaacaacggcctggtggatgcgagcgattttgatgatgaacgtaacggctggccggtggaacaggtgtggaaagaaatgcataaactgctgccgtttagcccggatagcgtggtgacccacggcgattttagcctggataacctgattttcgatgaaggcaaactgattggctgcattgatgtgggccgtgtgggcattgcggatcgttatcaggatctggccattctgtggaactgcctgggcgaatttagcccgagcctgcaaaaacgtctgtttcagaaatatggcattgataatccggatatgaacaaactgcaatttcatctgatgctggatgaatttttctaataattaattggaccgttgtccttttccgctgcataaccctgcttcggggtcattatagcgattttttcggtatatccatcctttttcgcacgatatacaggattttgccaaagggttcgtgtagactttccttggtgtatccaacggcgtcagccgggcaggataggtgaagtaggcccacccgcgagcgggtgttccttcttcactgtccct

SEQ ID NO: 19 - DNA, 6796 bp, synthetic construct
  source 1..6796: mol_type = other DNA
taaagcatcgtgtagtgtttttcttagtccgttatgtaggtaggaatctgatgtaatggttgttggtattttgtcaccattcatttttatctggttgttctcaagttcggttacgagatccatttgtctatctagttcaacttggaaaatcaacgtatcagtcgggcggcctcgcttatcaaccaccaatttcatattgctgtaagtgtttaaatctttacttattggtttcaaaacccattggttaagccttttaaactcatggtagttattttcaagcattaacatgaacttaaattcatcaaggctaatctctatatttgccttgtgagttttcttttgtgttagttcttttaataaccactcataaatcctcatagagtatttgttttcaaaagacttaacatgttccagattatattttatgaatttttttaactggaaaagataaggcaatatctcttcactaaaaactaattctaatttttcgcttgagaacttggcatagtttgtccactggaaaatctcaaagcctttaaccaaaggattcctgatttccacagttctcgtcatcagctctctggttgctttagctaatacaccataagcattttccctactgatgttcatcatctgagcgtattggttataagtgaacgataccgtccgttctttccttgtagggttttcaatcgtggggttgagtagtgccacacagcataaaattagcttggtttcatgctccgttaagtcatagcgactaatcgctagttcatttgctttgaaaacaactaattcagacatacatctcaattggtctaggtgattttaatcactataccaattgagatgggctagtcaatgataattacatgtccttttcctttgagttgtgggtatctgtaaattctgctagacctttgctggaaaacttgtaaattctgctagaccctctgtaaattccgctagacctttgtgtgttttttttgtttatattcaagtggttataatttatagaataaagaaagaataaaaaaagataaaaagaatagatcccagccctgtgtataactcactactttagtcagttccgcagtattacaaaaggatgtcgcaaacgctgtttgctcctctacaaaacagaccttaaaaccctaaaggcttaagtagcaccctcgcaagctcgggcaaatcgctgaatattccttttgtctccgaccatcaggcacctgagtcgctgtctttttcgtgacattcagttcgctgcgctcacggctctggcagtgaatgggggtaaatggcactacaggcgcggcgcgcccagctgtctagggcggcggatttgtcctactcaggagagcgttcaccgacaaacaacagataaaacgaaaggcccagtctttcgactgagcctttcgttttatttgatgcctttaattaagcggccgcggcgcgcccgtcgacgcgcgcgcggctgaggatacctcagcataggcctaaaaagagtattgacttaaagtctaacctataggtataatgtgtggatcttaatcatgctaaggaggattaactttatgagccagaatggccgtccggtagtcctcatcgccgataagcttgcgcagtccactgttgacgcgcttggagatgcagtagaagtccgttgggttgacggacctaaccgcccagaactgcttgatgcagttaaggaagcggacgcactgctcgtgcgttctgctaccactgtcgatgctgaagtcatcgccgctgcccctaacttgaagatcgtcggtcgtgccggcgtgggcttggacaacgttgacatccctgctgccactgaagctggcgtcatggttgctaacgcaccgacctctaatattcactccgcttgtgagcacgcaatttctttgctgctgtctactgctcgccagatccctgctgctgatgcgacgctgcgtgagggcgagtggaagcggtcttctttcaacggtgtggaaattttcggaaaaactgtcggtatcgtcggttttggccacattggtcagttgtttgctcagcgtcttgctgcgtttgagaccaccattgttgcttacgatccttacgctaaccctgctcgtgcggctcagctgaacgttgagttggttgagttggatgagctgatgagccgttctgactttgtcaccattcaccttcctaagaccaaggaaactgctggcatgtttgatgcgcagctccttgctaagtccaagaagggccagatcatcatcaacgctgctcgtggtggccttgttgatgagcaggctttggctgatgcgattgagtccggtcacattcgtggcgctggtttcgatgtgtactccaccgagccttgcactgattctcctttgttcaagttgcctcaggttgttgtgactcctcacttgggtgggtctactgaagaggctcaggatcgtgcgggtactgacgttgctgattctgtgctcaaggcgctggctggcgagttcgtggcggatgctgtgaacgtttccggtggtcgcgtgggcgaagaggttgctgtgtggatggatctggctcgcaagcttggtcttcttgctggcaagcttgtcgacgccgccccagtctccattgaggttgaggctcgaggcgagctttcttccgagcaggtcgatgcacttggtttgtccgctgttcgtggtttgttctccggaattatcgaagagtccgttactttcgtcaacgctcctcgcattgctgaagagcgtggcctggacatctccgtgaagaccaactctgagtctgttactcaccgttccgtcctgcaggtcaaggtcattactggcagcggcgcgagcgcaactgttgttggtgccctgactggtcttgagcgcgttgagaagatcacccgcatcaatggccgtggcctggatctgcgcgcagagggtctgaacctcttcctgcaggccactgacgctcctggtgcactgggtaccgttggtaccaagctgggtgctgctggcatcaacatcgaggctgctgcgttgactcaggctgagaagggtgacggcgctgtcctgatcctgcgtgttgagtccgctgtctctgaagagctggaagctgaaatcaacgctgagttgggtgctacttccttccaggttgatcttgactaataaagcttggttgataaaagaaggagaccagtttatggctcaaatcttcaattttagttctggtccggcaatgctaccggcagaggtgcttaaacaggctcaacaggaactgcgcgactggaacggtcttggtacgtcggtgatggaagtgagtcaccgtggcaaagagttcattcaggttgcagaggaagccgagaaggattttcgcgatcttcttaatgtcccctccaactacaaggtattattctgccatggcggtggtcgcggtcagtttgctgcggtaccgctgaatattctcggtgataaaaccaccgcagattatgttgatgccggttactgggcggcaagtgccattaaagaagcgaaaaaatactgcacgcctaatgtctttgacgccaaagtgactgttgatggtctgcgcgcggttaagccaatgcgtgaatggcaactctctgataatgctgcttatatgcattattgcccgaatgaaaccatcgatggtatcgccatcgacgaaacgccagacttcggcgcagatgtggtggtcgccgctgacttctcttcaaccattctttcccgtccgattgacgtcagccgttatggtgtaatttacgctggcgcgcagaaaaatatcggcccggctggcctgacaatcgtcatcgttcgtgaagatttgctgggcaaagcgaatatcgcgtgtccgtcgattctggattattccatcctcaacgataacggctccatgtttaacacgccgccgacatttgcctggtatctatctggtctggtctttaaatggctgaaagcgaacggcggtgtagctgaaatggataaaatcaatcagcaaaaagcagaactgctatatggggtgattgataacagcgatttctaccgcaatgacgtggcgaaagctaaccgttcgcggatgaacgtgccgttccagttggcggacagtgcgcttgacaaattgttccttgaagagtcttttgctgctggccttcatgcactgaaaggtcaccgtgtggtcggcggaatgcgcgcttctatttataacgccatgccgctggaaggcgttaaagcgctgacagacttcatggttgagttcgaacgccgtcacggttgataaaagaaggagaccagtttatgcctaacattacctggtgcgacctgcctgaagatgtctctttatggccgggtctgcctctttcattaagtggtgatgaagtgatgccactggattaccacgcaggtcgtagcggctggctgctgtatggtcgtgggctggataaacaacgtctgacccaataccagagcaaactgggtgcggcgatggtgattgttgccgcctggtgcgtggaagattatcaggtgattcgtctggcaggttcactcaccgcacgggctacacgcctggcccacgaagcgcagctggatgtcgccccgctggggaaaatcccgcacctgcgcacgccgggtttgctggtgatggatatggactccaccgccatccagattgaatgtattgatgaaattgccaaactggccggaacgggcgagatggtggcggaagtaaccgaacgggcgatgcgcggcgaactcgattttaccgccagcctgcgcagccgtgtggcgacgctgaaaggcgctgacgccaatattctgcaacaggtgcgtgaaaatctgccgctgatgccaggcttaacgcaactggtgctcaagctggaaacgctgggctggaaagtggcgattgcctccggcggctttactttctttgctgaatacctgcgcgacaagctgcgcctgaccgccgtggtagccaatgaactggagatcatggacggtaaatttaccggcaatgtgatcggcgacatcgtagacgcgcagtacaaagcgaaaactctgactcgcctcgcgcaggagtatgaaatcccgctggcgcagaccgtggcgattggcgatggagccaatgacctgccgatgatcaaagcggcagggctggggattgcctaccatgccaagccaaaagtgaatgaaaaggcggaagtcaccatccgtcacgctgacctgatgggggtattctgcatcctctcaggcagcctgaatcagaagtgataagctgaggtcgcctcagcggccggcccctgcaggcgccggcgactagtcttggactcctgttgatagatccagtaatgacctcagaactccatctggatttgttcagaacgctcggttgccgccgggcgttttttattggtgagaatccaggggtccccaataattacgatttaaatttgtgtctcaaaatctctgatgttacattgcacaagataaaaatatatcatcatgaacaataaaactgtctgcttacataaacagtaatacaaggggtgttatgagccatattcagcgtgaaacgagctgtagccgtccgcgtctgaacagcaacatggatgcggatctgtatggctataaatgggcgcgtgataacgtgggtcagagcggcgcgaccatttatcgtctgtatggcaaaccggatgcgccggaactgtttctgaaacatggcaaaggcagcgtggcgaacgatgtgaccgatgaaatggtgcgtctgaactggctgaccgaatttatgccgctgccgaccattaaacattttattcgcaccccggatgatgcgtggctgctgaccaccgcgattccgggcaaaaccgcgtttcaggtgctggaagaatatccggatagcggcgaaaacattgtggatgcgctggccgtgtttctgcgtcgtctgcatagcattccggtgtgcaactgcccgtttaacagcgatcgtgtgtttcgtctggcccaggcgcagagccgtatgaacaacggcctggtggatgcgagcgattttgatgatgaacgtaacggctggccggtggaacaggtgtggaaagaaatgcataaactgctgccgtttagcccggatagcgtggtgacccacggcgattttagcctggataacctgattttcgatgaaggcaaactgattggctgcattgatgtgggccgtgtgggcattgcggatcgttatcaggatctggccattctgtggaactgcctgggcgaatttagcccgagcctgcaaaaacgtctgtttcagaaatatggcattgataatccggatatgaacaaactgcaatttcatctgatgctggatgaatttttctaataattaattggaccgttgtccttttccgctgcataaccctgcttcggggtcattatagcgattttttcggtatatccatcctttttcgcacgatatacaggattttgccaaagggttcgtgtagactttccttggtgtatccaacggcgtcagccgggcaggataggtgaagtaggcccacccgcgagcgggtgttccttcttcactgtcccttattcgcacctggcggtgctcaacgggaatcctgctctgcgaggctggccgtaggccggcctcagatccttccgtatttagccagtatgttctctagtgtggttcgttgtttttgcgtgagccatgagaacgaaccattgagatcatacttactttgcatgtcactcaaaaattttgcctcaaaactggtgagctgaatttttgcagt

SEQ ID NO: 20 - DNA, 6796 bp, synthetic construct
  source 1..6796: mol_type = other DNA
cgttatgtaggtaggaatctgatgtaatggttgttggtattttgtcaccattcatttttatctggttgttctcaagttcggttacgagatccatttgtctatctagttcaacttggaaaatcaacgtatcagtcgggcggcctcgcttatcaaccaccaatttcatattgctgtaagtgtttaaatctttacttattggtttcaaaacccattggttaagccttttaaactcatggtagttattttcaagcattaacatgaacttaaattcatcaaggctaatctctatatttgccttgtgagttttcttttgtgttagttcttttaataaccactcataaatcctcatagagtatttgttttcaaaagacttaacatgttccagattatattttatgaatttttttaactggaaaagataaggcaatatctcttcactaaaaactaattctaatttttcgcttgagaacttggcatagtttgtccactggaaaatctcaaagcctttaaccaaaggattcctgatttccacagttctcgtcatcagctctctggttgctttagctaatacaccataagcattttccctactgatgttcatcatctgagcgtattggttataagtgaacgataccgtccgttctttccttgtagggttttcaatcgtggggttgagtagtgccacacagcataaaattagcttggtttcatgctccgttaagtcatagcgactaatcgctagttcatttgctttgaaaacaactaattcagacatacatctcaattggtctaggtgattttaatcactataccaattgagatgggctagtcaatgataattacatgtccttttcctttgagttgtgggtatctgtaaattctgctagacctttgctggaaaacttgtaaattctgctagaccctctgtaaattccgctagacctttgtgtgttttttttgtttatattcaagtggttataatttatagaataaagaaagaataaaaaaagataaaaagaatagatcccagccctgtgtataactcactactttagtcagttccgcagtattacaaaaggatgtcgcaaacgctgtttgctcctctacaaaacagaccttaaaaccctaaaggcttaagtagcaccctcgcaagctcgggcaaatcgctgaatattccttttgtctccgaccatcaggcacctgagtcgctgtctttttcgtgacattcagttcgctgcgctcacggctctggcagtgaatgggggtaaatggcactacaggcgcggcgcgcccagctgtctagggcggcggatttgtcctactcaggagagcgttcaccgacaaacaacagataaaacgaaaggcccagtctttcgactgagcctttcgttttatttgatgcctttaattaagcggccgcggcgcgcccgtcgacgcgcgcgcggctgaggatacctcagcataggcctaaaaaatttatttgctttcgcatctttttgtacctataatgtgtggatcttaatcatgctaaggaggattaactttatgagccagaatggccgtccggtagtcctcatcgccgataagcttgcgcagtccactgttgacgcgcttggagatgcagtagaagtccgttgggttgacggacctaaccgcccagaactgcttgatgcagttaaggaagcggacgcactgctcgtgcgttctgctaccactgtcgatgctgaagtcatcgccgctgcccctaacttgaagatcgtcggtcgtgccggcgtgggcttggacaacgttgacatccctgctgccactgaagctggcgtcatggttgctaacgcaccgacctctaatattcactccgcttgtgagcacgcaatttctttgctgctgtctactgctcgccagatccctgctgctgatgcgacgctgcgtgagggcgagtggaagcggtcttctttcaacggtgtggaaattttcggaaaaactgtcggtatcgtcggttttggccacattggtcagttgtttgctcagcgtcttgctgcgtttgagaccaccattgttgcttacgatccttacgctaaccctgctcgtgcggctcagctgaacgttgagttggttgagttggatgagctgatgagccgttctgactttgtcaccattcaccttcctaagaccaaggaaactgctggcatgtttgatgcgcagctccttgctaagtccaagaagggccagatcatcatcaacgctgctcgtggtggccttgttgatgagcaggctttggctgatgcgattgagtccggtcacattcgtggcgctggtttcgatgtgtactccaccgagccttgcactgattctcctttgttcaagttgcctcaggttgttgtgactcctcacttgggtgggtctactgaagaggctcaggatcgtgcgggtactgacgttgctgattctgtgctcaaggcgctggctggcgagttcgtggcggatgctgtgaacgtttccggtggtcgcgtgggcgaagaggttgctgtgtggatggatctggctcgcaagcttggtcttcttgctggcaagcttgtcgacgccgccccagtctccattgaggttgaggctcgaggcgagctttcttccgagcaggtcgatgcacttggtttgtccgctgttcgtggtttgttctccggaattatcgaagagtccgttactttcgtcaacgctcctcgcattgctgaagagcgtggcctggacatctccgtgaagaccaactctgagtctgttactcaccgttccgtcctgcaggtcaaggtcattactggcagcggcgcgagcgcaactgttgttggtgccctgactggtcttgagcgcgttgagaagatcacccgcatcaatggccgtggcctggatctgcgcgcagagggtctgaacctcttcctgcaggccactgacgctcctggtgcactgggtaccgttggtaccaagctgggtgctgctggcatcaacatcgaggctgctgcgttgactcaggctgagaagggtgacggcgctgtcctgatcctgcgtgttgagtccgctgtctctgaagagctggaagctgaaatcaacgctgagttgggtgctacttccttccaggttgatcttgactaataaagcttggttgataaaagaaggagaccagtttatggctcaaatcttcaattttagttctggtccggcaatgctaccggcagaggtgcttaaacaggctcaacaggaactgcgcgactggaacggtcttggtacgtcggtgatggaagtgagtcaccgtggcaaagagttcattcaggttgcagaggaagccgagaaggattttcgcgatcttcttaatgtcccctccaactacaaggtattattctgccatggcggtggtcgcggtcagtttgctgcggtaccgctgaatattctcggtgataaaaccaccgcagattatgttgatgccggttactgggcggcaagtgccattaaagaagcgaaaaaatactgcacgcctaatgtctttgacgccaaagtgactgttgatggtctgcgcgcggttaagccaatgcgtgaatggcaactctctgataatgctgcttatatgcattattgcccgaatgaaaccatcgatggtatcgccatcgacgaaacgccagacttcggcgcagatgtggtggtcgccgctgacttctcttcaaccattctttcccgtccgattgacgtcagccgttatggtgtaatttacgctggcgcgcagaaaaatatcggcccggctggcctgacaatcgtcatcgttcgtgaagatttgctgggcaaagcgaatatcgcgtgtccgtcgattctggattattccatcctcaacgataacggctccatgtttaacacgccgccgacatttgcctggtatctatctggtctggtctttaaatggctgaaagcgaacggcggtgtagctgaaatggataaaatcaatcagcaaaaagcagaactgctatatggggtgattgataacagcgatttctaccgcaatgacgtggcgaaagctaaccgttcgcggatgaacgtgccgttccagttggcggacagtgcgcttgacaaattgttccttgaagagtcttttgctgctggccttcatgcactgaaaggtcaccgtgtggtcggcggaatgcgcgcttctatttataacgccatgccgctggaaggcgttaaagcgctgacagacttcatggttgagttcgaacgccgtcacggttgataaaagaaggagaccagtttatgcctaacattacctggtgcgacctgcctgaagatgtctctttatggccgggtctgcctctttcattaagtggtgatgaagtgatgccactggattaccacgcaggtcgtagcggctggctgctgtatggtcgtgggctggataaacaacgtctgacccaataccagagcaaactgggtgcggcgatggtgattgttgccgcctggtgcgtggaagattatcaggtgattcgtctggcaggttcactcaccgcacgggctacacgcctggcccacgaagcgcagctggatgtcgccccgctggggaaaatcccgcacctgcgcacgccgggtttgctggtgatggatatggactccaccgccatccagattgaatgtattgatgaaattgccaaactggccggaacgggcgagatggtggcggaagtaaccgaacgggcgatgcgcggcgaactcgattttaccgccagcctgcgcagccgtgtggcgacgctgaaaggcgctgacgccaatattctgcaacaggtgcgtgaaaatctgccgctgatgccaggcttaacgcaactggtgctcaagctggaaacgctgggctggaaagtggcgattgcctccggcggctttactttctttgctgaatacctgcgcgacaagctgcgcctgaccgccgtggtagccaatgaactggagatcatggacggtaaatttaccggcaatgtgatcggcgacatcgtagacgcgcagtacaaagcgaaaactctgactcgcctcgcgcaggagtatgaaatcccgctggcgcagaccgtggcgattggcgatggagccaatgacctgccgatgatcaaagcggcagggctggggattgcctaccatgccaagccaaaagtgaatgaaaaggcggaagtcaccatccgtcacgctgacctgatgggggtattctgcatcctctcaggcagcctgaatcagaagtgataagctgaggtcgcctcagcggccggcccctgcaggcgccggcgactagtcttggactcctgttgatagatccagtaatgacctcagaactccatctggatttgttcagaacgctcggttgccgccgggcgttttttattggtgagaatccaggggtccccaataattacgatttaaatttgtgtctcaaaatctctgatgttacattgcacaagataaaaatatatcatcatgaacaataaaactgtctgcttacataaacagtaatacaaggggtgttatgagccatattcagcgtgaaacgagctgtagccgtccgcgtctgaacagcaacatggatgcggatctgtatggctataaatgggcgcgtgataacgtgggtcagagcggcgcgaccatttatcgtctgtatggcaaaccggatgcgccggaactgtttctgaaacatggcaaaggcagcgtggcgaacgatgtgaccgatgaaatggtgcgtctgaactggctgaccgaatttatgccgctgccgaccattaaacattttattcgcaccccggatgatgcgtggctgctgaccaccgcgattccgggcaaaaccgcgtttcaggtgctggaagaatatccggatagcggcgaaaacattgtggatgcgctggccgtgtttctgcgtcgtctgcatagcattccggtgtgcaactgcccgtttaacagcgatcgtgtgtttcgtctggcccaggcgcagagccgtatgaacaacggcctggtggatgcgagcgattttgatgatgaacgtaacggctggccggtggaacaggtgtggaaagaaatgcataaactgctgccgtttagcccggatagcgtggtgacccacggcgattttagcctggataacctgattttcgatgaaggcaaactgattggctgcattgatgtgggccgtgtgggcattgcggatcgttatcaggatctggccattctgtggaactgcctgggcgaatttagcccgagcctgcaaaaacgtctgtttcagaaatatggcattgataatccggatatgaacaaactgcaatttcatctgatgctggatgaatttttctaataattaattggaccgttgtccttttccgctgcataaccctgcttcggggtcattatagcgattttttcggtatatccatcctttttcgcacgatatacaggattttgccaaagggttcgtgtagactttccttggtgtatccaacggcgtcagccgggcaggataggtgaagtaggcccacccgcgagcgggtgttccttcttcactgtcccttattcgcacctggcggtgctcaacgggaatcctgctctgcgaggctggccgtaggccggcctcagatccttccgtatttagccagtatgttctctagtgtggttcgttgtttttgcgtgagccatgagaacgaaccattgagatcatacttactttgcatgtcactcaaaaattttgcctcaaaactggtgagctgaatttttgcagttaaagcatcgtgtagtgtttttcttagtc

SEQ ID NO: 21 - DNA, 6795 bp, synthetic construct
  source 1..6795: mol_type = other DNA
tggtattttgtcaccattcatttttatctggttgttctcaagttcggttacgagatccatttgtctatctagttcaacttggaaaatcaacgtatcagtcgggcggcctcgcttatcaaccaccaatttcatattgctgtaagtgtttaaatctttacttattggtttcaaaacccattggttaagccttttaaactcatggtagttattttcaagcattaacatgaacttaaattcatcaaggctaatctctatatttgccttgtgagttttcttttgtgttagttcttttaataaccactcataaatcctcatagagtatttgttttcaaaagacttaacatgttccagattatattttatgaatttttttaactggaaaagataaggcaatatctcttcactaaaaactaattctaatttttcgcttgagaacttggcatagtttgtccactggaaaatctcaaagcctttaaccaaaggattcctgatttccacagttctcgtcatcagctctctggttgctttagctaatacaccataagcattttccctactgatgttcatcatctgagcgtattggttataagtgaacgataccgtccgttctttccttgtagggttttcaatcgtggggttgagtagtgccacacagcataaaattagcttggtttcatgctccgttaagtcatagcgactaatcgctagttcatttgctttgaaaacaactaattcagacatacatctcaattggtctaggtgattttaatcactataccaattgagatgggctagtcaatgataattacatgtccttttcctttgagttgtgggtatctgtaaattctgctagacctttgctggaaaacttgtaaattctgctagaccctctgtaaattccgctagacctttgtgtgttttttttgtttatattcaagtggttataatttatagaataaagaaagaataaaaaaagataaaaagaatagatcccagccctgtgtataactcactactttagtcagttccgcagtattacaaaaggatgtcgcaaacgctgtttgctcctctacaaaacagaccttaaaaccctaaaggcttaagtagcaccctcgcaagctcgggcaaatcgctgaatattccttttgtctccgaccatcaggcacctgagtcgctgtctttttcgtgacattcagttcgctgcgctcacggctctggcagtgaatgggggtaaatggcactacaggcgcggcgcgcccagctgtctagggcggcggatttgtcctactcaggagagcgttcaccgacaaacaacagataaaacgaaaggcccagtctttcgactgagcctttcgttttatttgatgcctttaattaagcggccgcggcgcgcccgtcgacgcgcgcgcggctgaggatacctcagcataggcctaaaaagagtattgacttcgcatctttttgtacctataatgtgtggatcttaatcatgctaaggaggattaactttatgagccagaatggccgtccggtagtcctcatcgccgataagcttgcgcagtccactgttgacgcgcttggagatgcagtagaagtccgttgggttgacggacctaaccgcccagaactgcttgatgcagttaaggaagcggacgcactgctcgtgcgttctgctaccactgtcgatgctgaagtcatcgccgctgcccctaacttgaagatcgtcggtcgtgccggcgtgggcttggacaacgttgacatccctgctgccactgaagctggcgtcatggttgctaacgcaccgacctctaatattcactccgcttgtgagcacgcaatttctttgctgctgtctactgctcgccagatccctgctgctgatgcgacgctgcgtgagggcgagtggaagcggtcttctttcaacggtgtggaaattttcggaaaaactgtcggtatcgtcggttttggccacattggtcagttgtttgctcagcgtcttgctgcgtttgagaccaccattgttgcttacgatccttacgctaaccctgctcgtgcggctcagctgaacgttgagttggttgagttggatgagctgatgagccgttctgactttgtcaccattcaccttcctaagaccaaggaaactgctggcatgtttgatgcgcagctccttgctaagtccaagaagggccagatcatcatcaacgctgctcgtggtggccttgttgatgagcaggctttggctgatgcgattgagtccggtcacattcgtggcgctggtttcgatgtgtactccaccgagccttgcactgattctcctttgttcaagttgcctcaggttgttgtgactcctcacttgggtgggtctactgaagaggctcaggatcgtgcgggtactgacgttgctgattctgtgctcaaggcgctggctggcgagttcgtggcggatgctgtgaacgtttccggtggtcgcgtgggcgaagaggttgctgtgtggatggatctggctcgcaagcttggtcttcttgctggcaagcttgtcgacgccgccccagtctccattgaggttgaggctcgaggcgagctttcttccgagcaggtcgatgcacttggtttgtccgctgttcgtggtttgttctccggaattatcgaagagtccgttactttcgtcaacgctcctcgcattgctgaagagcgtggcctggacatctccgtgaagaccaactctgagtctgttactcaccgttccgtcctgcaggtcaaggtcattactggcagcggcgcgagcgcaactgttgttggtgccctgactggtcttgagcgcgttgagaagatcacccgcatcaatggccgtggcctggatctgcgcgcagagggtctgaacctcttcctgcaggccactgacgctcctggtgcactgggtaccgttggtaccaagctgggtgctgctggcatcaacatcgaggctgctgcgttgactcaggctgagaagggtgacggcgctgtcctgatcctgcgtgttgagtccgctgtctctgaagagctggaagctgaaatcaacgctgagttgggtgctacttccttccaggttgatcttgactaataaagcttggttgataaaagaaggagaccagtttatggctcaaatcttcaattttagttctggtccggcaatgctaccggcagaggtgcttaaacaggctcaacaggaactgcgcgactggaacggtcttggtacgtcggtgatggaagtgagtcaccgtggcaaagagttcattcaggttgcagaggaagccgagaaggattttcgcgatcttcttaatgtcccctccaactacaaggtattattctgccatggcggtggtcgcggtcagtttgctgcggtaccgctgaatattctcggtgataaaaccaccgcagattatgttgatgccggttactgggcggcaagtgccattaaagaagcgaaaaaatactgcacgcctaatgtctttgacgccaaagtgactgttgatggtctgcgcgcggttaagccaatgcgtgaatggcaactctctgataatgctgcttatatgcattattgcccgaatgaaaccatcgatggtatcgccatcgacgaaacgccagacttcggcgcagatgtggtggtcgccgctgacttctcttcaaccattctttcccgtccgattgacgtcagccgttatggtgtaatttacgctggcgcgcagaaaaatatcggcccggctggcctgacaatcgtcatcgttcgtgaagatttgctgggcaaagcgaatatcgcgtgtccgtcgattctggattattccatcctcaacgataacggctccatgtttaacacgccgccgacatttgcctggtatctatctggtctggtctttaaatggctgaaagcgaacggcggtgtagctgaaatggataaaatcaatcagcaaaaagcagaactgctatatggggtgattgataacagcgatttctaccgcaatgacgtggcgaaagctaaccgttcgcggatgaacgtgccgttccagttggcggacagtgcgcttgacaaattgttccttgaagagtcttttgctgctggccttcatgcactgaaaggtcaccgtgtggtcggcggaatgcgcgcttctatttataacgccatgccgctggaaggcgttaaagcgctgacagacttcatggttgagttcgaacgccgtcacggttgataaaagaaggagaccagtttatgcctaacattacctggtgcgacctgcctgaagatgtctctttatggccgggtctgcctctttcattaagtggtgatgaagtgatgccactggattaccacgcaggtcgtagcggctggctgctgtatggtcgtgggctggataaacaacgtctgacccaataccagagcaaactgggtgcggcgatggtgattgttgccgcctggtgcgtggaagattatcaggtgattcgtctggcaggttcactcaccgcacgggctacacgcctggcccacgaagcgcagctggatgtcgccccgctggggaaaatcccgcacctgcgcacgccgggtttgctggtgatggatatggactccaccgccatccagattgaatgtattgatgaaattgccaaactggccggaacgggcgagatggtggcggaagtaaccgaacgggcgatgcgcggcgaactcgattttaccgccagcctgcgcagccgtgtggcgacgctgaaaggcgctgacgccaatattctgcaacaggtgcgtgaaaatctgccgctgatgccaggcttaacgcaactggtgctcaagctggaaacgctgggctggaaagtggcgattgcctccggcggctttactttctttgctgaatacctgcgcgacaagctgcgcctgaccgccgtggtagccaatgaactggagatcatggacggtaaatttaccggcaatgtgatcggcgacatcgtagacgcgcagtacaaagcgaaaactctgactcgcctcgcgcaggagtatgaaatcccgctggcgcagaccgtggcgattggcgatggagccaatgacctgccgatgatcaaagcggcagggctggggattgcctaccatgccaagccaaaagtgaatgaaaaggcggaagtcaccatccgtcacgctgacctgatgggggtattctgcatcctctcaggcagcctgaatcagaagtgataagctgaggtcgcctcagcggccggcccctgcaggcgccggcgactagtcttggactcctgttgatagatccagtaatgacctcagaactccatctggatttgttcagaacgctcggttgccgccgggcgttttttattggtgagaatccaggggtccccaataattacgatttaaatttgtgtctcaaaatctctgatgttacattgcacaagataaaaatatatcatcatgaacaataaaactgtctgcttacataaacagtaatacaaggggtgttatgagccatattcagcgtgaaacgagctgtagccgtccgcgtctgaacagcaacatggatgcggatctgtatggctataaatgggcgcgtgataacgtgggtcagagcggcgcgaccatttatcgtctgtatggcaaaccggatgcgccggaactgtttctgaaacatggcaaaggcagcgtggcgaacgatgtgaccgatgaaatggtgcgtctgaactggctgaccgaatttatgccgctgccgaccattaaacattttattcgcaccccggatgatgcgtggctgctgaccaccgcgattccgggcaaaaccgcgtttcaggtgctggaagaatatccggatagcggcgaaaacattgtggatgcgctggccgtgtttctgcgtcgtctgcatagcattccggtgtgcaactgcccgtttaacagcgatcgtgtgtttcgtctggcccaggcgcagagccgtatgaacaacggcctggtggatgcgagcgattttgatgatgaacgtaacggctggccggtggaacaggtgtggaaagaaatgcataaactgctgccgtttagcccggatagcgtggtgacccacggcgattttagcctggataacctgattttcgatgaaggcaaactgattggctgcattgatgtgggccgtgtgggcattgcggatcgttatcaggatctggccattctgtggaactgcctgggcgaatttagcccgagcctgcaaaaacgtctgtttcagaaatatggcattgataatccggatatgaacaaactgcaatttcatctgatgctggatgaatttttctaataattaattggaccgttgtccttttccgctgcataaccctgcttcggggtcattatagcgattttttcggtatatccatcctttttcgcacgatatacaggattttgccaaagggttcgtgtagactttccttggtgtatccaacggcgtcagccgggcaggataggtgaagtaggcccacccgcgagcgggtgttccttcttcactgtcccttattcgcacctggcggtgctcaacgggaatcctgctctgcgaggctggccgtaggccggcctcagatccttccgtatttagccagtatgttctctagtgtggttcgttgtttttgcgtgagccatgagaacgaaccattgagatcatacttactttgcatgtcactcaaaaattttgcctcaaaactggtgagctgaatttttgcagttaaagcatcgtgtagtgtttttcttagtccgttatgtaggtaggaatctgatgtaatggttgt

SEQ ID NO: 22 - DNA, 6784 bp, synthetic construct
  source 1..6784: mol_type = other DNA
cgtatttagccagtatgttctctagtgtggttcgttgtttttgcgtgagccatgagaacgaaccattgagatcatacttactttgcatgtcactcaaaaattttgcctcaaaactggtgagctgaatttttgcagttaaagcatcgtgtagtgtttttcttagtccgttatgtaggtaggaatctgatgtaatggttgttggtattttgtcaccattcatttttatctggttgttctcaagttcggttacgagatccatttgtctatctagttcaacttggaaaatcaacgtatcagtcgggcggcctcgcttatcaaccaccaatttcatattgctgtaagtgtttaaatctttacttattggtttcaaaacccattggttaagccttttaaactcatggtagttattttcaagcattaacatgaacttaaattcatcaaggctaatctctatatttgccttgtgagttttcttttgtgttagttcttttaataaccactcataaatcctcatagagtatttgttttcaaaagacttaacatgttccagattatattttatgaatttttttaactggaaaagataaggcaatatctcttcactaaaaactaattctaatttttcgcttgagaacttggcatagtttgtccactggaaaatctcaaagcctttaaccaaaggattcctgatttccacagttctcgtcatcagctctctggttgctttagctaatacaccataagcattttccctactgatgttcatcatctgagcgtattggttataagtgaacgataccgtccgttctttccttgtagggttttcaatcgtggggttgagtagtgccacacagcataaaattagcttggtttcatgctccgttaagtcatagcgactaatcgctagttcatttgctttgaaaacaactaattcagacatacatctcaattggtctaggtgattttaatcactataccaattgagatgggctagtcaatgataattacatgtccttttcctttgagttgtgggtatctgtaaattctgctagacctttgctggaaaacttgtaaattctgctagaccctctgtaaattccgctagacctttgtgtgttttttttgtttatattcaagtggttataatttatagaataaagaaagaataaaaaaagataaaaagaatagatcccagccctgtgtataactcactactttagtcagttccgcagtattacaaaaggatgtcgcaaacgctgtttgctcctctacaaaacagaccttaaaaccctaaaggcttaagtagcaccctcgcaagctcgggcaaatcgctgaatattccttttgtctccgaccatcaggcacctgagtcgctgtctttttcgtgacattcagttcgctgcgctcacggctctggcagtgaatgggggtaaatggcactacaggcgcggcgcgcccagctgtctagggcggcggatttgtcctactcaggagagcgttcaccgacaaacaacagataaaacgaaaggcccagtctttcgactgagcctttcgttttatttgatgcctttaattaagcggccgcggcgcgcccgtcgacgcgcgcgcggctgaggatacctcagcataggcctttgacagctagctcagtcctaggtactgtgctagctcttaatcatgctaaggaggattaactttatgagccagaatggccgtccggtagtcctcatcgccgataagcttgcgcagtccactgttgacgcgcttggagatgcagtagaagtccgttgggttgacggacctaaccgcccagaactgcttgatgcagttaaggaagcggacgcactgctcgtgcgttctgctaccactgtcgatgctgaagtcatcgccgctgcccctaacttgaagatcgtcggtcgtgccggcgtgggcttggacaacgttgacatccctgctgccactgaagctggcgtcatggttgctaacgcaccgacctctaatattcactccgcttgtgagcacgcaatttctttgctgctgtctactgctcgccagatccctgctgctgatgcgacgctgcgtgagggcgagtggaagcggtcttctttcaacggtgtggaaattttcggaaaaactgtcggtatcgtcggttttggccacattggtcagttgtttgctcagcgtcttgctgcgtttgagaccaccattgttgcttacgatccttacgctaaccctgctcgtgcggctcagctgaacgttgagttggttgagttggatgagctgatgagccgttctgactttgtcaccattcaccttcctaagaccaaggaaactgctggcatgtttgatgcgcagctccttgctaagtccaagaagggccagatcatcatcaacgctgctcgtggtggccttgttgatgagcaggctttggctgatgcgattgagtccggtcacattcgtggcgctggtttcgatgtgtactccaccgagccttgcactgattctcctttgttcaagttgcctcaggttgttgtgactcctcacttgggtgggtctactgaagaggctcaggatcgtgcgggtactgacgttgctgattctgtgctcaaggcgctggctggcgagttcgtggcggatgctgtgaacgtttccggtggtcgcgtgggcgaagaggttgctgtgtggatggatctggctcgcaagcttggtcttcttgctggcaagcttgtcgacgccgccccagtctccattgaggttgaggctcgaggcgagctttcttccgagcaggtcgatgcacttggtttgtccgctgttcgtggtttgttctccggaattatcgaagagtccgttactttcgtcaacgctcctcgcattgctgaagagcgtggcctggacatctccgtgaagaccaactctgagtctgttactcaccgttccgtcctgcaggtcaaggtcattactggcagcggcgcgagcgcaactgttgttggtgccctgactggtcttgagcgcgttgagaagatcacccgcatcaatggccgtggcctggatctgcgcgcagagggtctgaacctcttcctgcaggccactgacgctcctggtgcactgggtaccgttggtaccaagctgggtgctgctggcatcaacatcgaggctgctgcgttgactcaggctgagaagggtgacggcgctgtcctgatcctgcgtgttgagtccgctgtctctgaagagctggaagctgaaatcaacgctgagttgggtgctacttccttccaggttgatcttgactaataaagcttggttgataaaagaaggagaccagtttatggctcaaatcttcaattttagttctggtccggcaatgctaccggcagaggtgcttaaacaggctcaacaggaactgcgcgactggaacggtcttggtacgtcggtgatggaagtgagtcaccgtggcaaagagttcattcaggttgcagaggaagccgagaaggattttcgcgatcttcttaatgtcccctccaactacaaggtattattctgccatggcggtggtcgcggtcagtttgctgcggtaccgctgaatattctcggtgataaaaccaccgcagattatgttgatgccggttactgggcggcaagtgccattaaagaagcgaaaaaatactgcacgcctaatgtctttgacgccaaagtgactgttgatggtctgcgcgcggttaagccaatgcgtgaatggcaactctctgataatgctgcttatatgcattattgcccgaatgaaaccatcgatggtatcgccatcgacgaaacgccagacttcggcgcagatgtggtggtcgccgctgacttctcttcaaccattctttcccgtccgattgacgtcagccgttatggtgtaatttacgctggcgcgcagaaaaatatcggcccggctggcctgacaatcgtcatcgttcgtgaagatttgctgggcaaagcgaatatcgcgtgtccgtcgattctggattattccatcctcaacgataacggctccatgtttaacacgccgccgacatttgcctggtatctatctggtctggtctttaaatggctgaaagcgaacggcggtgtagctgaaatggataaaatcaatcagcaaaaagcagaactgctatatggggtgattgataacagcgatttctaccgcaatgacgtggcgaaagctaaccgttcgcggatgaacgtgccgttccagttggcggacagtgcgcttgacaaattgttccttgaagagtcttttgctgctggccttcatgcactgaaaggtcaccgtgtggtcggcggaatgcgcgcttctatttataacgccatgccgctggaaggcgttaaagcgctgacagacttcatggttgagttcgaacgccgtcacggttgataaaagaaggagaccagtttatgcctaacattacctggtgcgacctgcctgaagatgtctctttatggccgggtctgcctctttcattaagtggtgatgaagtgatgccactggattaccacgcaggtcgtagcggctggctgctgtatggtcgtgggctggataaacaacgtctgacccaataccagagcaaactgggtgcggcgatggtgattgttgccgcctggtgcgtggaagattatcaggtgattcgtctggcaggttcactcaccgcacgggctacacgcctggcccacgaagcgcagctggatgtcgccccgctggggaaaatcccgcacctgcgcacgccgggtttgctggtgatggatatggactccaccgccatccagattgaatgtattgatgaaattgccaaactggccggaacgggcgagatggtggcggaagtaaccgaacgggcgatgcgcggcgaactcgattttaccgccagcctgcgcagccgtgtggcgacgctgaaaggcgctgacgccaatattctgcaacaggtgcgtgaaaatctgccgctgatgccaggcttaacgcaactggtgctcaagctggaaacgctgggctggaaagtggcgattgcctccggcggctttactttctttgctgaatacctgcgcgacaagctgcgcctgaccgccgtggtagccaatgaactggagatcatggacggtaaatttaccggcaatgtgatcggcgacatcgtagacgcgcagtacaaagcgaaaactctgactcgcctcgcgcaggagtatgaaatcccgctggcgcagaccgtggcgattggcgatggagccaatgacctgccgatgatcaaagcggcagggctggggattgcctaccatgccaagccaaaagtgaatgaaaaggcggaagtcaccatccgtcacgctgacctgatgggggtattctgcatcctctcaggcagcctgaatcagaagtgataagctgaggtcgcctcagcggccggcccctgcaggcgccggcgactagtcttggactcctgttgatagatccagtaatgacctcagaactccatctggatttgttcagaacgctcggttgccgccgggcgttttttattggtgagaatccaggggtccccaataattacgatttaaatttgtgtctcaaaatctctgatgttacattgcacaagataaaaatatatcatcatgaacaataaaactgtctgcttacataaacagtaatacaaggggtgttatgagccatattcagcgtgaaacgagctgtagccgtccgcgtctgaacagcaacatggatgcggatctgtatggctataaatgggcgcgtgataacgtgggtcagagcggcgcgaccatttatcgtctgtatggcaaaccggatgcgccggaactgtttctgaaacatggcaaaggcagcgtggcgaacgatgtgaccgatgaaatggtgcgtctgaactggctgaccgaatttatgccgctgccgaccattaaacattttattcgcaccccggatgatgcgtggctgctgaccaccgcgattccgggcaaaaccgcgtttcaggtgctggaagaatatccggatagcggcgaaaacattgtggatgcgctggccgtgtttctgcgtcgtctgcatagcattccggtgtgcaactgcccgtttaacagcgatcgtgtgtttcgtctggcccaggcgcagagccgtatgaacaacggcctggtggatgcgagcgattttgatgatgaacgtaacggctggccggtggaacaggtgtggaaagaaatgcataaactgctgccgtttagcccggatagcgtggtgacccacggcgattttagcctggataacctgattttcgatgaaggcaaactgattggctgcattgatgtgggccgtgtgggcattgcggatcgttatcaggatctggccattctgtggaactgcctgggcgaatttagcccgagcctgcaaaaacgtctgtttcagaaatatggcattgataatccggatatgaacaaactgcaatttcatctgatgctggatgaatttttctaataattaattggaccgttgtccttttccgctgcataaccctgcttcggggtcattatagcgattttttcggtatatccatcctttttcgcacgatatacaggattttgccaaagggttcgtgtagactttccttggtgtatccaacggcgtcagccgggcaggataggtgaagtaggcccacccgcgagcgggtgttccttcttcactgtcccttattcgcacctggcggtgctcaacgggaatcctgctctgcgaggctggccgtaggccggcctcagatccttc

SEQ ID NO: 23 - DNA, 6785 bp, synthetic construct
  source 1..6785: mol_type = other DNA
gataggtgaagtaggcccacccgcgagcgggtgttccttcttcactgtcccttattcgcacctggcggtgctcaacgggaatcctgctctgcgaggctggccgtaggccggcctcagatccttccgtatttagccagtatgttctctagtgtggttcgttgtttttgcgtgagccatgagaacgaaccattgagatcatacttactttgcatgtcactcaaaaattttgcctcaaaactggtgagctgaatttttgcagttaaagcatcgtgtagtgtttttcttagtccgttatgtaggtaggaatctgatgtaatggttgttggtattttgtcaccattcatttttatctggttgttctcaagttcggttacgagatccatttgtctatctagttcaacttggaaaatcaacgtatcagtcgggcggcctcgcttatcaaccaccaatttcatattgctgtaagtgtttaaatctttacttattggtttcaaaacccattggttaagccttttaaactcatggtagttattttcaagcattaacatgaacttaaattcatcaaggctaatctctatatttgccttgtgagttttcttttgtgttagttcttttaataaccactcataaatcctcatagagtatttgttttcaaaagacttaacatgttccagattatattttatgaatttttttaactggaaaagataaggcaatatctcttcactaaaaactaattctaatttttcgcttgagaacttggcatagtttgtccactggaaaatctcaaagcctttaaccaaaggattcctgatttccacagttctcgtcatcagctctctggttgctttagctaatacaccataagcattttccctactgatgttcatcatctgagcgtattggttataagtgaacgataccgtccgttctttccttgtagggttttcaatcgtggggttgagtagtgccacacagcataaaattagcttggtttcatgctccgttaagtcatagcgactaatcgctagttcatttgctttgaaaacaactaattcagacatacatctcaattggtctaggtgattttaatcactataccaattgagatgggctagtcaatgataattacatgtccttttcctttgagttgtgggtatctgtaaattctgctagacctttgctggaaaacttgtaaattctgctagaccctctgtaaattccgctagacctttgtgtgttttttttgtttatattcaagtggttataatttatagaataaagaaagaataaaaaaagataaaaagaatagatcccagccctgtgtataactcactactttagtcagttccgcagtattacaaaaggatgtcgcaaacgctgtttgctcctctacaaaacagaccttaaaaccctaaaggcttaagtagcaccctcgcaagctcgggcaaatcgctgaatattccttttgtctccgaccatcaggcacctgagtcgctgtctttttcgtgacattcagttcgctgcgctcacggctctggcagtgaatgggggtaaatggcactacaggcgcggcgcgcccagctgtctagggcggcggatttgtcctactcaggagagcgttcaccgacaaacaacagataaaacgaaaggcccagtctttcgactgagcctttcgttttatttgatgcctttaattaagcggccgcggcgcgcccgtcgacgcgcgcgcggctgaggatacctcagcataggcctttgacaattaatcatccggctcgtaatttatgtggatcttaatcatgctaaggaggattaactttatgagccagaatggccgtccggtagtcctcatcgccgataagcttgcgcagtccactgttgacgcgcttggagatgcagtagaagtccgttgggttgacggacctaaccgcccagaactgcttgatgcagttaaggaagcggacgcactgctcgtgcgttctgctaccactgtcgatgctgaagtcatcgccgctgcccctaacttgaagatcgtcggtcgtgccggcgtgggcttggacaacgttgacatccctgctgccactgaagctggcgtcatggttgctaacgcaccgacctctaatattcactccgcttgtgagcacgcaatttctttgctgctgtctactgctcgccagatccctgctgctgatgcgacgctgcgtgagggcgagtggaagcggtcttctttcaacggtgtggaaattttcggaaaaactgtcggtatcgtcggttttggccacattggtcagttgtttgctcagcgtcttgctgcgtttgagaccaccattgttgcttacgatccttacgctaaccctgctcgtgcggctcagctgaacgttgagttggttgagttggatgagctgatgagccgttctgactttgtcaccattcaccttcctaagaccaaggaaactgctggcatgtttgatgcgcagctccttgctaagtccaagaagggccagatcatcatcaacgctgctcgtggtggccttgttgatgagcaggctttggctgatgcgattgagtccggtcacattcgtggcgctggtttcgatgtgtactccaccgagccttgcactgattctcctttgttcaagttgcctcaggttgttgtgactcctcacttgggtgggtctactgaagaggctcaggatcgtgcgggtactgacgttgctgattctgtgctcaaggcgctggctggcgagttcgtggcggatgctgtgaacgtttccggtggtcgcgtgggcgaagaggttgctgtgtggatggatctggctcgcaagcttggtcttcttgctggcaagcttgtcgacgccgccccagtctccattgaggttgaggctcgaggcgagctttcttccgagcaggtcgatgcacttggtttgtccgctgttcgtggtttgttctccggaattatcgaagagtccgttactttcgtcaacgctcctcgcattgctgaagagcgtggcctggacatctccgtgaagaccaactctgagtctgttactcaccgttccgtcctgcaggtcaaggtcattactggcagcggcgcgagcgcaactgttgttggtgccctgactggtcttgagcgcgttgagaagatcacccgcatcaatggccgtggcctggatctgcgcgcagagggtctgaacctcttcctgcaggccactgacgctcctggtgcactgggtaccgttggtaccaagctgggtgctgctggcatcaacatcgaggctgctgcgttgactcaggctgagaagggtgacggcgctgtcctgatcctgcgtgttgagtccgctgtctctgaagagctggaagctgaaatcaacgctgagttgggtgctacttccttccaggttgatcttgactaataaagcttggttgataaaagaaggagaccagtttatggctcaaatcttcaattttagttctggtccggcaatgctaccggcagaggtgcttaaacaggctcaacaggaactgcgcgactggaacggtcttggtacgtcggtgatggaagtgagtcaccgtggcaaagagttcattcaggttgcagaggaagccgagaaggattttcgcgatcttcttaatgtcccctccaactacaaggtattattctgccatggcggtggtcgcggtcagtttgctgcggtaccgctgaatattctcggtgataaaaccaccgcagattatgttgatgccggttactgggcggcaagtgccattaaagaagcgaaaaaatactgcacgcctaatgtctttgacgccaaagtgactgttgatggtctgcgcgcggttaagccaatgcgtgaatggcaactctctgataatgctgcttatatgcattattgcccgaatgaaaccatcgatggtatcgccatcgacgaaacgccagacttcggcgcagatgtggtggtcgccgctgacttctcttcaaccattctttcccgtccgattgacgtcagccgttatggtgtaatttacgctggcgcgcagaaaaatatcggcccggctggcctgacaatcgtcatcgttcgtgaagatttgctgggcaaagcgaatatcgcgtgtccgtcgattctggattattccatcctcaacgataacggctccatgtttaacacgccgccgacatttgcctggtatctatctggtctggtctttaaatggctgaaagcgaacggcggtgtagctgaaatggataaaatcaatcagcaaaaagcagaactgctatatggggtgattgataacagcgatttctaccgcaatgacgtggcgaaagctaaccgttcgcggatgaacgtgccgttccagttggcggacagtgcgcttgacaaattgttccttgaagagtcttttgctgctggccttcatgcactgaaaggtcaccgtgtggtcggcggaatgcgcgcttctatttataacgccatgccgctggaaggcgttaaagcgctgacagacttcatggttgagttcgaacgccgtcacggttgataaaagaaggagaccagtttatgcctaacattacctggtgcgacctgcctgaagatgtctctttatggccgggtctgcctctttcattaagtggtgatgaagtgatgccactggattaccacgcaggtcgtagcggctggctgctgtatggtcgtgggctggataaacaacgtctgacccaataccagagcaaactgggtgcggcgatggtgattgttgccgcctggtgcgtggaagattatcaggtgattcgtctggcaggttcactcaccgcacgggctacacgcctggcccacgaagcgcagctggatgtcgccccgctggggaaaatcccgcacctgcgcacgccgggtttgctggtgatggatatggactccaccgccatccagattgaatgtattgatgaaattgccaaactggccggaacgggcgagatggtggcggaagtaaccgaacgggcgatgcgcggcgaactcgattttaccgccagcctgcgcagccgtgtggcgacgctgaaaggcgctgacgccaatattctgcaacaggtgcgtgaaaatctgccgctgatgccaggcttaacgcaactggtgctcaagctggaaacgctgggctggaaagtggcgattgcctccggcggctttactttctttgctgaatacctgcgcgacaagctgcgcctgaccgccgtggtagccaatgaactggagatcatggacggtaaatttaccggcaatgtgatcggcgacatcgtagacgcgcagtacaaagcgaaaactctgactcgcctcgcgcaggagtatgaaatcccgctggcgcagaccgtggcgattggcgatggagccaatgacctgccgatgatcaaagcggcagggctggggattgcctaccatgccaagccaaaagtgaatgaaaaggcggaagtcaccatccgtcacgctgacctgatgggggtattctgcatcctctcaggcagcctgaatcagaagtgataagctgaggtcgcctcagcggccggcccctgcaggcgccggcgactagtcttggactcctgttgatagatccagtaatgacctcagaactccatctggatttgttcagaacgctcggttgccgccgggcgttttttattggtgagaatccaggggtccccaataattacgatttaaatttgtgtctcaaaatctctgatgttacattgcacaagataaaaatatatcatcatgaacaataaaactgtctgcttacataaacagtaatacaaggggtgttatgagccatattcagcgtgaaacgagctgtagccgtccgcgtctgaacagcaacatggatgcggatctgtatggctataaatgggcgcgtgataacgtgggtcagagcggcgcgaccatttatcgtctgtatggcaaaccggatgcgccggaactgtttctgaaacatggcaaaggcagcgtggcgaacgatgtgaccgatgaaatggtgcgtctgaactggctgaccgaatttatgccgctgccgaccattaaacattttattcgcaccccggatgatgcgtggctgctgaccaccgcgattccgggcaaaaccgcgtttcaggtgctggaagaatatccggatagcggcgaaaacattgtggatgcgctggccgtgtttctgcgtcgtctgcatagcattccggtgtgcaactgcccgtttaacagcgatcgtgtgtttcgtctggcccaggcgcagagccgtatgaacaacggcctggtggatgcgagcgattttgatgatgaacgtaacggctggccggtggaacaggtgtggaaagaaatgcataaactgctgccgtttagcccggatagcgtggtgacccacggcgattttagcctggataacctgattttcgatgaaggcaaactgattggctgcattgatgtgggccgtgtgggcattgcggatcgttatcaggatctggccattctgtggaactgcctgggcgaatttagcccgagcctgcaaaaacgtctgtttcagaaatatggcattgataatccggatatgaacaaactgcaatttcatctgatgctggatgaatttttctaataattaattggaccgttgtccttttccgctgcataaccctgcttcggggtcattatagcgattttttcggtatatccatcctttttcgcacgatatacaggattttgccaaagggttcgtgtagactttccttggtgtatccaacggcgtcagccgggcag

SEQ ID NO: 24 - DNA, 6785 bp, synthetic construct
  source 1..6785: mol_type = other DNA
gaaaagataaggcaatatctcttcactaaaaactaattctaatttttcgcttgagaacttggcatagtttgtccactggaaaatctcaaagcctttaaccaaaggattcctgatttccacagttctcgtcatcagctctctggttgctttagctaatacaccataagcattttccctactgatgttcatcatctgagcgtattggttataagtgaacgataccgtccgttctttccttgtagggttttcaatcgtggggttgagtagtgccacacagcataaaattagcttggtttcatgctccgttaagtcatagcgactaatcgctagttcatttgctttgaaaacaactaattcagacatacatctcaattggtctaggtgattttaatcactataccaattgagatgggctagtcaatgataattacatgtccttttcctttgagttgtgggtatctgtaaattctgctagacctttgctggaaaacttgtaaattctgctagaccctctgtaaattccgctagacctttgtgtgttttttttgtttatattcaagtggttataatttatagaataaagaaagaataaaaaaagataaaaagaatagatcccagccctgtgtataactcactactttagtcagttccgcagtattacaaaaggatgtcgcaaacgctgtttgctcctctacaaaacagaccttaaaaccctaaaggcttaagtagcaccctcgcaagctcgggcaaatcgctgaatattccttttgtctccgaccatcaggcacctgagtcgctgtctttttcgtgacattcagttcgctgcgctcacggctctggcagtgaatgggggtaaatggcactacaggcgcggcgcgcccagctgtctagggcggcggatttgtcctactcaggagagcgttcaccgacaaacaacagataaaacgaaaggcccagtctttcgactgagcctttcgttttatttgatgcctttaattaagcggccgcggcgcgcccgtcgacgcgcgcgcggctgaggatacctcagcataggcctttgacaattaatcatccggctcgtaatgtttgtggatcttaatcatgctaaggaggattaactttatgagccagaatggccgtccggtagtcctcatcgccgataagcttgcgcagtccactgttgacgcgcttggagatgcagtagaagtccgttgggttgacggacctaaccgcccagaactgcttgatgcagttaaggaagcggacgcactgctcgtgcgttctgctaccactgtcgatgctgaagtcatcgccgctgcccctaacttgaagatcgtcggtcgtgccggcgtgggcttggacaacgttgacatccctgctgccactgaagctggcgtcatggttgctaacgcaccgacctctaatattcactccgcttgtgagcacgcaatttctttgctgctgtctactgctcgccagatccctgctgctgatgcgacgctgcgtgagggcgagtggaagcggtcttctttcaacggtgtggaaattttcggaaaaactgtcggtatcgtcggttttggccacattggtcagttgtttgctcagcgtcttgctgcgtttgagaccaccattgttgcttacgatccttacgctaaccctgctcgtgcggctcagctgaacgttgagttggttgagttggatgagctgatgagccgttctgactttgtcaccattcaccttcctaagaccaaggaaactgctggcatgtttgatgcgcagctccttgctaagtccaagaagggccagatcatcatcaacgctgctcgtggtggccttgttgatgagcaggctttggctgatgcgattgagtccggtcacattcgtggcgctggtttcgatgtgtactccaccgagccttgcactgattctcctttgttcaagttgcctcaggttgttgtgactcctcacttgggtgggtctactgaagaggctcaggatcgtgcgggtactgacgttgctgattctgtgctcaaggcgctggctggcgagttcgtggcggatgctgtgaacgtttccggtggtcgcgtgggcgaagaggttgctgtgtggatggatctggctcgcaagcttggtcttcttgctggcaagcttgtcgacgccgccccagtctccattgaggttgaggctcgaggcgagctttcttccgagcaggtcgatgcacttggtttgtccgctgttcgtggtttgttctccggaattatcgaagagtccgttactttcgtcaacgctcctcgcattgctgaagagcgtggcctggacatctccgtgaagaccaactctgagtctgttactcaccgttccgtcctgcaggtcaaggtcattactggcagcggcgcgagcgcaactgttgttggtgccctgactggtcttgagcgcgttgagaagatcacccgcatcaatggccgtggcctggatctgcgcgcagagggtctgaacctcttcctgcaggccactgacgctcctggtgcactgggtaccgttggtaccaagctgggtgctgctggcatcaacatcgaggctgctgcgttgactcaggctgagaagggtgacggcgctgtcctgatcctgcgtgttgagtccgctgtctctgaagagctggaagctgaaatcaacgctgagttgggtgctacttccttccaggttgatcttgactaataaagcttggttgataaaagaaggagaccagtttatggctcaaatcttcaattttagttctggtccggcaatgctaccggcagaggtgcttaaacaggctcaacaggaactgcgcgactggaacggtcttggtacgtcggtgatggaagtgagtcaccgtggcaaagagttcattcaggttgcagaggaagccgagaaggattttcgcgatcttcttaatgtcccctccaactacaaggtattattctgccatggcggtggtcgcggtcagtttgctgcggtaccgctgaatattctcggtgataaaaccaccgcagattatgttgatgccggttactgggcggcaagtgccattaaagaagcgaaaaaatactgcacgcctaatgtctttgacgccaaagtgactgttgatggtctgcgcgcggttaagccaatgcgtgaatggcaactctctgataatgctgcttatatgcattattgcccgaatgaaaccatcgatggtatcgccatcgacgaaacgccagacttcggcgcagatgtggtggtcgccgctgacttctcttcaaccattctttcccgtccgattgacgtcagccgttatggtgtaatttacgctggcgcgcagaaaaatatcggcccggctggcctgacaatcgtcatcgttcgtgaagatttgctgggcaaagcgaatatcgcgtgtccgtcgattctggattattccatcctcaacgataacggctccatgtttaacacgccgccgacatttgcctggtatctatctggtctggtctttaaatggctgaaagcgaacggcggtgtagctgaaatggataaaatcaatcagcaaaaagcagaactgctatatggggtgattgataacagcgatttctaccgcaatgacgtggcgaaagctaaccgttcgcggatgaacgtgccgttccagttggcggacagtgcgcttgacaaattgttccttgaagagtcttttgctgctggccttcatgcactgaaaggtcaccgtgtggtcggcggaatgcgcgcttctatttataacgccatgccgctggaaggcgttaaagcgctgacagacttcatggttgagttcgaacgccgtcacggttgataaaagaaggagaccagtttatgcctaacattacctggtgcgacctgcctgaagatgtctctttatggccgggtctgcctctttcattaagtggtgatgaagtgatgccactggattaccacgcaggtcgtagcggctggctgctgtatggtcgtgggctggataaacaacgtctgacccaataccagagcaaactgggtgcggcgatggtgattgttgccgcctggtgcgtggaagattatcaggtgattcgtctggcaggttcactcaccgcacgggctacacgcctggcccacgaagcgcagctggatgtcgccccgctggggaaaatcccgcacctgcgcacgccgggtttgctggtgatggatatggactccaccgccatccagattgaatgtattgatgaaattgccaaactggccggaacgggcgagatggtggcggaagtaaccgaacgggcgatgcgcggcgaactcgattttaccgccagcctgcgcagccgtgtggcgacgctgaaaggcgctgacgccaatattctgcaacaggtgcgtgaaaatctgccgctgatgccaggcttaacgcaactggtgctcaagctggaaacgctgggctggaaagtggcgattgcctccggcggctttactttctttgctgaatacctgcgcgacaagctgcgcctgaccgccgtggtagccaatgaactggagatcatggacggtaaatttaccggcaatgtgatcggcgacatcgtagacgcgcagtacaaagcgaaaactctgactcgcctcgcgcaggagtatgaaatcccgctggcgcagaccgtggcgattggcgatggagccaatgacctgccgatgatcaaagcggcagggctggggattgcctaccatgccaagccaaaagtgaatgaaaaggcggaagtcaccatccgtcacgctgacctgatgggggtattctgcatcctctcaggcagcctgaatcagaagtgataagctgaggtcgcctcagcggccggcccctgcaggcgccggcgactagtcttggactcctgttgatagatccagtaatgacctcagaactccatctggatttgttcagaacgctcggttgccgccgggcgttttttattggtgagaatccaggggtccccaataattacgatttaaatttgtgtctcaaaatctctgatgttacattgcacaagataaaaatatatcatcatgaacaataaaactgtctgcttacataaacagtaatacaaggggtgttatgagccatattcagcgtgaaacgagctgtagccgtccgcgtctgaacagcaacatggatgcggatctgtatggctataaatgggcgcgtgataacgtgggtcagagcggcgcgaccatttatcgtctgtatggcaaaccggatgcgccggaactgtttctgaaacatggcaaaggcagcgtggcgaacgatgtgaccgatgaaatggtgcgtctgaactggctgaccgaatttatgccgctgccgaccattaaacattttattcgcaccccggatgatgcgtggctgctgaccaccgcgattccgggcaaaaccgcgtttcaggtgctggaagaatatccggatagcggcgaaaacattgtggatgcgctggccgtgtttctgcgtcgtctgcatagcattccggtgtgcaactgcccgtttaacagcgatcgtgtgtttcgtctggcccaggcgcagagccgtatgaacaacggcctggtggatgcgagcgattttgatgatgaacgtaacggctggccggtggaacaggtgtggaaagaaatgcataaactgctgccgtttagcccggatagcgtggtgacccacggcgattttagcctggataacctgattttcgatgaaggcaaactgattggctgcattgatgtgggccgtgtgggcattgcggatcgttatcaggatctggccattctgtggaactgcctgggcgaatttagcccgagcctgcaaaaacgtctgtttcagaaatatggcattgataatccggatatgaacaaactgcaatttcatctgatgctggatgaatttttctaataattaattggaccgttgtccttttccgctgcataaccctgcttcggggtcattatagcgattttttcggtatatccatcctttttcgcacgatatacaggattttgccaaagggttcgtgtagactttccttggtgtatccaacggcgtcagccgggcaggataggtgaagtaggcccacccgcgagcgggtgttccttcttcactgtcccttattcgcacctggcggtgctcaacgggaatcctgctctgcgaggctggccgtaggccggcctcagatccttccgtatttagccagtatgttctctagtgtggttcgttgtttttgcgtgagccatgagaacgaaccattgagatcatacttactttgcatgtcactcaaaaattttgcctcaaaactggtgagctgaatttttgcagttaaagcatcgtgtagtgtttttcttagtccgttatgtaggtaggaatctgatgtaatggttgttggtattttgtcaccattcatttttatctggttgttctcaagttcggttacgagatccatttgtctatctagttcaacttggaaaatcaacgtatcagtcgggcggcctcgcttatcaaccaccaatttcatattgctgtaagtgtttaaatctttacttattggtttcaaaacccattggttaagccttttaaactcatggtagttattttcaagcattaacatgaacttaaattcatcaaggctaatctctatatttgccttgtgagttttcttttgtgttagttcttttaataaccactcataaatcctcatagagtatttgttttcaaaagacttaacatgttccagattatattttatgaatttttttaactg

SEQ ID NO: 25 - DNA, 6785 bp, synthetic construct
  source 1..6785: mol_type = other DNA
ccttccgtatttagccagtatgttctctagtgtggttcgttgtttttgcgtgagccatgagaacgaaccattgagatcatacttactttgcatgtcactcaaaaattttgcctcaaaactggtgagctgaatttttgcagttaaagcatcgtgtagtgtttttcttagtccgttatgtaggtaggaatctgatgtaatggttgttggtattttgtcaccattcatttttatctggttgttctcaagttcggttacgagatccatttgtctatctagttcaacttggaaaatcaacgtatcagtcgggcggcctcgcttatcaaccaccaatttcatattgctgtaagtgtttaaatctttacttattggtttcaaaacccattggttaagccttttaaactcatggtagttattttcaagcattaacatgaacttaaattcatcaaggctaatctctatatttgccttgtgagttttcttttgtgttagttcttttaataaccactcataaatcctcatagagtatttgttttcaaaagacttaacatgttccagattatattttatgaatttttttaactggaaaagataaggcaatatctcttcactaaaaactaattctaatttttcgcttgagaacttggcatagtttgtccactggaaaatctcaaagcctttaaccaaaggattcctgatttccacagttctcgtcatcagctctctggttgctttagctaatacaccataagcattttccctactgatgttcatcatctgagcgtattggttataagtgaacgataccgtccgttctttccttgtagggttttcaatcgtggggttgagtagtgccacacagcataaaattagcttggtttcatgctccgttaagtcatagcgactaatcgctagttcatttgctttgaaaacaactaattcagacatacatctcaattggtctaggtgattttaatcactataccaattgagatgggctagtcaatgataattacatgtccttttcctttgagttgtgggtatctgtaaattctgctagacctttgctggaaaacttgtaaattctgctagaccctctgtaaattccgctagacctttgtgtgttttttttgtttatattcaagtggttataatttatagaataaagaaagaataaaaaaagataaaaagaatagatcccagccctgtgtataactcactactttagtcagttccgcagtattacaaaaggatgtcgcaaacgctgtttgctcctctacaaaacagaccttaaaaccctaaaggcttaagtagcaccctcgcaagctcgggcaaatcgctgaatattccttttgtctccgaccatcaggcacctgagtcgctgtctttttcgtgacattcagttcgctgcgctcacggctctggcagtgaatgggggtaaatggcactacaggcgcggcgcgcccagctgtctagggcggcggatttgtcctactcaggagagcgttcaccgacaaacaacagataaaacgaaaggcccagtctttcgactgagcctttcgttttatttgatgcctttaattaagcggccgcggcgcgcccgtcgacgcgcgcgcggctgaggatacctcagcataggcctttgacaattaatcatccggctcgtataatgtgtggatcttaatcatgctaaggaggattaactttatgagccagaatggccgtccggtagtcctcatcgccgataagcttgcgcagtccactgttgacgcgcttggagatgcagtagaagtccgttgggttgacggacctaaccgcccagaactgcttgatgcagttaaggaagcggacgcactgctcgtgcgttctgctaccactgtcgatgctgaagtcatcgccgctgcccctaacttgaagatcgtcggtcgtgccggcgtgggcttggacaacgttgacatccctgctgccactgaagctggcgtcatggttgctaacgcaccgacctctaatattcactccgcttgtgagcacgcaatttctttgctgctgtctactgctcgccagatccctgctgctgatgcgacgctgcgtgagggcgagtggaagcggtcttctttcaacggtgtggaaattttcggaaaaactgtcggtatcgtcggttttggccacattggtcagttgtttgctcagcgtcttgctgcgtttgagaccaccattgttgcttacgatccttacgctaaccctgctcgtgcggctcagctgaacgttgagttggttgagttggatgagctgatgagccgttctgactttgtcaccattcaccttcctaagaccaaggaaactgctggcatgtttgatgcgcagctccttgctaagtccaagaagggccagatcatcatcaacgctgctcgtggtggccttgttgatgagcaggctttggctgatgcgattgagtccggtcacattcgtggcgctggtttcgatgtgtactccaccgagccttgcactgattctcctttgttcaagttgcctcaggttgttgtgactcctcacttgggtgggtctactgaagaggctcaggatcgtgcgggtactgacgttgctgattctgtgctcaaggcgctggctggcgagttcgtggcggatgctgtgaacgtttccggtggtcgcgtgggcgaagaggttgctgtgtggatggatctggctcgcaagcttggtcttcttgctggcaagcttgtcgacgccgccccagtctccattgaggttgaggctcgaggcgagctttcttccgagcaggtcgatgcacttggtttgtccgctgttcgtggtttgttctccggaattatcgaagagtccgttactttcgtcaacgctcctcgcattgctgaagagcgtggcctggacatctccgtgaagaccaactctgagtctgttactcaccgttccgtcctgcaggtcaaggtcattactggcagcggcgcgagcgcaactgttgttggtgccctgactggtcttgagcgcgttgagaagatcacccgcatcaatggccgtggcctggatctgcgcgcagagggtctgaacctcttcctgcaggccactgacgctcctggtgcactgggtaccgttggtaccaagctgggtgctgctggcatcaacatcgaggctgctgcgttgactcaggctgagaagggtgacggcgctgtcctgatcctgcgtgttgagtccgctgtctctgaagagctggaagctgaaatcaacgctgagttgggtgctacttccttccaggttgatcttgactaataaagcttggttgataaaagaaggagaccagtttatggctcaaatcttcaattttagttctggtccggcaatgctaccggcagaggtgcttaaacaggctcaacaggaactgcgcgactggaacggtcttggtacgtcggtgatggaagtgagtcaccgtggcaaagagttcattcaggttgcagaggaagccgagaaggattttcgcgatcttcttaatgtcccctccaactacaaggtattattctgccatggcggtggtcgcggtcagtttgctgcggtaccgctgaatattctcggtgataaaaccaccgcagattatgttgatgccggttactgggcggcaagtgccattaaagaagcgaaaaaatactgcacgcctaatgtctttgacgccaaagtgactgttgatggtctgcgcgcggttaagccaatgcgtgaatggcaactctctgataatgctgcttatatgcattattgcccgaatgaaaccatcgatggtatcgccatcgacgaaacgccagacttcggcgcagatgtggtggtcgccgctgacttctcttcaaccattctttcccgtccgattgacgtcagccgttatggtgtaatttacgctggcgcgcagaaaaatatcggcccggctggcctgacaatcgtcatcgttcgtgaagatttgctgggcaaagcgaatatcgcgtgtccgtcgattctggattattccatcctcaacgataacggctccatgtttaacacgccgccgacatttgcctggtatctatctggtctggtctttaaatggctgaaagcgaacggcggtgtagctgaaatggataaaatcaatcagcaaaaagcagaactgctatatggggtgattgataacagcgatttctaccgcaatgacgtggcgaaagctaaccgttcgcggatgaacgtgccgttccagttggcggacagtgcgcttgacaaattgttccttgaagagtcttttgctgctggccttcatgcactgaaaggtcaccgtgtggtcggcggaatgcgcgcttctatttataacgccatgccgctggaaggcgttaaagcgctgacagacttcatggttgagttcgaacgccgtcacggttgataaaagaaggagaccagtttatgcctaacattacctggtgcgacctgcctgaagatgtctctttatggccgggtctgcctctttcattaagtggtgatgaagtgatgccactggattaccacgcaggtcgtagcggctggctgctgtatggtcgtgggctggataaacaacgtctgacccaataccagagcaaactgggtgcggcgatggtgattgttgccgcctggtgcgtggaagattatcaggtgattcgtctggcaggttcactcaccgcacgggctacacgcctggcccacgaagcgcagctggatgtcgccccgctggggaaaatcccgcacctgcgcacgccgggtttgctggtgatggatatggactccaccgccatccagattgaatgtattgatgaaattgccaaactggccggaacgggcgagatggtggcggaagtaaccgaacgggcgatgcgcggcgaactcgattttaccgccagcctgcgcagccgtgtggcgacgctgaaaggcgctgacgccaatattctgcaacaggtgcgtgaaaatctgccgctgatgccaggcttaacgcaactggtgctcaagctggaaacgctgggctggaaagtggcgattgcctccggcggctttactttctttgctgaatacctgcgcgacaagctgcgcctgaccgccgtggtagccaatgaactggagatcatggacggtaaatttaccggcaatgtgatcggcgacatcgtagacgcgcagtacaaagcgaaaactctgactcgcctcgcgcaggagtatgaaatcccgctggcgcagaccgtggcgattggcgatggagccaatgacctgccgatgatcaaagcggcagggctggggattgcctaccatgccaagccaaaagtgaatgaaaaggcggaagtcaccatccgtcacgctgacctgatgggggtattctgcatcctctcaggcagcctgaatcagaagtgataagctgaggtcgcctcagcggccggcccctgcaggcgccggcgactagtcttggactcctgttgatagatccagtaatgacctcagaactccatctggatttgttcagaacgctcggttgccgccgggcgttttttattggtgagaatccaggggtccccaataattacgatttaaatttgtgtctcaaaatctctgatgttacattgcacaagataaaaatatatcatcatgaacaataaaactgtctgcttacataaacagtaatacaaggggtgttatgagccatattcagcgtgaaacgagctgtagccgtccgcgtctgaacagcaacatggatgcggatctgtatggctataaatgggcgcgtgataacgtgggtcagagcggcgcgaccatttatcgtctgtatggcaaaccggatgcgccggaactgtttctgaaacatggcaaaggcagcgtggcgaacgatgtgaccgatgaaatggtgcgtctgaactggctgaccgaatttatgccgctgccgaccattaaacattttattcgcaccccggatgatgcgtggctgctgaccaccgcgattccgggcaaaaccgcgtttcaggtgctggaagaatatccggatagcggcgaaaacattgtggatgcgctggccgtgtttctgcgtcgtctgcatagcattccggtgtgcaactgcccgtttaacagcgatcgtgtgtttcgtctggcccaggcgcagagccgtatgaacaacggcctggtggatgcgagcgattttgatgatgaacgtaacggctggccggtggaacaggtgtggaaagaaatgcataaactgctgccgtttagcccggatagcgtggtgacccacggcgattttagcctggataacctgattttcgatgaaggcaaactgattggctgcattgatgtgggccgtgtgggcattgcggatcgttatcaggatctggccattctgtggaactgcctgggcgaatttagcccgagcctgcaaaaacgtctgtttcagaaatatggcattgataatccggatatgaacaaactgcaatttcatctgatgctggatgaatttttctaataattaattggaccgttgtccttttccgctgcataaccctgcttcggggtcattatagcgattttttcggtatatccatcctttttcgcacgatatacaggattttgccaaagggttcgtgtagactttccttggtgtatccaacggcgtcagccgggcaggataggtgaagtaggcccacccgcgagcgggtgttccttcttcactgtcccttattcgcacctggcggtgctcaacgggaatcctgctctgcgaggctggccgtaggccggcctcagat

SEQ ID NO: 26 - DNA, 6785 bp, synthetic construct
  source 1..6785: mol_type = other DNA
atttttgcagttaaagcatcgtgtagtgtttttcttagtccgttatgtaggtaggaatctgatgtaatggttgttggtattttgtcaccattcatttttatctggttgttctcaagttcggttacgagatccatttgtctatctagttcaacttggaaaatcaacgtatcagtcgggcggcctcgcttatcaaccaccaatttcatattgctgtaagtgtttaaatctttacttattggtttcaaaacccattggttaagccttttaaactcatggtagttattttcaagcattaacatgaacttaaattcatcaaggctaatctctatatttgccttgtgagttttcttttgtgttagttcttttaataaccactcataaatcctcatagagtatttgttttcaaaagacttaacatgttccagattatattttatgaatttttttaactggaaaagataaggcaatatctcttcactaaaaactaattctaatttttcgcttgagaacttggcatagtttgtccactggaaaatctcaaagcctttaaccaaaggattcctgatttccacagttctcgtcatcagctctctggttgctttagctaatacaccataagcattttccctactgatgttcatcatctgagcgtattggttataagtgaacgataccgtccgttctttccttgtagggttttcaatcgtggggttgagtagtgccacacagcataaaattagcttggtttcatgctccgttaagtcatagcgactaatcgctagttcatttgctttgaaaacaactaattcagacatacatctcaattggtctaggtgattttaatcactataccaattgagatgggctagtcaatgataattacatgtccttttcctttgagttgtgggtatctgtaaattctgctagacctttgctggaaaacttgtaaattctgctagaccctctgtaaattccgctagacctttgtgtgttttttttgtttatattcaagtggttataatttatagaataaagaaagaataaaaaaagataaaaagaatagatcccagccctgtgtataactcactactttagtcagttccgcagtattacaaaaggatgtcgcaaacgctgtttgctcctctacaaaacagaccttaaaaccctaaaggcttaagtagcaccctcgcaagctcgggcaaatcgctgaatattccttttgtctccgaccatcaggcacctgagtcgctgtctttttcgtgacattcagttcgctgcgctcacggctctggcagtgaatgggggtaaatggcactacaggcgcggcgcgcccagctgtctagggcggcggatttgtcctactcaggagagcgttcaccgacaaacaacagataaaacgaaaggcccagtctttcgactgagcctttcgttttatttgatgcctttaattaagcggccgcggcgcgcccgtcgacgcgcgcgcggctgaggatacctcagcataggcctttgacaattaatcatccggctcttagtgtttgtggatcttaatcatgctaaggaggattaactttatgagccagaatggccgtccggtagtcctcatcgccgataagcttgcgcagtccactgttgacgcgcttggagatgcagtagaagtccgttgggttgacggacctaaccgcccagaactgcttgatgcagttaaggaagcggacgcactgctcgtgcgttctgctaccactgtcgatgctgaagtcatcgccgctgcccctaacttgaagatcgtcggtcgtgccggcgtgggcttggacaacgttgacatccctgctgccactgaagctggcgtcatggttgctaacgcaccgacctctaatattcactccgcttgtgagcacgcaatttctttgctgctgtctactgctcgccagatccctgctgctgatgcgacgctgcgtgagggcgagtggaagcggtcttctttcaacggtgtggaaattttcggaaaaactgtcggtatcgtcggttttggccacattggtcagttgtttgctcagcgtcttgctgcgtttgagaccaccattgttgcttacgatccttacgctaaccctgctcgtgcggctcagctgaacgttgagttggttgagttggatgagctgatgagccgttctgactttgtcaccattcaccttcctaagaccaaggaaactgctggcatgtttgatgcgcagctccttgctaagtccaagaagggccagatcatcatcaacgctgctcgtggtggccttgttgatgagcaggctttggctgatgcgattgagtccggtcacattcgtggcgctggtttcgatgtgtactccaccgagccttgcactgattctcctttgttcaagttgcctcaggttgttgtgactcctcacttgggtgggtctactgaagaggctcaggatcgtgcgggtactgacgttgctgattctgtgctcaaggcgctggctggcgagttcgtggcggatgctgtgaacgtttccggtggtcgcgtgggcgaagaggttgctgtgtggatggatctggctcgcaagcttggtcttcttgctggcaagcttgtcgacgccgccccagtctccattgaggttgaggctcgaggcgagctttcttccgagcaggtcgatgcacttggtttgtccgctgttcgtggtttgttctccggaattatcgaagagtccgttactttcgtcaacgctcctcgcattgctgaagagcgtggcctggacatctccgtgaagaccaactctgagtctgttactcaccgttccgtcctgcaggtcaaggtcattactggcagcggcgcgagcgcaactgttgttggtgccctgactggtcttgagcgcgttgagaagatcacccgcatcaatggccgtggcctggatctgcgcgcagagggtctgaacctcttcctgcaggccactgacgctcctggtgcactgggtaccgttggtaccaagctgggtgctgctggcatcaacatcgaggctgctgcgttgactcaggctgagaagggtgacggcgctgtcctgatcctgcgtgttgagtccgctgtctctgaagagctggaagctgaaatcaacgctgagttgggtgctacttccttccaggttgatcttgactaataaagcttggttgataaaagaaggagaccagtttatggctcaaatcttcaattttagttctggtccggcaatgctaccggcagaggtgcttaaacaggctcaacaggaactgcgcgactggaacggtcttggtacgtcggtgatggaagtgagtcaccgtggcaaagagttcattcaggttgcagaggaagccgagaaggattttcgcgatcttcttaatgtcccctccaactacaaggtattattctgccatggcggtggtcgcggtcagtttgctgcggtaccgctgaatattctcggtgataaaaccaccgcagattatgttgatgccggttactgggcggcaagtgccattaaagaagcgaaaaaatactgcacgcctaatgtctttgacgccaaagtgactgttgatggtctgcgcgcggttaagccaatgcgtgaatggcaactctctgataatgctgcttatatgcattattgcccgaatgaaaccatcgatggtatcgccatcgacgaaacgccagacttcggcgcagatgtggtggtcgccgctgacttctcttcaaccattctttcccgtccgattgacgtcagccgttatggtgtaatttacgctggcgcgcagaaaaatatcggcccggctggcctgacaatcgtcatcgttcgtgaagatttgctgggcaaagcgaatatcgcgtgtccgtcgattctggattattccatcctcaacgataacggctccatgtttaacacgccgccgacatttgcctggtatctatctggtctggtctttaaatggctgaaagcgaacggcggtgtagctgaaatggataaaatcaatcagcaaaaagcagaactgctatatggggtgattgataacagcgatttctaccgcaatgacgtggcgaaagctaaccgttcgcggatgaacgtgccgttccagttggcggacagtgcgcttgacaaattgttccttgaagagtcttttgctgctggccttcatgcactgaaaggtcaccgtgtggtcggcggaatgcgcgcttctatttataacgccatgccgctggaaggcgttaaagcgctgacagacttcatggttgagttcgaacgccgtcacggttgataaaagaaggagaccagtttatgcctaacattacctggtgcgacctgcctgaagatgtctctttatggccgggtctgcctctttcattaagtggtgatgaagtgatgccactggattaccacgcaggtcgtagcggctggctgctgtatggtcgtgggctggataaacaacgtctgacccaataccagagcaaactgggtgcggcgatggtgattgttgccgcctggtgcgtggaagattatcaggtgattcgtctggcaggttcactcaccgcacgggctacacgcctggcccacgaagcgcagctggatgtcgccccgctggggaaaatcccgcacctgcgcacgccgggtttgctggtgatggatatggactccaccgccatccagattgaatgtattgatgaaattgccaaactggccggaacgggcgagatggtggcggaagtaaccgaacgggcgatgcgcggcgaactcgattttaccgccagcctgcgcagccgtgtggcgacgctgaaaggcgctgacgccaatattctgcaacaggtgcgtgaaaatctgccgctgatgccaggcttaacgcaactggtgctcaagctggaaacgctgggctggaaagtggcgattgcctccggcggctttactttctttgctgaatacctgcgcgacaagctgcgcctgaccgccgtggtagccaatgaactggagatcatggacggtaaatttaccggcaatgtgatcggcgacatcgtagacgcgcagtacaaagcgaaaactctgactcgcctcgcgcaggagtatgaaatcccgctggcgcagaccgtggcgattggcgatggagccaatgacctgccgatgatcaaagcggcagggctggggattgcctaccatgccaagccaaaagtgaatgaaaaggcggaagtcaccatccgtcacgctgacctgatgggggtattctgcatcctctcaggcagcctgaatcagaagtgataagctgaggtcgcctcagcggccggcccctgcaggcgccggcgactagtcttggactcctgttgatagatccagtaatgacctcagaactccatctggatttgttcagaacgctcggttgccgccgggcgttttttattggtgagaatccaggggtccccaataattacgatttaaatttgtgtctcaaaatctctgatgttacattgcacaagataaaaatatatcatcatgaacaataaaactgtctgcttacataaacagtaatacaaggggtgttatgagccatattcagcgtgaaacgagctgtagccgtccgcgtctgaacagcaacatggatgcggatctgtatggctataaatgggcgcgtgataacgtgggtcagagcggcgcgaccatttatcgtctgtatggcaaaccggatgcgccggaactgtttctgaaacatggcaaaggcagcgtggcgaacgatgtgaccgatgaaatggtgcgtctgaactggctgaccgaatttatgccgctgccgaccattaaacattttattcgcaccccggatgatgcgtggctgctgaccaccgcgattccgggcaaaaccgcgtttcaggtgctggaagaatatccggatagcggcgaaaacattgtggatgcgctggccgtgtttctgcgtcgtctgcatagcattccggtgtgcaactgcccgtttaacagcgatcgtgtgtttcgtctggcccaggcgcagagccgtatgaacaacggcctggtggatgcgagcgattttgatgatgaacgtaacggctggccggtggaacaggtgtggaaagaaatgcataaactgctgccgtttagcccggatagcgtggtgacccacggcgattttagcctggataacctgattttcgatgaaggcaaactgattggctgcattgatgtgggccgtgtgggcattgcggatcgttatcaggatctggccattctgtggaactgcctgggcgaatttagcccgagcctgcaaaaacgtctgtttcagaaatatggcattgataatccggatatgaacaaactgcaatttcatctgatgctggatgaatttttctaataattaattggaccgttgtccttttccgctgcataaccctgcttcggggtcattatagcgattttttcggtatatccatcctttttcgcacgatatacaggattttgccaaagggttcgtgtagactttccttggtgtatccaacggcgtcagccgggcaggataggtgaagtaggcccacccgcgagcgggtgttccttcttcactgtcccttattcgcacctggcggtgctcaacgggaatcctgctctgcgaggctggccgtaggccggcctcagatccttccgtatttagccagtatgttctctagtgtggttcgttgtttttgcgtgagccatgagaacgaaccattgagatcatacttactttgcatgtcactcaaaaattttgcctcaaaactggtgagctga

SEQ ID NO: 27 - DNA, 6784 bp, synthetic construct
  source 1..6784: mol_type = other DNA
ccgtatttagccagtatgttctctagtgtggttcgttgtttttgcgtgagccatgagaacgaaccattgagatcatacttactttgcatgtcactcaaaaattttgcctcaaaactggtgagctgaatttttgcagttaaagcatcgtgtagtgtttttcttagtccgttatgtaggtaggaatctgatgtaatggttgttggtattttgtcaccattcatttttatctggttgttctcaagttcggttacgagatccatttgtctatctagttcaacttggaaaatcaacgtatcagtcgggcggcctcgcttatcaaccaccaatttcatattgctgtaagtgtttaaatctttacttattggtttcaaaacccattggttaagccttttaaactcatggtagttattttcaagcattaacatgaacttaaattcatcaaggctaatctctatatttgccttgtgagttttcttttgtgttagttcttttaataaccactcataaatcctcatagagtatttgttttcaaaagacttaacatgttccagattatattttatgaatttttttaactggaaaagataaggcaatatctcttcactaaaaactaattctaatttttcgcttgagaacttggcatagtttgtccactggaaaatctcaaagcctttaaccaaaggattcctgatttccacagttctcgtcatcagctctctggttgctttagctaatacaccataagcattttccctactgatgttcatcatctgagcgtattggttataagtgaacgataccgtccgttctttccttgtagggttttcaatcgtggggttgagtagtgccacacagcataaaattagcttggtttcatgctccgttaagtcatagcgactaatcgctagttcatttgctttgaaaacaactaattcagacatacatctcaattggtctaggtgattttaatcactataccaattgagatgggctagtcaatgataattacatgtccttttcctttgagttgtgggtatctgtaaattctgctagacctttgctggaaaacttgtaaattctgctagaccctctgtaaattccgctagacctttgtgtgttttttttgtttatattcaagtggttataatttatagaataaagaaagaataaaaaaagataaaaagaatagatcccagccctgtgtataactcactactttagtcagttccgcagtattacaaaaggatgtcgcaaacgctgtttgctcctctacaaaacagaccttaaaaccctaaaggcttaagtagcaccctcgcaagctcgggcaaatcgctgaatattccttttgtctccgaccatcaggcacctgagtcgctgtctttttcgtgacattcagttcgctgcgctcacggctctggcagtgaatgggggtaaatggcactacaggcgcggcgcgcccagctgtctagggcggcggatttgtcctactcaggagagcgttcaccgacaaacaacagataaaacgaaaggcccagtctttcgactgagcctttcgttttatttgatgcctttaattaagcggccgcggcgcgcccgtcgacgcgcgcgcggctgaggatacctcagcataggcctttgcctcttaatcatcggctcgtataatgtgtggatcttaatcatgctaaggaggattaactttatgagccagaatggccgtccggtagtcctcatcgccgataagcttgcgcagtccactgttgacgcgcttggagatgcagtagaagtccgttgggttgacggacctaaccgcccagaactgcttgatgcagttaaggaagcggacgcactgctcgtgcgttctgctaccactgtcgatgctgaagtcatcgccgctgcccctaacttgaagatcgtcggtcgtgccggcgtgggcttggacaacgttgacatccctgctgccactgaagctggcgtcatggttgctaacgcaccgacctctaatattcactccgcttgtgagcacgcaatttctttgctgctgtctactgctcgccagatccctgctgctgatgcgacgctgcgtgagggcgagtggaagcggtcttctttcaacggtgtggaaattttcggaaaaactgtcggtatcgtcggttttggccacattggtcagttgtttgctcagcgtcttgctgcgtttgagaccaccattgttgcttacgatccttacgctaaccctgctcgtgcggctcagctgaacgttgagttggttgagttggatgagctgatgagccgttctgactttgtcaccattcaccttcctaagaccaaggaaactgctggcatgtttgatgcgcagctccttgctaagtccaagaagggccagatcatcatcaacgctgctcgtggtggccttgttgatgagcaggctttggctgatgcgattgagtccggtcacattcgtggcgctggtttcgatgtgtactccaccgagccttgcactgattctcctttgttcaagttgcctcaggttgttgtgactcctcacttgggtgggtctactgaagaggctcaggatcgtgcgggtactgacgttgctgattctgtgctcaaggcgctggctggcgagttcgtggcggatgctgtgaacgtttccggtggtcgcgtgggcgaagaggttgctgtgtggatggatctggctcgcaagcttggtcttcttgctggcaagcttgtcgacgccgccccagtctccattgaggttgaggctcgaggcgagctttcttccgagcaggtcgatgcacttggtttgtccgctgttcgtggtttgttctccggaattatcgaagagtccgttactttcgtcaacgctcctcgcattgctgaagagcgtggcctggacatctccgtgaagaccaactctgagtctgttactcaccgttccgtcctgcaggtcaaggtcattactggcagcggcgcgagcgcaactgttgttggtgccctgactggtcttgagcgcgttgagaagatcacccgcatcaatggccgtggcctggatctgcgcgcagagggtctgaacctcttcctgcaggccactgacgctcctggtgcactgggtaccgttggtaccaagctgggtgctgctggcatcaacatcgaggctgctgcgttgactcaggctgagaagggtgacggcgctgtcctgatcctgcgtgttgagtccgctgtctctgaagagctggaagctgaaatcaacgctgagttgggtgctacttccttccaggttgatcttgactaataaagcttggttgataaaagaaggagaccagtttatggctcaaatcttcaattttagttctggtccggcaatgctaccggcagaggtgcttaaacaggctcaacaggaactgcgcgactggaacggtcttggtacgtcggtgatggaagtgagtcaccgtggcaaagagttcattcaggttgcagaggaagccgagaaggattttcgcgatcttcttaatgtcccctccaactacaaggtattattctgccatggcggtggtcgcggtcagtttgctgcggtaccgctgaatattctcggtgataaaaccaccgcagattatgttgatgccggttactgggcggcaagtgccattaaagaagcgaaaaaatactgcacgcctaatgtctttgacgccaaagtgactgttgatggtctgcgcgcggttaagccaatgcgtgaatggcaactctctgataatgctgcttatatgcattattgcccgaatgaaaccatcgatggtatcgccatcgacgaaacgccagacttcggcgcagatgtggtggtcgccgctgacttctcttcaaccattctttcccgtccgattgacgtcagccgttatggtgtaatttacgctggcgcgcagaaaaatatcggcccggctggcctgacaatcgtcatcgttcgtgaagatttgctgggcaaagcgaatatcgcgtgtccgtcgattctggattattccatcctcaacgataacggctccatgtttaacacgccgccgacatttgcctggtatctatctggtctggtctttaaatggctgaaagcgaacggcggtgtagctgaaatggataaaatcaatcagcaaaaagcagaactgctatatggggtgattgataacagcgatttctaccgcaatgacgtggcgaaagctaaccgttcgcggatgaacgtgccgttccagttggcggacagtgcgcttgacaaattgttccttgaagagtcttttgctgctggccttcatgcactgaaaggtcaccgtgtggtcggcggaatgcgcgcttctatttataacgccatgccgctggaaggcgttaaagcgctgacagacttcatggttgagttcgaacgccgtcacggttgataaaagaaggagaccagtttatgcctaacattacctggtgcgacctgcctgaagatgtctctttatggccgggtctgcctctttcattaagtggtgatgaagtgatgccactggattaccacgcaggtcgtagcggctggctgctgtatggtcgtgggctggataaacaacgtctgacccaataccagagcaaactgggtgcggcgatggtgattgttgccgcctggtgcgtggaagattatcaggtgattcgtctggcaggttcactcaccgcacgggctacacgcctggcccacgaagcgcagctggatgtcgccccgctggggaaaatcccgcacctgcgcacgccgggtttgctggtgatggatatggactccaccgccatccagattgaatgtattgatgaaattgccaaactggccggaacgggcgagatggtggcggaagtaaccgaacgggcgatgcgcggcgaactcgattttaccgccagcctgcgcagccgtgtggcgacgctgaaaggcgctgacgccaatattctgcaacaggtgcgtgaaaatctgccgctgatgccaggcttaacgcaactggtgctcaagctggaaacgctgggctggaaagtggcgattgcctccggcggctttactttctttgctgaatacctgcgcgacaagctgcgcctgaccgccgtggtagccaatgaactggagatcatggacggtaaatttaccggcaatgtgatcggcgacatcgtagacgcgcagtacaaagcgaaaactctgactcgcctcgcgcaggagtatgaaatcccgctggcgcagaccgtggcgattggcgatggagccaatgacctgccgatgatcaaagcggcagggctggggattgcctaccatgccaagccaaaagtgaatgaaaaggcggaagtcaccatccgtcacgctgacctgatgggggtattctgcatcctctcaggcagcctgaatcagaagtgataagctgaggtcgcctcagcggccggcccctgcaggcgccggcgactagtcttggactcctgttgatagatccagtaatgacctcagaactccatctggatttgttcagaacgctcggttgccgccgggcgttttttattggtgagaatccaggggtccccaataattacgatttaaatttgtgtctcaaaatctctgatgttacattgcacaagataaaaatatatcatcatgaacaataaaactgtctgcttacataaacagtaatacaaggggtgttatgagccatattcagcgtgaaacgagctgtagccgtccgcgtctgaacagcaacatggatgcggatctgtatggctataaatgggcgcgtgataacgtgggtcagagcggcgcgaccatttatcgtctgtatggcaaaccggatgcgccggaactgtttctgaaacatggcaaaggcagcgtggcgaacgatgtgaccgatgaaatggtgcgtctgaactggctgaccgaatttatgccgctgccgaccattaaacattttattcgcaccccggatgatgcgtggctgctgaccaccgcgattccgggcaaaaccgcgtttcaggtgctggaagaatatccggatagcggcgaaaacattgtggatgcgctggccgtgtttctgcgtcgtctgcatagcattccggtgtgcaactgcccgtttaacagcgatcgtgtgtttcgtctggcccaggcgcagagccgtatgaacaacggcctggtggatgcgagcgattttgatgatgaacgtaacggctggccggtggaacaggtgtggaaagaaatgcataaactgctgccgtttagcccggatagcgtggtgacccacggcgattttagcctggataacctgattttcgatgaaggcaaactgattggctgcattgatgtgggccgtgtgggcattgcggatcgttatcaggatctggccattctgtggaactgcctgggcgaatttagcccgagcctgcaaaaacgtctgtttcagaaatatggcattgataatccggatatgaacaaactgcaatttcatctgatgctggatgaatttttctaataattaattggaccgttgtccttttccgctgcataaccctgcttcggggtcattatagcgattttttcggtatatccatcctttttcgcacgatatacaggattttgccaaagggttcgtgtagactttccttggtgtatccaacggcgtcagccgggcaggataggtgaagtaggcccacccgcgagcgggtgttccttcttcactgtcccttattcgcacctggcggtgctcaacgggaatcctgctctgcgaggctggccgtaggccggcctcagatcctt

SEQ ID NO: 28 - DNA, 6784 bp, synthetic construct
  source 1..6784: mol_type = other DNA
gccatgagaacgaaccattgagatcatacttactttgcatgtcactcaaaaattttgcctcaaaactggtgagctgaatttttgcagttaaagcatcgtgtagtgtttttcttagtccgttatgtaggtaggaatctgatgtaatggttgttggtattttgtcaccattcatttttatctggttgttctcaagttcggttacgagatccatttgtctatctagttcaacttggaaaatcaacgtatcagtcgggcggcctcgcttatcaaccaccaatttcatattgctgtaagtgtttaaatctttacttattggtttcaaaacccattggttaagccttttaaactcatggtagttattttcaagcattaacatgaacttaaattcatcaaggctaatctctatatttgccttgtgagttttcttttgtgttagttcttttaataaccactcataaatcctcatagagtatttgttttcaaaagacttaacatgttccagattatattttatgaatttttttaactggaaaagataaggcaatatctcttcactaaaaactaattctaatttttcgcttgagaacttggcatagtttgtccactggaaaatctcaaagcctttaaccaaaggattcctgatttccacagttctcgtcatcagctctctggttgctttagctaatacaccataagcattttccctactgatgttcatcatctgagcgtattggttataagtgaacgataccgtccgttctttccttgtagggttttcaatcgtggggttgagtagtgccacacagcataaaattagcttggtttcatgctccgttaagtcatagcgactaatcgctagttcatttgctttgaaaacaactaattcagacatacatctcaattggtctaggtgattttaatcactataccaattgagatgggctagtcaatgataattacatgtccttttcctttgagttgtgggtatctgtaaattctgctagacctttgctggaaaacttgtaaattctgctagaccctctgtaaattccgctagacctttgtgtgttttttttgtttatattcaagtggttataatttatagaataaagaaagaataaaaaaagataaaaagaatagatcccagccctgtgtataactcactactttagtcagttccgcagtattacaaaaggatgtcgcaaacgctgtttgctcctctacaaaacagaccttaaaaccctaaaggcttaagtagcaccctcgcaagctcgggcaaatcgctgaatattccttttgtctccgaccatcaggcacctgagtcgctgtctttttcgtgacattcagttcgctgcgctcacggctctggcagtgaatgggggtaaatggcactacaggcgcggcgcgcccagctgtctagggcggcggatttgtcctactcaggagagcgttcaccgacaaacaacagataaaacgaaaggcccagtctttcgactgagcctttcgttttatttgatgcctttaattaagcggccgcggcgcgcccgtcgacgcgcgcgcggctgaggatacctcagcataggcctctgacagctagctcagtcctaggtataatgctagctcttaatcatgctaaggaggattaactttatgagccagaatggccgtccggtagtcctcatcgccgataagcttgcgcagtccactgttgacgcgcttggagatgcagtagaagtccgttgggttgacggacctaaccgcccagaactgcttgatgcagttaaggaagcggacgcactgctcgtgcgttctgctaccactgtcgatgctgaagtcatcgccgctgcccctaacttgaagatcgtcggtcgtgccggcgtgggcttggacaacgttgacatccctgctgccactgaagctggcgtcatggttgctaacgcaccgacctctaatattcactccgcttgtgagcacgcaatttctttgctgctgtctactgctcgccagatccctgctgctgatgcgacgctgcgtgagggcgagtggaagcggtcttctttcaacggtgtggaaattttcggaaaaactgtcggtatcgtcggttttggccacattggtcagttgtttgctcagcgtcttgctgcgtttgagaccaccattgttgcttacgatccttacgctaaccctgctcgtgcggctcagctgaacgttgagttggttgagttggatgagctgatgagccgttctgactttgtcaccattcaccttcctaagaccaaggaaactgctggcatgtttgatgcgcagctccttgctaagtccaagaagggccagatcatcatcaacgctgctcgtggtggccttgttgatgagcaggctttggctgatgcgattgagtccggtcacattcgtggcgctggtttcgatgtgtactccaccgagccttgcactgattctcctttgttcaagttgcctcaggttgttgtgactcctcacttgggtgggtctactgaagaggctcaggatcgtgcgggtactgacgttgctgattctgtgctcaaggcgctggctggcgagttcgtggcggatgctgtgaacgtttccggtggtcgcgtgggcgaagaggttgctgtgtggatggatctggctcgcaagcttggtcttcttgctggcaagcttgtcgacgccgccccagtctccattgaggttgaggctcgaggcgagctttcttccgagcaggtcgatgcacttggtttgtccgctgttcgtggtttgttctccggaattatcgaagagtccgttactttcgtcaacgctcctcgcattgctgaagagcgtggcctggacatctccgtgaagaccaactctgagtctgttactcaccgttccgtcctgcaggtcaaggtcattactggcagcggcgcgagcgcaactgttgttggtgccctgactggtcttgagcgcgttgagaagatcacccgcatcaatggccgtggcctggatctgcgcgcagagggtctgaacctcttcctgcaggccactgacgctcctggtgcactgggtaccgttggtaccaagctgggtgctgctggcatcaacatcgaggctgctgcgttgactcaggctgagaagggtgacggcgctgtcctgatcctgcgtgttgagtccgctgtctctgaagagctggaagctgaaatcaacgctgagttgggtgctacttccttccaggttgatcttgactaataaagcttggttgataaaagaaggagaccagtttatggctcaaatcttcaattttagttctggtccggcaatgctaccggcagaggtgcttaaacaggctcaacaggaactgcgcgactggaacggtcttggtacgtcggtgatggaagtgagtcaccgtggcaaagagttcattcaggttgcagaggaagccgagaaggattttcgcgatcttcttaatgtcccctccaactacaaggtattattctgccatggcggtggtcgcggtcagtttgctgcggtaccgctgaatattctcggtgataaaaccaccgcagattatgttgatgccggttactgggcggcaagtgccattaaagaagcgaaaaaatactgcacgcctaatgtctttgacgccaaagtgactgttgatggtctgcgcgcggttaagccaatgcgtgaatggcaactctctgataatgctgcttatatgcattattgcccgaatgaaaccatcgatggtatcgccatcgacgaaacgccagacttcggcgcagatgtggtggtcgccgctgacttctcttcaaccattctttcccgtccgattgacgtcagccgttatggtgtaatttacgctggcgcgcagaaaaatatcggcccggctggcctgacaatcgtcatcgttcgtgaagatttgctgggcaaagcgaatatcgcgtgtccgtcgattctggattattccatcctcaacgataacggctccatgtttaacacgccgccgacatttgcctggtatctatctggtctggtctttaaatggctgaaagcgaacggcggtgtagctgaaatggataaaatcaatcagcaaaaagcagaactgctatatggggtgattgataacagcgatttctaccgcaatgacgtggcgaaagctaaccgttcgcggatgaacgtgccgttccagttggcggacagtgcgcttgacaaattgttccttgaagagtcttttgctgctggccttcatgcactgaaaggtcaccgtgtggtcggcggaatgcgcgcttctatttataacgccatgccgctggaaggcgttaaagcgctgacagacttcatggttgagttcgaacgccgtcacggttgataaaagaaggagaccagtttatgcctaacattacctggtgcgacctgcctgaagatgtctctttatggccgggtctgcctctttcattaagtggtgatgaagtgatgccactggattaccacgcaggtcgtagcggctggctgctgtatggtcgtgggctggataaacaacgtctgacccaataccagagcaaactgggtgcggcgatggtgattgttgccgcctggtgcgtggaagattatcaggtgattcgtctggcaggttcactcaccgcacgggctacacgcctggcccacgaagcgcagctggatgtcgccccgctggggaaaatcccgcacctgcgcacgccgggtttgctggtgatggatatggactccaccgccatccagattgaatgtattgatgaaattgccaaactggccggaacgggcgagatggtggcggaagtaaccgaacgggcgatgcgcggcgaactcgattttaccgccagcctgcgcagccgtgtggcgacgctgaaaggcgctgacgccaatattctgcaacaggtgcgtgaaaatctgccgctgatgccaggcttaacgcaactggtgctcaagctggaaacgctgggctggaaagtggcgattgcctccggcggctttactttctttgctgaatacctgcgcgacaagctgcgcctgaccgccgtggtagccaatgaactggagatcatggacggtaaatttaccggcaatgtgatcggcgacatcgtagacgcgcagtacaaagcgaaaactctgactcgcctcgcgcaggagtatgaaatcccgctggcgcagaccgtggcgattggcgatggagccaatgacctgccgatgatcaaagcggcagggctggggattgcctaccatgccaagccaaaagtgaatgaaaaggcggaagtcaccatccgtcacgctgacctgatgggggtattctgcatcctctcaggcagcctgaatcagaagtgataagctgaggtcgcctcagcggccggcccctgcaggcgccggcgactagtcttggactcctgttgatagatccagtaatgacctcagaactccatctggatttgttcagaacgctcggttgccgccgggcgttttttattggtgagaatccaggggtccccaataattacgatttaaatttgtgtctcaaaatctctgatgttacattgcacaagataaaaatatatcatcatgaacaataaaactgtctgcttacataaacagtaatacaaggggtgttatgagccatattcagcgtgaaacgagctgtagccgtccgcgtctgaacagcaacatggatgcggatctgtatggctataaatgggcgcgtgataacgtgggtcagagcggcgcgaccatttatcgtctgtatggcaaaccggatgcgccggaactgtttctgaaacatggcaaaggcagcgtggcgaacgatgtgaccgatgaaatggtgcgtctgaactggctgaccgaatttatgccgctgccgaccattaaacattttattcgcaccccggatgatgcgtggctgctgaccaccgcgattccgggcaaaaccgcgtttcaggtgctggaagaatatccggatagcggcgaaaacattgtggatgcgctggccgtgtttctgcgtcgtctgcatagcattccggtgtgcaactgcccgtttaacagcgatcgtgtgtttcgtctggcccaggcgcagagccgtatgaacaacggcctggtggatgcgagcgattttgatgatgaacgtaacggctggccggtggaacaggtgtggaaagaaatgcataaactgctgccgtttagcccggatagcgtggtgacccacggcgattttagcctggataacctgattttcgatgaaggcaaactgattggctgcattgatgtgggccgtgtgggcattgcggatcgttatcaggatctggccattctgtggaactgcctgggcgaatttagcccgagcctgcaaaaacgtctgtttcagaaatatggcattgataatccggatatgaacaaactgcaatttcatctgatgctggatgaatttttctaataattaattggaccgttgtccttttccgctgcataaccctgcttcggggtcattatagcgattttttcggtatatccatcctttttcgcacgatatacaggattttgccaaagggttcgtgtagactttccttggtgtatccaacggcgtcagccgggcaggataggtgaagtaggcccacccgcgagcgggtgttccttcttcactgtcccttattcgcacctggcggtgctcaacgggaatcctgctctgcgaggctggccgtaggccggcctcagatccttccgtatttagccagtatgttctctagtgtggttcgttgtttttgcgtga

SEQ ID NO: 29 - DNA, 6784 bp, synthetic construct
  source 1..6784: mol_type = other DNA
ttctctagtgtggttcgttgtttttgcgtgagccatgagaacgaaccattgagatcatacttactttgcatgtcactcaaaaattttgcctcaaaactggtgagctgaatttttgcagttaaagcatcgtgtagtgtttttcttagtccgttatgtaggtaggaatctgatgtaatggttgttggtattttgtcaccattcatttttatctggttgttctcaagttcggttacgagatccatttgtctatctagttcaacttggaaaatcaacgtatcagtcgggcggcctcgcttatcaaccaccaatttcatattgctgtaagtgtttaaatctttacttattggtttcaaaacccattggttaagccttttaaactcatggtagttattttcaagcattaacatgaacttaaattcatcaaggctaatctctatatttgccttgtgagttttcttttgtgttagttcttttaataaccactcataaatcctcatagagtatttgttttcaaaagacttaacatgttccagattatattttatgaatttttttaactggaaaagataaggcaatatctcttcactaaaaactaattctaatttttcgcttgagaacttggcatagtttgtccactggaaaatctcaaagcctttaaccaaaggattcctgatttccacagttctcgtcatcagctctctggttgctttagctaatacaccataagcattttccctactgatgttcatcatctgagcgtattggttataagtgaacgataccgtccgttctttccttgtagggttttcaatcgtggggttgagtagtgccacacagcataaaattagcttggtttcatgctccgttaagtcatagcgactaatcgctagttcatttgctttgaaaacaactaattcagacatacatctcaattggtctaggtgattttaatcactataccaattgagatgggctagtcaatgataattacatgtccttttcctttgagttgtgggtatctgtaaattctgctagacctttgctggaaaacttgtaaattctgctagaccctctgtaaattccgctagacctttgtgtgttttttttgtttatattcaagtggttataatttatagaataaagaaagaataaaaaaagataaaaagaatagatcccagccctgtgtataactcactactttagtcagttccgcagtattacaaaaggatgtcgcaaacgctgtttgctcctctacaaaacagaccttaaaaccctaaaggcttaagtagcaccctcgcaagctcgggcaaatcgctgaatattccttttgtctccgaccatcaggcacctgagtcgctgtctttttcgtgacattcagttcgctgcgctcacggctctggcagtgaatgggggtaaatggcactacaggcgcggcgcgcccagctgtctagggcggcggatttgtcctactcaggagagcgttcaccgacaaacaacagataaaacgaaaggcccagtctttcgactgagcctttcgttttatttgatgcctttaattaagcggccgcggcgcgcccgtcgacgcgcgcgcggctgaggatacctcagcataggcctttgacagctagctcagtcctaggtattgtgctagctcttaatcatgctaaggaggattaactttatgagccagaatggccgtccggtagtcctcatcgccgataagcttgcgcagtccactgttgacgcgcttggagatgcagtagaagtccgttgggttgacggacctaaccgcccagaactgcttgatgcagttaaggaagcggacgcactgctcgtgcgttctgctaccactgtcgatgctgaagtcatcgccgctgcccctaacttgaagatcgtcggtcgtgccggcgtgggcttggacaacgttgacatccctgctgccactgaagctggcgtcatggttgctaacgcaccgacctctaatattcactccgcttgtgagcacgcaatttctttgctgctgtctactgctcgccagatccctgctgctgatgcgacgctgcgtgagggcgagtggaagcggtcttctttcaacggtgtggaaattttcggaaaaactgtcggtatcgtcggttttggccacattggtcagttgtttgctcagcgtcttgctgcgtttgagaccaccattgttgcttacgatccttacgctaaccctgctcgtgcggctcagctgaacgttgagttggttgagttggatgagctgatgagccgttctgactttgtcaccattcaccttcctaagaccaaggaaactgctggcatgtttgatgcgcagctccttgctaagtccaagaagggccagatcatcatcaacgctgctcgtggtggccttgttgatgagcaggctttggctgatgcgattgagtccggtcacattcgtggcgctggtttcgatgtgtactccaccgagccttgcactgattctcctttgttcaagttgcctcaggttgttgtgactcctcacttgggtgggtctactgaagaggctcaggatcgtgcgggtactgacgttgctgattctgtgctcaaggcgctggctggcgagttcgtggcggatgctgtgaacgtttccggtggtcgcgtgggcgaagaggttgctgtgtggatggatctggctcgcaagcttggtcttcttgctggcaagcttgtcgacgccgccccagtctccattgaggttgaggctcgaggcgagctttcttccgagcaggtcgatgcacttggtttgtccgctgttcgtggtttgttctccggaattatcgaagagtccgttactttcgtcaacgctcctcgcattgctgaagagcgtggcctggacatctccgtgaagaccaactctgagtctgttactcaccgttccgtcctgcaggtcaaggtcattactggcagcggcgcgagcgcaactgttgttggtgccctgactggtcttgagcgcgttgagaagatcacccgcatcaatggccgtggcctggatctgcgcgcagagggtctgaacctcttcctgcaggccactgacgctcctggtgcactgggtaccgttggtaccaagctgggtgctgctggcatcaacatcgaggctgctgcgttgactcaggctgagaagggtgacggcgctgtcctgatcctgcgtgttgagtccgctgtctctgaagagctggaagctgaaatcaacgctgagttgggtgctacttccttccaggttgatcttgactaataaagcttggttgataaaagaaggagaccagtttatggctcaaatcttcaattttagttctggtccggcaatgctaccggcagaggtgcttaaacaggctcaacaggaactgcgcgactggaacggtcttggtacgtcggtgatggaagtgagtcaccgtggcaaagagttcattcaggttgcagaggaagccgagaaggattttcgcgatcttcttaatgtcccctccaactacaaggtattattctgccatggcggtggtcgcggtcagtttgctgcggtaccgctgaatattctcggtgataaaaccaccgcagattatgttgatgccggttactgggcggcaagtgccattaaagaagcgaaaaaatactgcacgcctaatgtctttgacgccaaagtgactgttgatggtctgcgcgcggttaagccaatgcgtgaatggcaactctctgataatgctgcttatatgcattattgcccgaatgaaaccatcgatggtatcgccatcgacgaaacgccagacttcggcgcagatgtggtggtcgccgctgacttctcttcaaccattctttcccgtccgattgacgtcagccgttatggtgtaatttacgctggcgcgcagaaaaatatcggcccggctggcctgacaatcgtcatcgttcgtgaagatttgctgggcaaagcgaatatcgcgtgtccgtcgattctggattattccatcctcaacgataacggctccatgtttaacacgccgccgacatttgcctggtatctatctggtctggtctttaaatggctgaaagcgaacggcggtgtagctgaaatggataaaatcaatcagcaaaaagcagaactgctatatggggtgattgataacagcgatttctaccgcaatgacgtggcgaaagctaaccgttcgcggatgaacgtgccgttccagttggcggacagtgcgcttgacaaattgttccttgaagagtcttttgctgctggccttcatgcactgaaaggtcaccgtgtggtcggcggaatgcgcgcttctatttataacgccatgccgctggaaggcgttaaagcgctgacagacttcatggttgagttcgaacgccgtcacggttgataaaagaaggagaccagtttatgcctaacattacctggtgcgacctgcctgaagatgtctctttatggccgggtctgcctctttcattaagtggtgatgaagtgatgccactggattaccacgcaggtcgtagcggctggctgctgtatggtcgtgggctggataaacaacgtctgacccaataccagagcaaactgggtgcggcgatggtgattgttgccgcctggtgcgtggaagattatcaggtgattcgtctggcaggttcactcaccgcacgggctacacgcctggcccacgaagcgcagctggatgtcgccccgctggggaaaatcccgcacctgcgcacgccgggtttgctggtgatggatatggactccaccgccatccagattgaatgtattgatgaaattgccaaactggccggaacgggcgagatggtggcggaagtaaccgaacgggcgatgcgcggcgaactcgattttaccgccagcctgcgcagccgtgtggcgacgctgaaaggcgctgacgccaatattctgcaacaggtgcgtgaaaatctgccgctgatgccaggcttaacgcaactggtgctcaagctggaaacgctgggctggaaagtggcgattgcctccggcggctttactttctttgctgaatacctgcgcgacaagctgcgcctgaccgccgtggtagccaatgaactggagatcatggacggtaaatttaccggcaatgtgatcggcgacatcgtagacgcgcagtacaaagcgaaaactctgactcgcctcgcgcaggagtatgaaatcccgctggcgcagaccgtggcgattggcgatggagccaatgacctgccgatgatcaaagcggcagggctggggattgcctaccatgccaagccaaaagtgaatgaaaaggcggaagtcaccatccgtcacgctgacctgatgggggtattctgcatcctctcaggcagcctgaatcagaagtgataagctgaggtcgcctcagcggccggcccctgcaggcgccggcgactagtcttggactcctgttgatagatccagtaatgacctcagaactccatctggatttgttcagaacgctcggttgccgccgggcgttttttattggtgagaatccaggggtccccaataattacgatttaaatttgtgtctcaaaatctctgatgttacattgcacaagataaaaatatatcatcatgaacaataaaactgtctgcttacataaacagtaatacaaggggtgttatgagccatattcagcgtgaaacgagctgtagccgtccgcgtctgaacagcaacatggatgcggatctgtatggctataaatgggcgcgtgataacgtgggtcagagcggcgcgaccatttatcgtctgtatggcaaaccggatgcgccggaactgtttctgaaacatggcaaaggcagcgtggcgaacgatgtgaccgatgaaatggtgcgtctgaactggctgaccgaatttatgccgctgccgaccattaaacattttattcgcaccccggatgatgcgtggctgctgaccaccgcgattccgggcaaaaccgcgtttcaggtgctggaagaatatccggatagcggcgaaaacattgtggatgcgctggccgtgtttctgcgtcgtctgcatagcattccggtgtgcaactgcccgtttaacagcgatcgtgtgtttcgtctggcccaggcgcagagccgtatgaacaacggcctggtggatgcgagcgattttgatgatgaacgtaacggctggccggtggaacaggtgtggaaagaaatgcataaactgctgccgtttagcccggatagcgtggtgacccacggcgattttagcctggataacctgattttcgatgaaggcaaactgattggctgcattgatgtgggccgtgtgggcattgcggatcgttatcaggatctggccattctgtggaactgcctgggcgaatttagcccgagcctgcaaaaacgtctgtttcagaaatatggcattgataatccggatatgaacaaactgcaatttcatctgatgctggatgaatttttctaataattaattggaccgttgtccttttccgctgcataaccctgcttcggggtcattatagcgattttttcggtatatccatcctttttcgcacgatatacaggattttgccaaagggttcgtgtagactttccttggtgtatccaacggcgtcagccgggcaggataggtgaagtaggcccacccgcgagcgggtgttccttcttcactgtcccttattcgcacctggcggtgctcaacgggaatcctgctctgcgaggctggccgtaggccggcctcagatccttccgtatttagccagtatg

SEQ ID NO: 30 - DNA, 6784 bp, synthetic construct
  source 1..6784: mol_type = other DNA
tgccaaagggttcgtgtagactttccttggtgtatccaacggcgtcagccgggcaggataggtgaagtaggcccacccgcgagcgggtgttccttcttcactgtcccttattcgcacctggcggtgctcaacgggaatcctgctctgcgaggctggccgtaggccggcctcagatccttccgtatttagccagtatgttctctagtgtggttcgttgtttttgcgtgagccatgagaacgaaccattgagatcatacttactttgcatgtcactcaaaaattttgcctcaaaactggtgagctgaatttttgcagttaaagcatcgtgtagtgtttttcttagtccgttatgtaggtaggaatctgatgtaatggttgttggtattttgtcaccattcatttttatctggttgttctcaagttcggttacgagatccatttgtctatctagttcaacttggaaaatcaacgtatcagtcgggcggcctcgcttatcaaccaccaatttcatattgctgtaagtgtttaaatctttacttattggtttcaaaacccattggttaagccttttaaactcatggtagttattttcaagcattaacatgaacttaaattcatcaaggctaatctctatatttgccttgtgagttttcttttgtgttagttcttttaataaccactcataaatcctcatagagtatttgttttcaaaagacttaacatgttccagattatattttatgaatttttttaactggaaaagataaggcaatatctcttcactaaaaactaattctaatttttcgcttgagaacttggcatagtttgtccactggaaaatctcaaagcctttaaccaaaggattcctgatttccacagttctcgtcatcagctctctggttgctttagctaatacaccataagcattttccctactgatgttcatcatctgagcgtattggttataagtgaacgataccgtccgttctttccttgtagggttttcaatcgtggggttgagtagtgccacacagcataaaattagcttggtttcatgctccgttaagtcatagcgactaatcgctagttcatttgctttgaaaacaactaattcagacatacatctcaattggtctaggtgattttaatcactataccaattgagatgggctagtcaatgataattacatgtccttttcctttgagttgtgggtatctgtaaattctgctagacctttgctggaaaacttgtaaattctgctagaccctctgtaaattccgctagacctttgtgtgttttttttgtttatattcaagtggttataatttatagaataaagaaagaataaaaaaagataaaaagaatagatcccagccctgtgtataactcactactttagtcagttccgcagtattacaaaaggatgtcgcaaacgctgtttgctcctctacaaaacagaccttaaaaccctaaaggcttaagtagcaccctcgcaagctcgggcaaatcgctgaatattccttttgtctccgaccatcaggcacctgagtcgctgtctttttcgtgacattcagttcgctgcgctcacggctctggcagtgaatgggggtaaatggcactacaggcgcggcgcgcccagctgtctagggcggcggatttgtcctactcaggagagcgttcaccgacaaacaacagataaaacgaaaggcccagtctttcgactgagcctttcgttttatttgatgcctttaattaagcggccgcggcgcgcccgtcgacgcgcgcgcggctgaggatacctcagcataggccttttacggctagctcagtcctaggtatagtgctagctcttaatcatgctaaggaggattaactttatgagccagaatggccgtccggtagtcctcatcgccgataagcttgcgcagtccactgttgacgcgcttggagatgcagtagaagtccgttgggttgacggacctaaccgcccagaactgcttgatgcagttaaggaagcggacgcactgctcgtgcgttctgctaccactgtcgatgctgaagtcatcgccgctgcccctaacttgaagatcgtcggtcgtgccggcgtgggcttggacaacgttgacatccctgctgccactgaagctggcgtcatggttgctaacgcaccgacctctaatattcactccgcttgtgagcacgcaatttctttgctgctgtctactgctcgccagatccctgctgctgatgcgacgctgcgtgagggcgagtggaagcggtcttctttcaacggtgtggaaattttcggaaaaactgtcggtatcgtcggttttggccacattggtcagttgtttgctcagcgtcttgctgcgtttgagaccaccattgttgcttacgatccttacgctaaccctgctcgtgcggctcagctgaacgttgagttggttgagttggatgagctgatgagccgttctgactttgtcaccattcaccttcctaagaccaaggaaactgctggcatgtttgatgcgcagctccttgctaagtccaagaagggccagatcatcatcaacgctgctcgtggtggccttgttgatgagcaggctttggctgatgcgattgagtccggtcacattcgtggcgctggtttcgatgtgtactccaccgagccttgcactgattctcctttgttcaagttgcctcaggttgttgtgactcctcacttgggtgggtctactgaagaggctcaggatcgtgcgggtactgacgttgctgattctgtgctcaaggcgctggctggcgagttcgtggcggatgctgtgaacgtttccggtggtcgcgtgggcgaagaggttgctgtgtggatggatctggctcgcaagcttggtcttcttgctggcaagcttgtcgacgccgccccagtctccattgaggttgaggctcgaggcgagctttcttccgagcaggtcgatgcacttggtttgtccgctgttcgtggtttgttctccggaattatcgaagagtccgttactttcgtcaacgctcctcgcattgctgaagagcgtggcctggacatctccgtgaagaccaactctgagtctgttactcaccgttccgtcctgcaggtcaaggtcattactggcagcggcgcgagcgcaactgttgttggtgccctgactggtcttgagcgcgttgagaagatcacccgcatcaatggccgtggcctggatctgcgcgcagagggtctgaacctcttcctgcaggccactgacgctcctggtgcactgggtaccgttggtaccaagctgggtgctgctggcatcaacatcgaggctgctgcgttgactcaggctgagaagggtgacggcgctgtcctgatcctgcgtgttgagtccgctgtctctgaagagctggaagctgaaatcaacgctgagttgggtgctacttccttccaggttgatcttgactaataaagcttggttgataaaagaaggagaccagtttatggctcaaatcttcaattttagttctggtccggcaatgctaccggcagaggtgcttaaacaggctcaacaggaactgcgcgactggaacggtcttggtacgtcggtgatggaagtgagtcaccgtggcaaagagttcattcaggttgcagaggaagccgagaaggattttcgcgatcttcttaatgtcccctccaactacaaggtattattctgccatggcggtggtcgcggtcagtttgctgcggtaccgctgaatattctcggtgataaaaccaccgcagattatgttgatgccggttactgggcggcaagtgccattaaagaagcgaaaaaatactgcacgcctaatgtctttgacgccaaagtgactgttgatggtctgcgcgcggttaagccaatgcgtgaatggcaactctctgataatgctgcttatatgcattattgcccgaatgaaaccatcgatggtatcgccatcgacgaaacgccagacttcggcgcagatgtggtggtcgccgctgacttctcttcaaccattctttcccgtccgattgacgtcagccgttatggtgtaatttacgctggcgcgcagaaaaatatcggcccggctggcctgacaatcgtcatcgttcgtgaagatttgctgggcaaagcgaatatcgcgtgtccgtcgattctggattattccatcctcaacgataacggctccatgtttaacacgccgccgacatttgcctggtatctatctggtctggtctttaaatggctgaaagcgaacggcggtgtagctgaaatggataaaatcaatcagcaaaaagcagaactgctatatggggtgattgataacagcgatttctaccgcaatgacgtggcgaaagctaaccgttcgcggatgaacgtgccgttccagttggcggacagtgcgcttgacaaattgttccttgaagagtcttttgctgctggccttcatgcactgaaaggtcaccgtgtggtcggcggaatgcgcgcttctatttataacgccatgccgctggaaggcgttaaagcgctgacagacttcatggttgagttcgaacgccgtcacggttgataaaagaaggagaccagtttatgcctaacattacctggtgcgacctgcctgaagatgtctctttatggccgggtctgcctctttcattaagtggtgatgaagtgatgccactggattaccacgcaggtcgtagcggctggctgctgtatggtcgtgggctggataaacaacgtctgacccaataccagagcaaactgggtgcggcgatggtgattgttgccgcctggtgcgtggaagattatcaggtgattcgtctggcaggttcactcaccgcacgggctacacgcctggcccacgaagcgcagctggatgtcgccccgctggggaaaatcccgcacctgcgcacgccgggtttgctggtgatggatatggactccaccgccatccagattgaatgtattgatgaaattgccaaactggccggaacgggcgagatggtggcggaagtaaccgaacgggcgatgcgcggcgaactcgattttaccgccagcctgcgcagccgtgtggcgacgctgaaaggcgctgacgccaatattctgcaacaggtgcgtgaaaatctgccgctgatgccaggcttaacgcaactggtgctcaagctggaaacgctgggctggaaagtggcgattgcctccggcggctttactttctttgctgaatacctgcgcgacaagctgcgcctgaccgccgtggtagccaatgaactggagatcatggacggtaaatttaccggcaatgtgatcggcgacatcgtagacgcgcagtacaaagcgaaaactctgactcgcctcgcgcaggagtatgaaatcccgctggcgcagaccgtggcgattggcgatggagccaatgacctgccgatgatcaaagcggcagggctggggattgcctaccatgccaagccaaaagtgaatgaaaaggcggaagtcaccatccgtcacgctgacctgatgggggtattctgcatcctctcaggcagcctgaatcagaagtgataagctgaggtcgcctcagcggccggcccctgcaggcgccggcgactagtcttggactcctgttgatagatccagtaatgacctcagaactccatctggatttgttcagaacgctcggttgccgccgggcgttttttattggtgagaatccaggggtccccaataattacgatttaaatttgtgtctcaaaatctctgatgttacattgcacaagataaaaatatatcatcatgaacaataaaactgtctgcttacataaacagtaatacaaggggtgttatgagccatattcagcgtgaaacgagctgtagccgtccgcgtctgaacagcaacatggatgcggatctgtatggctataaatgggcgcgtgataacgtgggtcagagcggcgcgaccatttatcgtctgtatggcaaaccggatgcgccggaactgtttctgaaacatggcaaaggcagcgtggcgaacgatgtgaccgatgaaatggtgcgtctgaactggctgaccgaatttatgccgctgccgaccattaaacattttattcgcaccccggatgatgcgtggctgctgaccaccgcgattccgggcaaaaccgcgtttcaggtgctggaagaatatccggatagcggcgaaaacattgtggatgcgctggccgtgtttctgcgtcgtctgcatagcattccggtgtgcaactgcccgtttaacagcgatcgtgtgtttcgtctggcccaggcgcagagccgtatgaacaacggcctggtggatgcgagcgattttgatgatgaacgtaacggctggccggtggaacaggtgtggaaagaaatgcataaactgctgccgtttagcccggatagcgtggtgacccacggcgattttagcctggataacctgattttcgatgaaggcaaactgattggctgcattgatgtgggccgtgtgggcattgcggatcgttatcaggatctggccattctgtggaactgcctgggcgaatttagcccgagcctgcaaaaacgtctgtttcagaaatatggcattgataatccggatatgaacaaactgcaatttcatctgatgctggatgaatttttctaataattaattggaccgttgtccttttccgctgcataaccctgcttcggggtcattatagcgattttttcggtatatccatcctttttcgcacgatatacaggattt

SEQ ID NO: 31 - DNA, 6784 bp, synthetic construct
  source 1..6784: mol_type = other DNA
ctctagtgtggttcgttgtttttgcgtgagccatgagaacgaaccattgagatcatacttactttgcatgtcactcaaaaattttgcctcaaaactggtgagctgaatttttgcagttaaagcatcgtgtagtgtttttcttagtccgttatgtaggtaggaatctgatgtaatggttgttggtattttgtcaccattcatttttatctggttgttctcaagttcggttacgagatccatttgtctatctagttcaacttggaaaatcaacgtatcagtcgggcggcctcgcttatcaaccaccaatttcatattgctgtaagtgtttaaatctttacttattggtttcaaaacccattggttaagccttttaaactcatggtagttattttcaagcattaacatgaacttaaattcatcaaggctaatctctatatttgccttgtgagttttcttttgtgttagttcttttaataaccactcataaatcctcatagagtatttgttttcaaaagacttaacatgttccagattatattttatgaatttttttaactggaaaagataaggcaatatctcttcactaaaaactaattctaatttttcgcttgagaacttggcatagtttgtccactggaaaatctcaaagcctttaaccaaaggattcctgatttccacagttctcgtcatcagctctctggttgctttagctaatacaccataagcattttccctactgatgttcatcatctgagcgtattggttataagtgaacgataccgtccgttctttccttgtagggttttcaatcgtggggttgagtagtgccacacagcataaaattagcttggtttcatgctccgttaagtcatagcgactaatcgctagttcatttgctttgaaaacaactaattcagacatacatctcaattggtctaggtgattttaatcactataccaattgagatgggctagtcaatgataattacatgtccttttcctttgagttgtgggtatctgtaaattctgctagacctttgctggaaaacttgtaaattctgctagaccctctgtaaattccgctagacctttgtgtgttttttttgtttatattcaagtggttataatttatagaataaagaaagaataaaaaaagataaaaagaatagatcccagccctgtgtataactcactactttagtcagttccgcagtattacaaaaggatgtcgcaaacgctgtttgctcctctacaaaacagaccttaaaaccctaaaggcttaagtagcaccctcgcaagctcgggcaaatcgctgaatattccttttgtctccgaccatcaggcacctgagtcgctgtctttttcgtgacattcagttcgctgcgctcacggctctggcagtgaatgggggtaaatggcactacaggcgcggcgcgcccagctgtctagggcggcggatttgtcctactcaggagagcgttcaccgacaaacaacagataaaacgaaaggcccagtctttcgactgagcctttcgttttatttgatgcctttaattaagcggccgcggcgcgcccgtcgacgcgcgcgcggctgaggatacctcagcataggccttttatagctagctcagcccttggtacaatgctagctcttaatcatgctaaggaggattaactttatgagccagaatggccgtccggtagtcctcatcgccgataagcttgcgcagtccactgttgacgcgcttggagatgcagtagaagtccgttgggttgacggacctaaccgcccagaactgcttgatgcagttaaggaagcggacgcactgctcgtgcgttctgctaccactgtcgatgctgaagtcatcgccgctgcccctaacttgaagatcgtcggtcgtgccggcgtgggcttggacaacgttgacatccctgctgccactgaagctggcgtcatggttgctaacgcaccgacctctaatattcactccgcttgtgagcacgcaatttctttgctgctgtctactgctcgccagatccctgctgctgatgcgacgctgcgtgagggcgagtggaagcggtcttctttcaacggtgtggaaattttcggaaaaactgtcggtatcgtcggttttggccacattggtcagttgtttgctcagcgtcttgctgcgtttgagaccaccattgttgcttacgatccttacgctaaccctgctcgtgcggctcagctgaacgttgagttggttgagttggatgagctgatgagccgttctgactttgtcaccattcaccttcctaagaccaaggaaactgctggcatgtttgatgcgcagctccttgctaagtccaagaagggccagatcatcatcaacgctgctcgtggtggccttgttgatgagcaggctttggctgatgcgattgagtccggtcacattcgtggcgctggtttcgatgtgtactccaccgagccttgcactgattctcctttgttcaagttgcctcaggttgttgtgactcctcacttgggtgggtctactgaagaggctcaggatcgtgcgggtactgacgttgctgattctgtgctcaaggcgctggctggcgagttcgtggcggatgctgtgaacgtttccggtggtcgcgtgggcgaagaggttgctgtgtggatggatctggctcgcaagcttggtcttcttgctggcaagcttgtcgacgccgccccagtctccattgaggttgaggctcgaggcgagctttcttccgagcaggtcgatgcacttggtttgtccgctgttcgtggtttgttctccggaattatcgaagagtccgttactttcgtcaacgctcctcgcattgctgaagagcgtggcctggacatctccgtgaagaccaactctgagtctgttactcaccgttccgtcctgcaggtcaaggtcattactggcagcggcgcgagcgcaactgttgttggtgccctgactggtcttgagcgcgttgagaagatcacccgcatcaatggccgtggcctggatctgcgcgcagagggtctgaacctcttcctgcaggccactgacgctcctggtgcactgggtaccgttggtaccaagctgggtgctgctggcatcaacatcgaggctgctgcgttgactcaggctgagaagggtgacggcgctgtcctgatcctgcgtgttgagtccgctgtctctgaagagctggaagctgaaatcaacgctgagttgggtgctacttccttccaggttgatcttgactaataaagcttggttgataaaagaaggagaccagtttatggctcaaatcttcaattttagttctggtccggcaatgctaccggcagaggtgcttaaacaggctcaacaggaactgcgcgactggaacggtcttggtacgtcggtgatggaagtgagtcaccgtggcaaagagttcattcaggttgcagaggaagccgagaaggattttcgcgatcttcttaatgtcccctccaactacaaggtattattctgccatggcggtggtcgcggtcagtttgctgcggtaccgctgaatattctcggtgataaaaccaccgcagattatgttgatgccggttactgggcggcaagtgccattaaagaagcgaaaaaatactgcacgcctaatgtctttgacgccaaagtgactgttgatggtctgcgcgcggttaagccaatgcgtgaatggcaactctctgataatgctgcttatatgcattattgcccgaatgaaaccatcgatggtatcgccatcgacgaaacgccagacttcggcgcagatgtggtggtcgccgctgacttctcttcaaccattctttcccgtccgattgacgtcagccgttatggtgtaatttacgctggcgcgcagaaaaatatcggcccggctggcctgacaatcgtcatcgttcgtgaagatttgctgggcaaagcgaatatcgcgtgtccgtcgattctggattattccatcctcaacgataacggctccatgtttaacacgccgccgacatttgcctggtatctatctggtctggtctttaaatggctgaaagcgaacggcggtgtagctgaaatggataaaatcaatcagcaaaaagcagaactgctatatggggtgattgataacagcgatttctaccgcaatgacgtggcgaaagctaaccgttcgcggatgaacgtgccgttccagttggcggacagtgcgcttgacaaattgttccttgaagagtcttttgctgctggccttcatgcactgaaaggtcaccgtgtggtcggcggaatgcgcgcttctatttataacgccatgccgctggaaggcgttaaagcgctgacagacttcatggttgagttcgaacgccgtcacggttgataaaagaaggagaccagtttatgcctaacattacctggtgcgacctgcctgaagatgtctctttatggccgggtctgcctctttcattaagtggtgatgaagtgatgccactggattaccacgcaggtcgtagcggctggctgctgtatggtcgtgggctggataaacaacgtctgacccaataccagagcaaactgggtgcggcgatggtgattgttgccgcctggtgcgtggaagattatcaggtgattcgtctggcaggttcactcaccgcacgggctacacgcctggcccacgaagcgcagctggatgtcgccccgctggggaaaatcccgcacctgcgcacgccgggtttgctggtgatggatatggactccaccgccatccagattgaatgtattgatgaaattgccaaactggccggaacgggcgagatggtggcggaagtaaccgaacgggcgatgcgcggcgaactcgattttaccgccagcctgcgcagccgtgtggcgacgctgaaaggcgctgacgccaatattctgcaacaggtgcgtgaaaatctgccgctgatgccaggcttaacgcaactggtgctcaagctggaaacgctgggctggaaagtggcgattgcctccggcggctttactttctttgctgaatacctgcgcgacaagctgcgcctgaccgccgtggtagccaatgaactggagatcatggacggtaaatttaccggcaatgtgatcggcgacatcgtagacgcgcagtacaaagcgaaaactctgactcgcctcgcgcaggagtatgaaatcccgctggcgcagaccgtggcgattggcgatggagccaatgacctgccgatgatcaaagcggcagggctggggattgcctaccatgccaagccaaaagtgaatgaaaaggcggaagtcaccatccgtcacgctgacctgatgggggtattctgcatcctctcaggcagcctgaatcagaagtgataagctgaggtcgcctcagcggccggcccctgcaggcgccggcgactagtcttggactcctgttgatagatccagtaatgacctcagaactccatctggatttgttcagaacgctcggttgccgccgggcgttttttattggtgagaatccaggggtccccaataattacgatttaaatttgtgtctcaaaatctctgatgttacattgcacaagataaaaatatatcatcatgaacaataaaactgtctgcttacataaacagtaatacaaggggtgttatgagccatattcagcgtgaaacgagctgtagccgtccgcgtctgaacagcaacatggatgcggatctgtatggctataaatgggcgcgtgataacgtgggtcagagcggcgcgaccatttatcgtctgtatggcaaaccggatgcgccggaactgtttctgaaacatggcaaaggcagcgtggcgaacgatgtgaccgatgaaatggtgcgtctgaactggctgaccgaatttatgccgctgccgaccattaaacattttattcgcaccccggatgatgcgtggctgctgaccaccgcgattccgggcaaaaccgcgtttcaggtgctggaagaatatccggatagcggcgaaaacattgtggatgcgctggccgtgtttctgcgtcgtctgcatagcattccggtgtgcaactgcccgtttaacagcgatcgtgtgtttcgtctggcccaggcgcagagccgtatgaacaacggcctggtggatgcgagcgattttgatgatgaacgtaacggctggccggtggaacaggtgtggaaagaaatgcataaactgctgccgtttagcccggatagcgtggtgacccacggcgattttagcctggataacctgattttcgatgaaggcaaactgattggctgcattgatgtgggccgtgtgggcattgcggatcgttatcaggatctggccattctgtggaactgcctgggcgaatttagcccgagcctgcaaaaacgtctgtttcagaaatatggcattgataatccggatatgaacaaactgcaatttcatctgatgctggatgaatttttctaataattaattggaccgttgtccttttccgctgcataaccctgcttcggggtcattatagcgattttttcggtatatccatcctttttcgcacgatatacaggattttgccaaagggttcgtgtagactttccttggtgtatccaacggcgtcagccgggcaggataggtgaagtaggcccacccgcgagcgggtgttccttcttcactgtcccttattcgcacctggcggtgctcaacgggaatcctgctctgcgaggctggccgtaggccggcctcagatccttccgtatttagccagtatgtt

SEQ ID NO: 32 - DNA, 6784 bp, synthetic construct
  source 1..6784: mol_type = other DNA
ttctaatttttcgcttgagaacttggcatagtttgtccactggaaaatctcaaagcctttaaccaaaggattcctgatttccacagttctcgtcatcagctctctggttgctttagctaatacaccataagcattttccctactgatgttcatcatctgagcgtattggttataagtgaacgataccgtccgttctttccttgtagggttttcaatcgtggggttgagtagtgccacacagcataaaattagcttggtttcatgctccgttaagtcatagcgactaatcgctagttcatttgctttgaaaacaactaattcagacatacatctcaattggtctaggtgattttaatcactataccaattgagatgggctagtcaatgataattacatgtccttttcctttgagttgtgggtatctgtaaattctgctagacctttgctggaaaacttgtaaattctgctagaccctctgtaaattccgctagacctttgtgtgttttttttgtttatattcaagtggttataatttatagaataaagaaagaataaaaaaagataaaaagaatagatcccagccctgtgtataactcactactttagtcagttccgcagtattacaaaaggatgtcgcaaacgctgtttgctcctctacaaaacagaccttaaaaccctaaaggcttaagtagcaccctcgcaagctcgggcaaatcgctgaatattccttttgtctccgaccatcaggcacctgagtcgctgtctttttcgtgacattcagttcgctgcgctcacggctctggcagtgaatgggggtaaatggcactacaggcgcggcgcgcccagctgtctagggcggcggatttgtcctactcaggagagcgttcaccgacaaacaacagataaaacgaaaggcccagtctttcgactgagcctttcgttttatttgatgcctttaattaagcggccgcggcgcgcccgtcgacgcgcgcgcggctgaggatacctcagcataggccttttacggctagctcagccctaggtattatgctagctcttaatcatgctaaggaggattaactttatgagccagaatggccgtccggtagtcctcatcgccgataagcttgcgcagtccactgttgacgcgcttggagatgcagtagaagtccgttgggttgacggacctaaccgcccagaactgcttgatgcagttaaggaagcggacgcactgctcgtgcgttctgctaccactgtcgatgctgaagtcatcgccgctgcccctaacttgaagatcgtcggtcgtgccggcgtgggcttggacaacgttgacatccctgctgccactgaagctggcgtcatggttgctaacgcaccgacctctaatattcactccgcttgtgagcacgcaatttctttgctgctgtctactgctcgccagatccctgctgctgatgcgacgctgcgtgagggcgagtggaagcggtcttctttcaacggtgtggaaattttcggaaaaactgtcggtatcgtcggttttggccacattggtcagttgtttgctcagcgtcttgctgcgtttgagaccaccattgttgcttacgatccttacgctaaccctgctcgtgcggctcagctgaacgttgagttggttgagttggatgagctgatgagccgttctgactttgtcaccattcaccttcctaagaccaaggaaactgctggcatgtttgatgcgcagctccttgctaagtccaagaagggccagatcatcatcaacgctgctcgtggtggccttgttgatgagcaggctttggctgatgcgattgagtccggtcacattcgtggcgctggtttcgatgtgtactccaccgagccttgcactgattctcctttgttcaagttgcctcaggttgttgtgactcctcacttgggtgggtctactgaagaggctcaggatcgtgcgggtactgacgttgctgattctgtgctcaaggcgctggctggcgagttcgtggcggatgctgtgaacgtttccggtggtcgcgtgggcgaagaggttgctgtgtggatggatctggctcgcaagcttggtcttcttgctggcaagcttgtcgacgccgccccagtctccattgaggttgaggctcgaggcgagctttcttccgagcaggtcgatgcacttggtttgtccgctgttcgtggtttgttctccggaattatcgaagagtccgttactttcgtcaacgctcctcgcattgctgaagagcgtggcctggacatctccgtgaagaccaactctgagtctgttactcaccgttccgtcctgcaggtcaaggtcattactggcagcggcgcgagcgcaactgttgttggtgccctgactggtcttgagcgcgttgagaagatcacccgcatcaatggccgtggcctggatctgcgcgcagagggtctgaacctcttcctgcaggccactgacgctcctggtgcactgggtaccgttggtaccaagctgggtgctgctggcatcaacatcgaggctgctgcgttgactcaggctgagaagggtgacggcgctgtcctgatcctgcgtgttgagtccgctgtctctgaagagctggaagctgaaatcaacgctgagttgggtgctacttccttccaggttgatcttgactaataaagcttggttgataaaagaaggagaccagtttatggctcaaatcttcaattttagttctggtccggcaatgctaccggcagaggtgcttaaacaggctcaacaggaactgcgcgactggaacggtcttggtacgtcggtgatggaagtgagtcaccgtggcaaagagttcattcaggttgcagaggaagccgagaaggattttcgcgatcttcttaatgtcccctccaactacaaggtattattctgccatggcggtggtcgcggtcagtttgctgcggtaccgctgaatattctcggtgataaaaccaccgcagattatgttgatgccggttactgggcggcaagtgccattaaagaagcgaaaaaatactgcacgcctaatgtctttgacgccaaagtgactgttgatggtctgcgcgcggttaagccaatgcgtgaatggcaactctctgataatgctgcttatatgcattattgcccgaatgaaaccatcgatggtatcgccatcgacgaaacgccagacttcggcgcagatgtggtggtcgccgctgacttctcttcaaccattctttcccgtccgattgacgtcagccgttatggtgtaatttacgctggcgcgcagaaaaatatcggcccggctggcctgacaatcgtcatcgttcgtgaagatttgctgggcaaagcgaatatcgcgtgtccgtcgattctggattattccatcctcaacgataacggctccatgtttaacacgccgccgacatttgcctggtatctatctggtctggtctttaaatggctgaaagcgaacggcggtgtagctgaaatggataaaatcaatcagcaaaaagcagaactgctatatggggtgattgataacagcgatttctaccgcaatgacgtggcgaaagctaaccgttcgcggatgaacgtgccgttccagttggcggacagtgcgcttgacaaattgttccttgaagagtcttttgctgctggccttcatgcactgaaaggtcaccgtgtggtcggcggaatgcgcgcttctatttataacgccatgccgctggaaggcgttaaagcgctgacagacttcatggttgagttcgaacgccgtcacggttgataaaagaaggagaccagtttatgcctaacattacctggtgcgacctgcctgaagatgtctctttatggccgggtctgcctctttcattaagtggtgatgaagtgatgccactggattaccacgcaggtcgtagcggctggctgctgtatggtcgtgggctggataaacaacgtctgacccaataccagagcaaactgggtgcggcgatggtgattgttgccgcctggtgcgtggaagattatcaggtgattcgtctggcaggttcactcaccgcacgggctacacgcctggcccacgaagcgcagctggatgtcgccccgctggggaaaatcccgcacctgcgcacgccgggtttgctggtgatggatatggactccaccgccatccagattgaatgtattgatgaaattgccaaactggccggaacgggcgagatggtggcggaagtaaccgaacgggcgatgcgcggcgaactcgattttaccgccagcctgcgcagccgtgtggcgacgctgaaaggcgctgacgccaatattctgcaacaggtgcgtgaaaatctgccgctgatgccaggcttaacgcaactggtgctcaagctggaaacgctgggctggaaagtggcgattgcctccggcggctttactttctttgctgaatacctgcgcgacaagctgcgcctgaccgccgtggtagccaatgaactggagatcatggacggtaaatttaccggcaatgtgatcggcgacatcgtagacgcgcagtacaaagcgaaaactctgactcgcctcgcgcaggagtatgaaatcccgctggcgcagaccgtggcgattggcgatggagccaatgacctgccgatgatcaaagcggcagggctggggattgcctaccatgccaagccaaaagtgaatgaaaaggcggaagtcaccatccgtcacgctgacctgatgggggtattctgcatcctctcaggcagcctgaatcagaagtgataagctgaggtcgcctcagcggccggcccctgcaggcgccggcgactagtcttggactcctgttgatagatccagtaatgacctcagaactccatctggatttgttcagaacgctcggttgccgccgggcgttttttattggtgagaatccaggggtccccaataattacgatttaaatttgtgtctcaaaatctctgatgttacattgcacaagataaaaatatatcatcatgaacaataaaactgtctgcttacataaacagtaatacaaggggtgttatgagccatattcagcgtgaaacgagctgtagccgtccgcgtctgaacagcaacatggatgcggatctgtatggctataaatgggcgcgtgataacgtgggtcagagcggcgcgaccatttatcgtctgtatggcaaaccggatgcgccggaactgtttctgaaacatggcaaaggcagcgtggcgaacgatgtgaccgatgaaatggtgcgtctgaactggctgaccgaatttatgccgctgccgaccattaaacattttattcgcaccccggatgatgcgtggctgctgaccaccgcgattccgggcaaaaccgcgtttcaggtgctggaagaatatccggatagcggcgaaaacattgtggatgcgctggccgtgtttctgcgtcgtctgcatagcattccggtgtgcaactgcccgtttaacagcgatcgtgtgtttcgtctggcccaggcgcagagccgtatgaacaacggcctggtggatgcgagcgattttgatgatgaacgtaacggctggccggtggaacaggtgtggaaagaaatgcataaactgctgccgtttagcccggatagcgtggtgacccacggcgattttagcctggataacctgattttcgatgaaggcaaactgattggctgcattgatgtgggccgtgtgggcattgcggatcgttatcaggatctggccattctgtggaactgcctgggcgaatttagcccgagcctgcaaaaacgtctgtttcagaaatatggcattgataatccggatatgaacaaactgcaatttcatctgatgctggatgaatttttctaataattaattggaccgttgtccttttccgctgcataaccctgcttcggggtcattatagcgattttttcggtatatccatcctttttcgcacgatatacaggattttgccaaagggttcgtgtagactttccttggtgtatccaacggcgtcagccgggcaggataggtgaagtaggcccacccgcgagcgggtgttccttcttcactgtcccttattcgcacctggcggtgctcaacgggaatcctgctctgcgaggctggccgtaggccggcctcagatccttccgtatttagccagtatgttctctagtgtggttcgttgtttttgcgtgagccatgagaacgaaccattgagatcatacttactttgcatgtcactcaaaaattttgcctcaaaactggtgagctgaatttttgcagttaaagcatcgtgtagtgtttttcttagtccgttatgtaggtaggaatctgatgtaatggttgttggtattttgtcaccattcatttttatctggttgttctcaagttcggttacgagatccatttgtctatctagttcaacttggaaaatcaacgtatcagtcgggcggcctcgcttatcaaccaccaatttcatattgctgtaagtgtttaaatctttacttattggtttcaaaacccattggttaagccttttaaactcatggtagttattttcaagcattaacatgaacttaaattcatcaaggctaatctctatatttgccttgtgagttttcttttgtgttagttcttttaataaccactcataaatcctcatagagtatttgttttcaaaagacttaacatgttccagattatattttatgaatttttttaactggaaaagataaggcaatatctcttcactaaaaactaa

SEQ ID NO: 33 - DNA, 7658 bp, synthetic construct
  source 1..7658: mol_type = other DNA
tattcgcacctggcggtgctcaacgggaatcctgctctgcgaggctggccgtaggccggcctcagatccttccgtatttagccagtatgttctctagtgtggttcgttgtttttgcgtgagccatgagaacgaaccattgagatcatacttactttgcatgtcactcaaaaattttgcctcaaaactggtgagctgaatttttgcagttaaagcatcgtgtagtgtttttcttagtccgttatgtaggtaggaatctgatgtaatggttgttggtattttgtcaccattcatttttatctggttgttctcaagttcggttacgagatccatttgtctatctagttcaacttggaaaatcaacgtatcagtcgggcggcctcgcttatcaaccaccaatttcatattgctgtaagtgtttaaatctttacttattggtttcaaaacccattggttaagccttttaaactcatggtagttattttcaagcattaacatgaacttaaattcatcaaggctaatctctatatttgccttgtgagttttcttttgtgttagttcttttaataaccactcataaatcctcatagagtatttgttttcaaaagacttaacatgttccagattatattttatgaatttttttaactggaaaagataaggcaatatctcttcactaaaaactaattctaatttttcgcttgagaacttggcatagtttgtccactggaaaatctcaaagcctttaaccaaaggattcctgatttccacagttctcgtcatcagctctctggttgctttagctaatacaccataagcattttccctactgatgttcatcatctgagcgtattggttataagtgaacgataccgtccgttctttccttgtagggttttcaatcgtggggttgagtagtgccacacagcataaaattagcttggtttcatgctccgttaagtcatagcgactaatcgctagttcatttgctttgaaaacaactaattcagacatacatctcaattggtctaggtgattttaatcactataccaattgagatgggctagtcaatgataattacatgtccttttcctttgagttgtgggtatctgtaaattctgctagacctttgctggaaaacttgtaaattctgctagaccctctgtaaattccgctagacctttgtgtgttttttttgtttatattcaagtggttataatttatagaataaagaaagaataaaaaaagataaaaagaatagatcccagccctgtgtataactcactactttagtcagttccgcagtattacaaaaggatgtcgcaaacgctgtttgctcctctacaaaacagaccttaaaaccctaaaggcttaagtagcaccctcgcaagctcgggcaaatcgctgaatattccttttgtctccgaccatcaggcacctgagtcgctgtctttttcgtgacattcagttcgctgcgctcacggctctggcagtgaatgggggtaaatggcactacaggcgcggcgcgcccagctgtctagggcggcggatttgtcctactcaggagagcgttcaccgacaaacaacagataaaacgaaaggcccagtctttcgactgagcctttcgttttatttgatgcctttaattaagcggccgcggcgcgcccgtcgacgcgcgcgcggctgaggatacctcagcataggcctttgacagctagctcagtcctaggtataatgctagctcttaatcatgctaaggaggattaactttatgagccagaatggccgtccggtagtcctcatcgccgataagcttgcgcagtccactgttgacgcgcttggagatgcagtagaagtccgttgggttgacggacctaaccgcccagaactgcttgatgcagttaaggaagcggacgcactgctcgtgcgttctgctaccactgtcgatgctgaagtcatcgccgctgcccctaacttgaagatcgtcggtcgtgccggcgtgggcttggacaacgttgacatccctgctgccactgaagctggcgtcatggttgctaacgcaccgacctctaatattcactccgcttgtgagcacgcaatttctttgctgctgtctactgctcgccagatccctgctgctgatgcgacgctgcgtgagggcgagtggaagcggtcttctttcaacggtgtggaaattttcggaaaaactgtcggtatcgtcggttttggccacattggtcagttgtttgctcagcgtcttgctgcgtttgagaccaccattgttgcttacgatccttacgctaaccctgctcgtgcggctcagctgaacgttgagttggttgagttggatgagctgatgagccgttctgactttgtcaccattcaccttcctaagaccaaggaaactgctggcatgtttgatgcgcagctccttgctaagtccaagaagggccagatcatcatcaacgctgctcgtggtggccttgttgatgagcaggctttggctgatgcgattgagtccggtcacattcgtggcgctggtttcgatgtgtactccaccgagccttgcactgattctcctttgttcaagttgcctcaggttgttgtgactcctcacttgggtgggtctactgaagaggctcaggatcgtgcgggtactgacgttgctgattctgtgctcaaggcgctggctggcgagttcgtggcggatgctgtgaacgtttccggtggtcgcgtgggcgaagaggttgctgtgtggatggatctggctcgcaagcttggtcttcttgctggcaagcttgtcgacgccgccccagtctccattgaggttgaggctcgaggcgagctttcttccgagcaggtcgatgcacttggtttgtccgctgttcgtggtttgttctccggaattatcgaagagtccgttactttcgtcaacgctcctcgcattgctgaagagcgtggcctggacatctccgtgaagaccaactctgagtctgttactcaccgttccgtcctgcaggtcaaggtcattactggcagcggcgcgagcgcaactgttgttggtgccctgactggtcttgagcgcgttgagaagatcacccgcatcaatggccgtggcctggatctgcgcgcagagggtctgaacctcttcctgcaggccactgacgctcctggtgcactgggtaccgttggtaccaagctgggtgctgctggcatcaacatcgaggctgctgcgttgactcaggctgagaagggtgacggcgctgtcctgatcctgcgtgttgagtccgctgtctctgaagagctggaagctgaaatcaacgctgagttgggtgctacttccttccaggttgatcttgactaataaagcttggttgataaaagaaggagaccagtttatggctcaaatcttcaattttagttctggtccggcaatgctaccggcagaggtgcttaaacaggctcaacaggaactgcgcgactggaacggtcttggtacgtcggtgatggaagtgagtcaccgtggcaaagagttcattcaggttgcagaggaagccgagaaggattttcgcgatcttcttaatgtcccctccaactacaaggtattattctgccatggcggtggtcgcggtcagtttgctgcggtaccgctgaatattctcggtgataaaaccaccgcagattatgttgatgccggttactgggcggcaagtgccattaaagaagcgaaaaaatactgcacgcctaatgtctttgacgccaaagtgactgttgatggtctgcgcgcggttaagccaatgcgtgaatggcaactctctgataatgctgcttatatgcattattgcccgaatgaaaccatcgatggtatcgccatcgacgaaacgccagacttcggcgcagatgtggtggtcgccgctgacttctcttcaaccattctttcccgtccgattgacgtcagccgttatggtgtaatttacgctggcgcgcagaaaaatatcggcccggctggcctgacaatcgtcatcgttcgtgaagatttgctgggcaaagcgaatatcgcgtgtccgtcgattctggattattccatcctcaacgataacggctccatgtttaacacgccgccgacatttgcctggtatctatctggtctggtctttaaatggctgaaagcgaacggcggtgtagctgaaatggataaaatcaatcagcaaaaagcagaactgctatatggggtgattgataacagcgatttctaccgcaatgacgtggcgaaagctaaccgttcgcggatgaacgtgccgttccagttggcggacagtgcgcttgacaaattgttccttgaagagtcttttgctgctggccttcatgcactgaaaggtcaccgtgtggtcggcggaatgcgcgcttctatttataacgccatgccgctggaaggcgttaaagcgctgacagacttcatggttgagttcgaacgccgtcacggttgataaaagaaggagaccagtttatgcctaacattacctggtgcgacctgcctgaagatgtctctttatggccgggtctgcctctttcattaagtggtgatgaagtgatgccactggattaccacgcaggtcgtagcggctggctgctgtatggtcgtgggctggataaacaacgtctgacccaataccagagcaaactgggtgcggcgatggtgattgttgccgcctggtgcgtggaagattatcaggtgattcgtctggcaggttcactcaccgcacgggctacacgcctggcccacgaagcgcagctggatgtcgccccgctggggaaaatcccgcacctgcgcacgccgggtttgctggtgatggatatggactccaccgccatccagattgaatgtattgatgaaattgccaaactggccggaacgggcgagatggtggcggaagtaaccgaacgggcgatgcgcggcgaactcgattttaccgccagcctgcgcagccgtgtggcgacgctgaaaggcgctgacgccaatattctgcaacaggtgcgtgaaaatctgccgctgatgccaggcttaacgcaactggtgctcaagctggaaacgctgggctggaaagtggcgattgcctccggcggctttactttctttgctgaatacctgcgcgacaagctgcgcctgaccgccgtggtagccaatgaactggagatcatggacggtaaatttaccggcaatgtgatcggcgacatcgtagacgcgcagtacaaagcgaaaactctgactcgcctcgcgcaggagtatgaaatcccgctggcgcagaccgtggcgattggcgatggagccaatgacctgccgatgatcaaagcggcagggctggggattgcctaccatgccaagccaaaagtgaatgaaaaggcggaagtcaccatccgtcacgctgacctgatgggggtattctgcatcctctcaggcagcctgaatcagaagtgacataggaggtcctcctatgtcaattcaacatttccgtgtcgcccttattcccttttttgcggcattttgccttcctgtttttgctcacccagaaacgctggtgaaagtaaaagatgctgaagatcagttgggtgcacgagtgggttacatcgaactggatctcaacagcggtaagatccttgagagttttcgccccgaagaacgttttccaatgatgagcacttttaaagttctgctatgtggcgcggtattatcccgtgttgacgccgggcaagagcaactcggtcgccgcatacactattctcagaatgacttggttgagtactcaccagtcacagaaaagcatcttacggatggcatgacagtaagagaattatgcagtgctgccataaccatgagtgataacactgcggccaacttacttctgacaacgatcggaggaccgaaggagctaaccgcttttttgcacaacatgggggatcatgtaactcgccttgatcgttgggaaccggagctgaatgaagccataccaaacgacgagcgtgacaccacgatgcctgcagcaatggcaacaacgttgcgcaaactattaactggcgaactacttactctagcttcccggcaacaattaatagactggatggaggcggataaagttgcaggaccacttctgcgctcggcccttccggctggctggtttattgctgataaatctggagccggtgagcgtgggtctcgcggtatcattgcagcactggggccagatggtaagccctcccgtatcgtagttatctacacgacggggagtcaggcaactatggatgaacgaaatagacagatcgctgagataggtgcctcactgattaagcattggtaagctgaggtcgcctcagcggccggcccctgcaggcgccggcgactagtcttggactcctgttgatagatccagtaatgacctcagaactccatctggatttgttcagaacgctcggttgccgccgggcgttttttattggtgagaatccaggggtccccaataattacgatttaaatttgtgtctcaaaatctctgatgttacattgcacaagataaaaatatatcatcatgaacaataaaactgtctgcttacataaacagtaatacaaggggtgttatgagccatattcagcgtgaaacgagctgtagccgtccgcgtctgaacagcaacatggatgcggatctgtatggctataaatgggcgcgtgataacgtgggtcagagcggcgcgaccatttatcgtctgtatggcaaaccggatgcgccggaactgtttctgaaacatggcaaaggcagcgtggcgaacgatgtgaccgatgaaatggtgcgtctgaactggctgaccgaatttatgccgctgccgaccattaaacattttattcgcaccccggatgatgcgtggctgctgaccaccgcgattccgggcaaaaccgcgtttcaggtgctggaagaatatccggatagcggcgaaaacattgtggatgcgctggccgtgtttctgcgtcgtctgcatagcattccggtgtgcaactgcccgtttaacagcgatcgtgtgtttcgtctggcccaggcgcagagccgtatgaacaacggcctggtggatgcgagcgattttgatgatgaacgtaacggctggccggtggaacaggtgtggaaagaaatgcataaactgctgccgtttagcccggatagcgtggtgacccacggcgattttagcctggataacctgattttcgatgaaggcaaactgattggctgcattgatgtgggccgtgtgggcattgcggatcgttatcaggatctggccattctgtggaactgcctgggcgaatttagcccgagcctgcaaaaacgtctgtttcagaaatatggcattgataatccggatatgaacaaactgcaatttcatctgatgctggatgaatttttctaataattaattggaccgttgtccttttccgctgcataaccctgcttcggggtcattatagcgattttttcggtatatccatcctttttcgcacgatatacaggattttgccaaagggttcgtgtagactttccttggtgtatccaacggcgtcagccgggcaggataggtgaagtaggcccacccgcgagcgggtgttccttcttcactgtccct

SEQ ID NO: 34 - DNA, 6783 bp, synthetic construct
  source 1..6783: mol_type = other DNA
tattcgcacctggcggtgctcaacgggaatcctgctctgcgaggctggccgtaggccggcctcagatccttccgtatttagccagtatgttctctagtgtggttcgttgtttttgcgtgagccatgagaacgaaccattgagatcatacttactttgcatgtcactcaaaaattttgcctcaaaactggtgagctgaatttttgcagttaaagcatcgtgtagtgtttttcttagtccgttatgtaggtaggaatctgatgtaatggttgttggtattttgtcaccattcatttttatctggttgttctcaagttcggttacgagatccatttgtctatctagttcaacttggaaaatcaacgtatcagtcgggcggcctcgcttatcaaccaccaatttcatattgctgtaagtgtttaaatctttacttattggtttcaaaacccattggttaagccttttaaactcatggtagttattttcaagcattaacatgaacttaaattcatcaaggctaatctctatatttgccttgtgagttttcttttgtgttagttcttttaataaccactcataaatcctcatagagtatttgttttcaaaagacttaacatgttccagattatattttatgaatttttttaactggaaaagataaggcaatatctcttcactaaaaactaattctaatttttcgcttgagaacttggcatagtttgtccactggaaaatctcaaagcctttaaccaaaggattcctgatttccacagttctcgtcatcagctctctggttgctttagctaatacaccataagcattttccctactgatgttcatcatctgagcgtattggttataagtgaacgataccgtccgttctttccttgtagggttttcaatcgtggggttgagtagtgccacacagcataaaattagcttggtttcatgctccgttaagtcatagcgactaatcgctagttcatttgctttgaaaacaactaattcagacatacatctcaattggtctaggtgattttaatcactataccaattgagatgggctagtcaatgataattacatgtccttttcctttgagttgtgggtatctgtaaattctgctagacctttgctggaaaacttgtaaattctgctagaccctctgtaaattccgctagacctttgtgtgttttttttgtttatattcaagtggttataatttatagaataaagaaagaataaaaaaagataaaaagaatagatcccagccctgtgtataactcactactttagtcagttccgcagtattacaaaaggatgtcgcaaacgctgtttgctcctctacaaaacagaccttaaaaccctaaaggcttaagtagcaccctcgcaagctcgggcaaatcgctgaatattccttttgtctccgaccatcaggcacctgagtcgctgtctttttcgtgacattcagttcgctgcgctcacggctctggcagtgaatgggggtaaatggcactacaggcgcggcgcgcccagctgtctagggcggcggatttgtcctactcaggagagcgttcaccgacaaacaacagataaaacgaaaggcccagtctttcgactgagcctttcgttttatttgatgcctttaattaagcggccgcggcgcgcccgtcgacgcgcgcgcggctgaggatacctcagcataggcctttgacagctagctcagtcctaggtataatgctagctcttaatcatgctaaggaggattggatacatgtcccaaaatggccgtccggtagtcctcatcgccgataagcttgcgcagtccactgttgacgcgcttggagatgcagtagaagtccgttgggttgacggacctaaccgcccagaactgcttgatgcagttaaggaagcggacgcactgctcgtgcgttctgctaccactgtcgatgctgaagtcatcgccgctgcccctaacttgaagatcgtcggtcgtgccggcgtgggcttggacaacgttgacatccctgctgccactgaagctggcgtcatggttgctaacgcaccgacctctaatattcactccgcttgtgagcacgcaatttctttgctgctgtctactgctcgccagatccctgctgctgatgcgacgctgcgtgagggcgagtggaagcggtcttctttcaacggtgtggaaattttcggaaaaactgtcggtatcgtcggttttggccacattggtcagttgtttgctcagcgtcttgctgcgtttgagaccaccattgttgcttacgatccttacgctaaccctgctcgtgcggctcagctgaacgttgagttggttgagttggatgagctgatgagccgttctgactttgtcaccattcaccttcctaagaccaaggaaactgctggcatgtttgatgcgcagctccttgctaagtccaagaagggccagatcatcatcaacgctgctcgtggtggccttgttgatgagcaggctttggctgatgcgattgagtccggtcacattcgtggcgctggtttcgatgtgtactccaccgagccttgcactgattctcctttgttcaagttgcctcaggttgttgtgactcctcacttgggtgggtctactgaagaggctcaggatcgtgcgggtactgacgttgctgattctgtgctcaaggcgctggctggcgagttcgtggcggatgctgtgaacgtttccggtggtcgcgtgggcgaagaggttgctgtgtggatggatctggctcgcaagcttggtcttcttgctggcaagcttgtcgacgccgccccagtctccattgaggttgaggctcgaggcgagctttcttccgagcaggtcgatgcacttggtttgtccgctgttcgtggtttgttctccggaattatcgaagagtccgttactttcgtcaacgctcctcgcattgctgaagagcgtggcctggacatctccgtgaagaccaactctgagtctgttactcaccgttccgtcctgcaggtcaaggtcattactggcagcggcgcgagcgcaactgttgttggtgccctgactggtcttgagcgcgttgagaagatcacccgcatcaatggccgtggcctggatctgcgcgcagagggtctgaacctcttcctgcaggccactgacgctcctggtgcactgggtaccgttggtaccaagctgggtgctgctggcatcaacatcgaggctgctgcgttgactcaggctgagaagggtgacggcgctgtcctgatcctgcgtgttgagtccgctgtctctgaagagctggaagctgaaatcaacgctgagttgggtgctacttccttccaggttgatcttgactaataaagcttggttgataaaagaaggagaccccggaatggcacaatcttcaattttagttctggtccggcaatgctaccggcagaggtgcttaaacaggctcaacaggaactgcgcgactggaacggtcttggtacgtcggtgatggaagtgagtcaccgtggcaaagagttcattcaggttgcagaggaagccgagaaggattttcgcgatcttcttaatgtcccctccaactacaaggtattattctgccatggcggtggtcgcggtcagtttgctgcggtaccgctgaatattctcggtgataaaaccaccgcagattatgttgatgccggttactgggcggcaagtgccattaaagaagcgaaaaaatactgcacgcctaatgtctttgacgccaaagtgactgttgatggtctgcgcgcggttaagccaatgcgtgaatggcaactctctgataatgctgcttatatgcattattgcccgaatgaaaccatcgatggtatcgccatcgacgaaacgccagacttcggcgcagatgtggtggtcgccgctgacttctcttcaaccattctttcccgtccgattgacgtcagccgttatggtgtaatttacgctggcgcgcagaaaaatatcggcccggctggcctgacaatcgtcatcgttcgtgaagatttgctgggcaaagcgaatatcgcgtgtccgtcgattctggattattccatcctcaacgataacggctccatgtttaacacgccgccgacatttgcctggtatctatctggtctggtctttaaatggctgaaagcgaacggcggtgtagctgaaatggataaaatcaatcagcaaaaagcagaactgctatatggggtgattgataacagcgatttctaccgcaatgacgtggcgaaagctaaccgttcgcggatgaacgtgccgttccagttggcggacagtgcgcttgacaaattgttccttgaagagtcttttgctgctggccttcatgcactgaaaggtcaccgtgtggtcggcggaatgcgcgcttctatttataacgccatgccgctggaaggcgttaaagcgctgacagacttcatggttgagttcgaacgccgtcacggttgataaaagaaggagaccagtttatgcctaacattacctggtgcgacctgcctgaagatgtctctttatggccgggtctgcctctttcattaagtggtgatgaagtgatgccactggattaccacgcaggtcgtagcggctggctgctgtatggtcgtgggctggataaacaacgtctgacccaataccagagcaaactgggtgcggcgatggtgattgttgccgcctggtgcgtggaagattatcaggtgattcgtctggcaggttcactcaccgcacgggctacacgcctggcccacgaagcgcagctggatgtcgccccgctggggaaaatcccgcacctgcgcacgccgggtttgctggtgatggatatggactccaccgccatccagattgaatgtattgatgaaattgccaaactggccggaacgggcgagatggtggcggaagtaaccgaacgggcgatgcgcggcgaactcgattttaccgccagcctgcgcagccgtgtggcgacgctgaaaggcgctgacgccaatattctgcaacaggtgcgtgaaaatctgccgctgatgccaggcttaacgcaactggtgctcaagctggaaacgctgggctggaaagtggcgattgcctccggcggctttactttctttgctgaatacctgcgcgacaagctgcgcctgaccgccgtggtagccaatgaactggagatcatggacggtaaatttaccggcaatgtgatcggcgacatcgtagacgcgcagtacaaagcgaaaactctgactcgcctcgcgcaggagtatgaaatcccgctggcgcagaccgtggcgattggcgatggagccaatgacctgccgatgatcaaagcggcagggctggggattgcctaccatgccaagccaaaagtgaatgaaaaggcggaagtcaccatccgtcacgctgacctgatgggggtattctgcatcctctcaggcagcctgaatcagaagtgataagctgaggtcgcctcagcggccggcccctgcaggcgccggcgactagtcttggactcctgttgatagatccagtaatgacctcagaactccatctggatttgttcagaacgctcggttgccgccgggcgttttttattggtgagaatccaggggtccccaataattacgatttaaatttgtgtctcaaaatctctgatgttacattgcacaagataaaaatatatcatcatgaacaataaaactgtctgcttacataaacagtaatacaaggggtgttatgagccatattcagcgtgaaacgagctgtagccgtccgcgtctgaacagcaacatggatgcggatctgtatggctataaatgggcgcgtgataacgtgggtcagagcggcgcgaccatttatcgtctgtatggcaaaccggatgcgccggaactgtttctgaaacatggcaaaggcagcgtggcgaacgatgtgaccgatgaaatggtgcgtctgaactggctgaccgaatttatgccgctgccgaccattaaacattttattcgcaccccggatgatgcgtggctgctgaccaccgcgattccgggcaaaaccgcgtttcaggtgctggaagaatatccggatagcggcgaaaacattgtggatgcgctggccgtgtttctgcgtcgtctgcatagcattccggtgtgcaactgcccgtttaacagcgatcgtgtgtttcgtctggcccaggcgcagagccgtatgaacaacggcctggtggatgcgagcgattttgatgatgaacgtaacggctggccggtggaacaggtgtggaaagaaatgcataaactgctgccgtttagcccggatagcgtggtgacccacggcgattttagcctggataacctgattttcgatgaaggcaaactgattggctgcattgatgtgggccgtgtgggcattgcggatcgttatcaggatctggccattctgtggaactgcctgggcgaatttagcccgagcctgcaaaaacgtctgtttcagaaatatggcattgataatccggatatgaacaaactgcaatttcatctgatgctggatgaatttttctaataattaattggaccgttgtccttttccgctgcataaccctgcttcggggtcattatagcgattttttcggtatatccatcctttttcgcacgatatacaggattttgccaaagggttcgtgtagactttccttggtgtatccaacggcgtcagccgggcaggataggtgaagtaggcccacccgcgagcgggtgttccttcttcactgtccct

SEQ ID NO: 35 - DNA, 6784 bp, synthetic construct
  source 1..6784: mol_type = other DNA
tattcgcacctggcggtgctcaacgggaatcctgctctgcgaggctggccgtaggccggcctcagatccttccgtatttagccagtatgttctctagtgtggttcgttgtttttgcgtgagccatgagaacgaaccattgagatcatacttactttgcatgtcactcaaaaattttgcctcaaaactggtgagctgaatttttgcagttaaagcatcgtgtagtgtttttcttagtccgttatgtaggtaggaatctgatgtaatggttgttggtattttgtcaccattcatttttatctggttgttctcaagttcggttacgagatccatttgtctatctagttcaacttggaaaatcaacgtatcagtcgggcggcctcgcttatcaaccaccaatttcatattgctgtaagtgtttaaatctttacttattggtttcaaaacccattggttaagccttttaaactcatggtagttattttcaagcattaacatgaacttaaattcatcaaggctaatctctatatttgccttgtgagttttcttttgtgttagttcttttaataaccactcataaatcctcatagagtatttgttttcaaaagacttaacatgttccagattatattttatgaatttttttaactggaaaagataaggcaatatctcttcactaaaaactaattctaatttttcgcttgagaacttggcatagtttgtccactggaaaatctcaaagcctttaaccaaaggattcctgatttccacagttctcgtcatcagctctctggttgctttagctaatacaccataagcattttccctactgatgttcatcatctgagcgtattggttataagtgaacgataccgtccgttctttccttgtagggttttcaatcgtggggttgagtagtgccacacagcataaaattagcttggtttcatgctccgttaagtcatagcgactaatcgctagttcatttgctttgaaaacaactaattcagacatacatctcaattggtctaggtgattttaatcactataccaattgagatgggctagtcaatgataattacatgtccttttcctttgagttgtgggtatctgtaaattctgctagacctttgctggaaaacttgtaaattctgctagaccctctgtaaattccgctagacctttgtgtgttttttttgtttatattcaagtggttataatttatagaataaagaaagaataaaaaaagataaaaagaatagatcccagccctgtgtataactcactactttagtcagttccgcagtattacaaaaggatgtcgcaaacgctgtttgctcctctacaaaacagaccttaaaaccctaaaggcttaagtagcaccctcgcaagctcgggcaaatcgctgaatattccttttgtctccgaccatcaggcacctgagtcgctgtctttttcgtgacattcagttcgctgcgctcacggctctggcagtgaatgggggtaaatggcactacaggcgcggcgcgcccagctgtctagggcggcggatttgtcctactcaggagagcgttcaccgacaaacaacagataaaacgaaaggcccagtctttcgactgagcctttcgttttatttgatgcctttaattaagcggccgcggcgcgcccgtcgacgcgcgcgcggctgaggatacctcagcataggcctttgacagctagctcagtcctaggtataatgctagctcttaatcatgctaaggaggattcatgttatgagtcagaatggccgtccggtagtcctcatcgccgataagcttgcgcagtccactgttgacgcgcttggagatgcagtagaagtccgttgggttgacggacctaaccgcccagaactgcttgatgcagttaaggaagcggacgcactgctcgtgcgttctgctaccactgtcgatgctgaagtcatcgccgctgcccctaacttgaagatcgtcggtcgtgccggcgtgggcttggacaacgttgacatccctgctgccactgaagctggcgtcatggttgctaacgcaccgacctctaatattcactccgcttgtgagcacgcaatttctttgctgctgtctactgctcgccagatccctgctgctgatgcgacgctgcgtgagggcgagtggaagcggtcttctttcaacggtgtggaaattttcggaaaaactgtcggtatcgtcggttttggccacattggtcagttgtttgctcagcgtcttgctgcgtttgagaccaccattgttgcttacgatccttacgctaaccctgctcgtgcggctcagctgaacgttgagttggttgagttggatgagctgatgagccgttctgactttgtcaccattcaccttcctaagaccaaggaaactgctggcatgtttgatgcgcagctccttgctaagtccaagaagggccagatcatcatcaacgctgctcgtggtggccttgttgatgagcaggctttggctgatgcgattgagtccggtcacattcgtggcgctggtttcgatgtgtactccaccgagccttgcactgattctcctttgttcaagttgcctcaggttgttgtgactcctcacttgggtgggtctactgaagaggctcaggatcgtgcgggtactgacgttgctgattctgtgctcaaggcgctggctggcgagttcgtggcggatgctgtgaacgtttccggtggtcgcgtgggcgaagaggttgctgtgtggatggatctggctcgcaagcttggtcttcttgctggcaagcttgtcgacgccgccccagtctccattgaggttgaggctcgaggcgagctttcttccgagcaggtcgatgcacttggtttgtccgctgttcgtggtttgttctccggaattatcgaagagtccgttactttcgtcaacgctcctcgcattgctgaagagcgtggcctggacatctccgtgaagaccaactctgagtctgttactcaccgttccgtcctgcaggtcaaggtcattactggcagcggcgcgagcgcaactgttgttggtgccctgactggtcttgagcgcgttgagaagatcacccgcatcaatggccgtggcctggatctgcgcgcagagggtctgaacctcttcctgcaggccactgacgctcctggtgcactgggtaccgttggtaccaagctgggtgctgctggcatcaacatcgaggctgctgcgttgactcaggctgagaagggtgacggcgctgtcctgatcctgcgtgttgagtccgctgtctctgaagagctggaagctgaaatcaacgctgagttgggtgctacttccttccaggttgatcttgactaataaagcttggttgataaaagaaggagactttgatatggcgcaaatcttcaattttagttctggtccggcaatgctaccggcagaggtgcttaaacaggctcaacaggaactgcgcgactggaacggtcttggtacgtcggtgatggaagtgagtcaccgtggcaaagagttcattcaggttgcagaggaagccgagaaggattttcgcgatcttcttaatgtcccctccaactacaaggtattattctgccatggcggtggtcgcggtcagtttgctgcggtaccgctgaatattctcggtgataaaaccaccgcagattatgttgatgccggttactgggcggcaagtgccattaaagaagcgaaaaaatactgcacgcctaatgtctttgacgccaaagtgactgttgatggtctgcgcgcggttaagccaatgcgtgaatggcaactctctgataatgctgcttatatgcattattgcccgaatgaaaccatcgatggtatcgccatcgacgaaacgccagacttcggcgcagatgtggtggtcgccgctgacttctcttcaaccattctttcccgtccgattgacgtcagccgttatggtgtaatttacgctggcgcgcagaaaaatatcggcccggctggcctgacaatcgtcatcgttcgtgaagatttgctgggcaaagcgaatatcgcgtgtccgtcgattctggattattccatcctcaacgataacggctccatgtttaacacgccgccgacatttgcctggtatctatctggtctggtctttaaatggctgaaagcgaacggcggtgtagctgaaatggataaaatcaatcagcaaaaagcagaactgctatatggggtgattgataacagcgatttctaccgcaatgacgtggcgaaagctaaccgttcgcggatgaacgtgccgttccagttggcggacagtgcgcttgacaaattgttccttgaagagtcttttgctgctggccttcatgcactgaaaggtcaccgtgtggtcggcggaatgcgcgcttctatttataacgccatgccgctggaaggcgttaaagcgctgacagacttcatggttgagttcgaacgccgtcacggttgataaaagaaggagaccagtttatgcctaacattacctggtgcgacctgcctgaagatgtctctttatggccgggtctgcctctttcattaagtggtgatgaagtgatgccactggattaccacgcaggtcgtagcggctggctgctgtatggtcgtgggctggataaacaacgtctgacccaataccagagcaaactgggtgcggcgatggtgattgttgccgcctggtgcgtggaagattatcaggtgattcgtctggcaggttcactcaccgcacgggctacacgcctggcccacgaagcgcagctggatgtcgccccgctggggaaaatcccgcacctgcgcacgccgggtttgctggtgatggatatggactccaccgccatccagattgaatgtattgatgaaattgccaaactggccggaacgggcgagatggtggcggaagtaaccgaacgggcgatgcgcggcgaactcgattttaccgccagcctgcgcagccgtgtggcgacgctgaaaggcgctgacgccaatattctgcaacaggtgcgtgaaaatctgccgctgatgccaggcttaacgcaactggtgctcaagctggaaacgctgggctggaaagtggcgattgcctccggcggctttactttctttgctgaatacctgcgcgacaagctgcgcctgaccgccgtggtagccaatgaactggagatcatggacggtaaatttaccggcaatgtgatcggcgacatcgtagacgcgcagtacaaagcgaaaactctgactcgcctcgcgcaggagtatgaaatcccgctggcgcagaccgtggcgattggcgatggagccaatgacctgccgatgatcaaagcggcagggctggggattgcctaccatgccaagccaaaagtgaatgaaaaggcggaagtcaccatccgtcacgctgacctgatgggggtattctgcatcctctcaggcagcctgaatcagaagtgataagctgaggtcgcctcagcggccggcccctgcaggcgccggcgactagtcttggactcctgttgatagatccagtaatgacctcagaactccatctggatttgttcagaacgctcggttgccgccgggcgttttttattggtgagaatccaggggtccccaataattacgatttaaatttgtgtctcaaaatctctgatgttacattgcacaagataaaaatatatcatcatgaacaataaaactgtctgcttacataaacagtaatacaaggggtgttatgagccatattcagcgtgaaacgagctgtagccgtccgcgtctgaacagcaacatggatgcggatctgtatggctataaatgggcgcgtgataacgtgggtcagagcggcgcgaccatttatcgtctgtatggcaaaccggatgcgccggaactgtttctgaaacatggcaaaggcagcgtggcgaacgatgtgaccgatgaaatggtgcgtctgaactggctgaccgaatttatgccgctgccgaccattaaacattttattcgcaccccggatgatgcgtggctgctgaccaccgcgattccgggcaaaaccgcgtttcaggtgctggaagaatatccggatagcggcgaaaacattgtggatgcgctggccgtgtttctgcgtcgtctgcatagcattccggtgtgcaactgcccgtttaacagcgatcgtgtgtttcgtctggcccaggcgcagagccgtatgaacaacggcctggtggatgcgagcgattttgatgatgaacgtaacggctggccggtggaacaggtgtggaaagaaatgcataaactgctgccgtttagcccggatagcgtggtgacccacggcgattttagcctggataacctgattttcgatgaaggcaaactgattggctgcattgatgtgggccgtgtgggcattgcggatcgttatcaggatctggccattctgtggaactgcctgggcgaatttagcccgagcctgcaaaaacgtctgtttcagaaatatggcattgataatccggatatgaacaaactgcaatttcatctgatgctggatgaatttttctaataattaattggaccgttgtccttttccgctgcataaccctgcttcggggtcattatagcgattttttcggtatatccatcctttttcgcacgatatacaggattttgccaaagggttcgtgtagactttccttggtgtatccaacggcgtcagccgggcaggataggtgaagtaggcccacccgcgagcgggtgttccttcttcactgtccct

SEQ ID NO: 36 - DNA, 6784 bp, synthetic construct
  source 1..6784: mol_type = other DNA
tattcgcacctggcggtgctcaacgggaatcctgctctgcgaggctggccgtaggccggcctcagatccttccgtatttagccagtatgttctctagtgtggttcgttgtttttgcgtgagccatgagaacgaaccattgagatcatacttactttgcatgtcactcaaaaattttgcctcaaaactggtgagctgaatttttgcagttaaagcatcgtgtagtgtttttcttagtccgttatgtaggtaggaatctgatgtaatggttgttggtattttgtcaccattcatttttatctggttgttctcaagttcggttacgagatccatttgtctatctagttcaacttggaaaatcaacgtatcagtcgggcggcctcgcttatcaaccaccaatttcatattgctgtaagtgtttaaatctttacttattggtttcaaaacccattggttaagccttttaaactcatggtagttattttcaagcattaacatgaacttaaattcatcaaggctaatctctatatttgccttgtgagttttcttttgtgttagttcttttaataaccactcataaatcctcatagagtatttgttttcaaaagacttaacatgttccagattatattttatgaatttttttaactggaaaagataaggcaatatctcttcactaaaaactaattctaatttttcgcttgagaacttggcatagtttgtccactggaaaatctcaaagcctttaaccaaaggattcctgatttccacagttctcgtcatcagctctctggttgctttagctaatacaccataagcattttccctactgatgttcatcatctgagcgtattggttataagtgaacgataccgtccgttctttccttgtagggttttcaatcgtggggttgagtagtgccacacagcataaaattagcttggtttcatgctccgttaagtcatagcgactaatcgctagttcatttgctttgaaaacaactaattcagacatacatctcaattggtctaggtgattttaatcactataccaattgagatgggctagtcaatgataattacatgtccttttcctttgagttgtgggtatctgtaaattctgctagacctttgctggaaaacttgtaaattctgctagaccctctgtaaattccgctagacctttgtgtgttttttttgtttatattcaagtggttataatttatagaataaagaaagaataaaaaaagataaaaagaatagatcccagccctgtgtataactcactactttagtcagttccgcagtattacaaaaggatgtcgcaaacgctgtttgctcctctacaaaacagaccttaaaaccctaaaggcttaagtagcaccctcgcaagctcgggcaaatcgctgaatattccttttgtctccgaccatcaggcacctgagtcgctgtctttttcgtgacattcagttcgctgcgctcacggctctggcagtgaatgggggtaaatggcactacaggcgcggcgcgcccagctgtctagggcggcggatttgtcctactcaggagagcgttcaccgacaaacaacagataaaacgaaaggcccagtctttcgactgagcctttcgttttatttgatgcctttaattaagcggccgcggcgcgcccgtcgacgcgcgcgcggctgaggatacctcagcataggcctttgacagctagctcagtcctaggtataatgctagctcttaatcatgctaaggaggattctgttcatgtctcagaatggccgtccggtagtcctcatcgccgataagcttgcgcagtccactgttgacgcgcttggagatgcagtagaagtccgttgggttgacggacctaaccgcccagaactgcttgatgcagttaaggaagcggacgcactgctcgtgcgttctgctaccactgtcgatgctgaagtcatcgccgctgcccctaacttgaagatcgtcggtcgtgccggcgtgggcttggacaacgttgacatccctgctgccactgaagctggcgtcatggttgctaacgcaccgacctctaatattcactccgcttgtgagcacgcaatttctttgctgctgtctactgctcgccagatccctgctgctgatgcgacgctgcgtgagggcgagtggaagcggtcttctttcaacggtgtggaaattttcggaaaaactgtcggtatcgtcggttttggccacattggtcagttgtttgctcagcgtcttgctgcgtttgagaccaccattgttgcttacgatccttacgctaaccctgctcgtgcggctcagctgaacgttgagttggttgagttggatgagctgatgagccgttctgactttgtcaccattcaccttcctaagaccaaggaaactgctggcatgtttgatgcgcagctccttgctaagtccaagaagggccagatcatcatcaacgctgctcgtggtggccttgttgatgagcaggctttggctgatgcgattgagtccggtcacattcgtggcgctggtttcgatgtgtactccaccgagccttgcactgattctcctttgttcaagttgcctcaggttgttgtgactcctcacttgggtgggtctactgaagaggctcaggatcgtgcgggtactgacgttgctgattctgtgctcaaggcgctggctggcgagttcgtggcggatgctgtgaacgtttccggtggtcgcgtgggcgaagaggttgctgtgtggatggatctggctcgcaagcttggtcttcttgctggcaagcttgtcgacgccgccccagtctccattgaggttgaggctcgaggcgagctttcttccgagcaggtcgatgcacttggtttgtccgctgttcgtggtttgttctccggaattatcgaagagtccgttactttcgtcaacgctcctcgcattgctgaagagcgtggcctggacatctccgtgaagaccaactctgagtctgttactcaccgttccgtcctgcaggtcaaggtcattactggcagcggcgcgagcgcaactgttgttggtgccctgactggtcttgagcgcgttgagaagatcacccgcatcaatggccgtggcctggatctgcgcgcagagggtctgaacctcttcctgcaggccactgacgctcctggtgcactgggtaccgttggtaccaagctgggtgctgctggcatcaacatcgaggctgctgcgttgactcaggctgagaagggtgacggcgctgtcctgatcctgcgtgttgagtccgctgtctctgaagagctggaagctgaaatcaacgctgagttgggtgctacttccttccaggttgatcttgactaataaagcttggttgataaaagaaggagacacccaaatggcccaaatcttcaattttagttctggtccggcaatgctaccggcagaggtgcttaaacaggctcaacaggaactgcgcgactggaacggtcttggtacgtcggtgatggaagtgagtcaccgtggcaaagagttcattcaggttgcagaggaagccgagaaggattttcgcgatcttcttaatgtcccctccaactacaaggtattattctgccatggcggtggtcgcggtcagtttgctgcggtaccgctgaatattctcggtgataaaaccaccgcagattatgttgatgccggttactgggcggcaagtgccattaaagaagcgaaaaaatactgcacgcctaatgtctttgacgccaaagtgactgttgatggtctgcgcgcggttaagccaatgcgtgaatggcaactctctgataatgctgcttatatgcattattgcccgaatgaaaccatcgatggtatcgccatcgacgaaacgccagacttcggcgcagatgtggtggtcgccgctgacttctcttcaaccattctttcccgtccgattgacgtcagccgttatggtgtaatttacgctggcgcgcagaaaaatatcggcccggctggcctgacaatcgtcatcgttcgtgaagatttgctgggcaaagcgaatatcgcgtgtccgtcgattctggattattccatcctcaacgataacggctccatgtttaacacgccgccgacatttgcctggtatctatctggtctggtctttaaatggctgaaagcgaacggcggtgtagctgaaatggataaaatcaatcagcaaaaagcagaactgctatatggggtgattgataacagcgatttctaccgcaatgacgtggcgaaagctaaccgttcgcggatgaacgtgccgttccagttggcggacagtgcgcttgacaaattgttccttgaagagtcttttgctgctggccttcatgcactgaaaggtcaccgtgtggtcggcggaatgcgcgcttctatttataacgccatgccgctggaaggcgttaaagcgctgacagacttcatggttgagttcgaacgccgtcacggttgataaaagaaggagaccagtttatgcctaacattacctggtgcgacctgcctgaagatgtctctttatggccgggtctgcctctttcattaagtggtgatgaagtgatgccactggattaccacgcaggtcgtagcggctggctgctgtatggtcgtgggctggataaacaacgtctgacccaataccagagcaaactgggtgcggcgatggtgattgttgccgcctggtgcgtggaagattatcaggtgattcgtctggcaggttcactcaccgcacgggctacacgcctggcccacgaagcgcagctggatgtcgccccgctggggaaaatcccgcacctgcgcacgccgggtttgctggtgatggatatggactccaccgccatccagattgaatgtattgatgaaattgccaaactggccggaacgggcgagatggtggcggaagtaaccgaacgggcgatgcgcggcgaactcgattttaccgccagcctgcgcagccgtgtggcgacgctgaaaggcgctgacgccaatattctgcaacaggtgcgtgaaaatctgccgctgatgccaggcttaacgcaactggtgctcaagctggaaacgctgggctggaaagtggcgattgcctccggcggctttactttctttgctgaatacctgcgcgacaagctgcgcctgaccgccgtggtagccaatgaactggagatcatggacggtaaatttaccggcaatgtgatcggcgacatcgtagacgcgcagtacaaagcgaaaactctgactcgcctcgcgcaggagtatgaaatcccgctggcgcagaccgtggcgattggcgatggagccaatgacctgccgatgatcaaagcggcagggctggggattgcctaccatgccaagccaaaagtgaatgaaaaggcggaagtcaccatccgtcacgctgacctgatgggggtattctgcatcctctcaggcagcctgaatcagaagtgataagctgaggtcgcctcagcggccggcccctgcaggcgccggcgactagtcttggactcctgttgatagatccagtaatgacctcagaactccatctggatttgttcagaacgctcggttgccgccgggcgttttttattggtgagaatccaggggtccccaataattacgatttaaatttgtgtctcaaaatctctgatgttacattgcacaagataaaaatatatcatcatgaacaataaaactgtctgcttacataaacagtaatacaaggggtgttatgagccatattcagcgtgaaacgagctgtagccgtccgcgtctgaacagcaacatggatgcggatctgtatggctataaatgggcgcgtgataacgtgggtcagagcggcgcgaccatttatcgtctgtatggcaaaccggatgcgccggaactgtttctgaaacatggcaaaggcagcgtggcgaacgatgtgaccgatgaaatggtgcgtctgaactggctgaccgaatttatgccgctgccgaccattaaacattttattcgcaccccggatgatgcgtggctgctgaccaccgcgattccgggcaaaaccgcgtttcaggtgctggaagaatatccggatagcggcgaaaacattgtggatgcgctggccgtgtttctgcgtcgtctgcatagcattccggtgtgcaactgcccgtttaacagcgatcgtgtgtttcgtctggcccaggcgcagagccgtatgaacaacggcctggtggatgcgagcgattttgatgatgaacgtaacggctggccggtggaacaggtgtggaaagaaatgcataaactgctgccgtttagcccggatagcgtggtgacccacggcgattttagcctggataacctgattttcgatgaaggcaaactgattggctgcattgatgtgggccgtgtgggcattgcggatcgttatcaggatctggccattctgtggaactgcctgggcgaatttagcccgagcctgcaaaaacgtctgtttcagaaatatggcattgataatccggatatgaacaaactgcaatttcatctgatgctggatgaatttttctaataattaattggaccgttgtccttttccgctgcataaccctgcttcggggtcattatagcgattttttcggtatatccatcctttttcgcacgatatacaggattttgccaaagggttcgtgtagactttccttggtgtatccaacggcgtcagccgggcaggataggtgaagtaggcccacccgcgagcgggtgttccttcttcactgtccct

SEQ ID NO: 37 - DNA, 6784 bp, synthetic construct
  source 1..6784: mol_type = other DNA
tattcgcacctggcggtgctcaacgggaatcctgctctgcgaggctggccgtaggccggcctcagatccttccgtatttagccagtatgttctctagtgtggttcgttgtttttgcgtgagccatgagaacgaaccattgagatcatacttactttgcatgtcactcaaaaattttgcctcaaaactggtgagctgaatttttgcagttaaagcatcgtgtagtgtttttcttagtccgttatgtaggtaggaatctgatgtaatggttgttggtattttgtcaccattcatttttatctggttgttctcaagttcggttacgagatccatttgtctatctagttcaacttggaaaatcaacgtatcagtcgggcggcctcgcttatcaaccaccaatttcatattgctgtaagtgtttaaatctttacttattggtttcaaaacccattggttaagccttttaaactcatggtagttattttcaagcattaacatgaacttaaattcatcaaggctaatctctatatttgccttgtgagttttcttttgtgttagttcttttaataaccactcataaatcctcatagagtatttgttttcaaaagacttaacatgttccagattatattttatgaatttttttaactggaaaagataaggcaatatctcttcactaaaaactaattctaatttttcgcttgagaacttggcatagtttgtccactggaaaatctcaaagcctttaaccaaaggattcctgatttccacagttctcgtcatcagctctctggttgctttagctaatacaccataagcattttccctactgatgttcatcatctgagcgtattggttataagtgaacgataccgtccgttctttccttgtagggttttcaatcgtggggttgagtagtgccacacagcataaaattagcttggtttcatgctccgttaagtcatagcgactaatcgctagttcatttgctttgaaaacaactaattcagacatacatctcaattggtctaggtgattttaatcactataccaattgagatgggctagtcaatgataattacatgtccttttcctttgagttgtgggtatctgtaaattctgctagacctttgctggaaaacttgtaaattctgctagaccctctgtaaattccgctagacctttgtgtgttttttttgtttatattcaagtggttataatttatagaataaagaaagaataaaaaaagataaaaagaatagatcccagccctgtgtataactcactactttagtcagttccgcagtattacaaaaggatgtcgcaaacgctgtttgctcctctacaaaacagaccttaaaaccctaaaggcttaagtagcaccctcgcaagctcgggcaaatcgctgaatattccttttgtctccgaccatcaggcacctgagtcgctgtctttttcgtgacattcagttcgctgcgctcacggctctggcagtgaatgggggtaaatggcactacaggcgcggcgcgcccagctgtctagggcggcggatttgtcctactcaggagagcgttcaccgacaaacaacagataaaacgaaaggcccagtctttcgactgagcctttcgttttatttgatgcctttaattaagcggccgcggcgcgcccgtcgacgcgcgcgcggctgaggatacctcagcataggcctttgacagctagctcagtcctaggtataatgctagctcttaatcatgctaaggaggattggatacatgtcccaaaatggccgtccggtagtcctcatcgccgataagcttgcgcagtccactgttgacgcgcttggagatgcagtagaagtccgttgggttgacggacctaaccgcccagaactgcttgatgcagttaaggaagcggacgcactgctcgtgcgttctgctaccactgtcgatgctgaagtcatcgccgctgcccctaacttgaagatcgtcggtcgtgccggcgtgggcttggacaacgttgacatccctgctgccactgaagctggcgtcatggttgctaacgcaccgacctctaatattcactccgcttgtgagcacgcaatttctttgctgctgtctactgctcgccagatccctgctgctgatgcgacgctgcgtgagggcgagtggaagcggtcttctttcaacggtgtggaaattttcggaaaaactgtcggtatcgtcggttttggccacattggtcagttgtttgctcagcgtcttgctgcgtttgagaccaccattgttgcttacgatccttacgctaaccctgctcgtgcggctcagctgaacgttgagttggttgagttggatgagctgatgagccgttctgactttgtcaccattcaccttcctaagaccaaggaaactgctggcatgtttgatgcgcagctccttgctaagtccaagaagggccagatcatcatcaacgctgctcgtggtggccttgttgatgagcaggctttggctgatgcgattgagtccggtcacattcgtggcgctggtttcgatgtgtactccaccgagccttgcactgattctcctttgttcaagttgcctcaggttgttgtgactcctcacttgggtgggtctactgaagaggctcaggatcgtgcgggtactgacgttgctgattctgtgctcaaggcgctggctggcgagttcgtggcggatgctgtgaacgtttccggtggtcgcgtgggcgaagaggttgctgtgtggatggatctggctcgcaagcttggtcttcttgctggcaagcttgtcgacgccgccccagtctccattgaggttgaggctcgaggcgagctttcttccgagcaggtcgatgcacttggtttgtccgctgttcgtggtttgttctccggaattatcgaagagtccgttactttcgtcaacgctcctcgcattgctgaagagcgtggcctggacatctccgtgaagaccaactctgagtctgttactcaccgttccgtcctgcaggtcaaggtcattactggcagcggcgcgagcgcaactgttgttggtgccctgactggtcttgagcgcgttgagaagatcacccgcatcaatggccgtggcctggatctgcgcgcagagggtctgaacctcttcctgcaggccactgacgctcctggtgcactgggtaccgttggtaccaagctgggtgctgctggcatcaacatcgaggctgctgcgttgactcaggctgagaagggtgacggcgctgtcctgatcctgcgtgttgagtccgctgtctctgaagagctggaagctgaaatcaacgctgagttgggtgctacttccttccaggttgatcttgactaataaagcttggttgataaaagaaggagaccccggaatggcacaaatcttcaattttagttctggtccggcaatgctaccggcagaggtgcttaaacaggctcaacaggaactgcgcgactggaacggtcttggtacgtcggtgatggaagtgagtcaccgtggcaaagagttcattcaggttgcagaggaagccgagaaggattttcgcgatcttcttaatgtcccctccaactacaaggtattattctgccatggcggtggtcgcggtcagtttgctgcggtaccgctgaatattctcggtgataaaaccaccgcagattatgttgatgccggttactgggcggcaagtgccattaaagaagcgaaaaaatactgcacgcctaatgtctttgacgccaaagtgactgttgatggtctgcgcgcggttaagccaatgcgtgaatggcaactctctgataatgctgcttatatgcattattgcccgaatgaaaccatcgatggtatcgccatcgacgaaacgccagacttcggcgcagatgtggtggtcgccgctgacttctcttcaaccattctttcccgtccgattgacgtcagccgttatggtgtaatttacgctggcgcgcagaaaaatatcggcccggctggcctgacaatcgtcatcgttcgtgaagatttgctgggcaaagcgaatatcgcgtgtccgtcgattctggattattccatcctcaacgataacggctccatgtttaacacgccgccgacatttgcctggtatctatctggtctggtctttaaatggctgaaagcgaacggcggtgtagctgaaatggataaaatcaatcagcaaaaagcagaactgctatatggggtgattgataacagcgatttctaccgcaatgacgtggcgaaagctaaccgttcgcggatgaacgtgccgttccagttggcggacagtgcgcttgacaaattgttccttgaagagtcttttgctgctggccttcatgcactgaaaggtcaccgtgtggtcggcggaatgcgcgcttctatttataacgccatgccgctggaaggcgttaaagcgctgacagacttcatggttgagttcgaacgccgtcacggttgataaaagaaggagaccagtttatgcctaacattacctggtgcgacctgcctgaagatgtctctttatggccgggtctgcctctttcattaagtggtgatgaagtgatgccactggattaccacgcaggtcgtagcggctggctgctgtatggtcgtgggctggataaacaacgtctgacccaataccagagcaaactgggtgcggcgatggtgattgttgccgcctggtgcgtggaagattatcaggtgattcgtctggcaggttcactcaccgcacgggctacacgcctggcccacgaagcgcagctggatgtcgccccgctggggaaaatcccgcacctgcgcacgccgggtttgctggtgatggatatggactccaccgccatccagattgaatgtattgatgaaattgccaaactggccggaacgggcgagatggtggcggaagtaaccgaacgggcgatgcgcggcgaactcgattttaccgccagcctgcgcagccgtgtggcgacgctgaaaggcgctgacgccaatattctgcaacaggtgcgtgaaaatctgccgctgatgccaggcttaacgcaactggtgctcaagctggaaacgctgggctggaaagtggcgattgcctccggcggctttactttctttgctgaatacctgcgcgacaagctgcgcctgaccgccgtggtagccaatgaactggagatcatggacggtaaatttaccggcaatgtgatcggcgacatcgtagacgcgcagtacaaagcgaaaactctgactcgcctcgcgcaggagtatgaaatcccgctggcgcagaccgtggcgattggcgatggagccaatgacctgccgatgatcaaagcggcagggctggggattgcctaccatgccaagccaaaagtgaatgaaaaggcggaagtcaccatccgtcacgctgacctgatgggggtattctgcatcctctcaggcagcctgaatcagaagtgataagctgaggtcgcctcagcggccggcccctgcaggcgccggcgactagtcttggactcctgttgatagatccagtaatgacctcagaactccatctggatttgttcagaacgctcggttgccgccgggcgttttttattggtgagaatccaggggtccccaataattacgatttaaatttgtgtctcaaaatctctgatgttacattgcacaagataaaaatatatcatcatgaacaataaaactgtctgcttacataaacagtaatacaaggggtgttatgagccatattcagcgtgaaacgagctgtagccgtccgcgtctgaacagcaacatggatgcggatctgtatggctataaatgggcgcgtgataacgtgggtcagagcggcgcgaccatttatcgtctgtatggcaaaccggatgcgccggaactgtttctgaaacatggcaaaggcagcgtggcgaacgatgtgaccgatgaaatggtgcgtctgaactggctgaccgaatttatgccgctgccgaccattaaacattttattcgcaccccggatgatgcgtggctgctgaccaccgcgattccgggcaaaaccgcgtttcaggtgctggaagaatatccggatagcggcgaaaacattgtggatgcgctggccgtgtttctgcgtcgtctgcatagcattccggtgtgcaactgcccgtttaacagcgatcgtgtgtttcgtctggcccaggcgcagagccgtatgaacaacggcctggtggatgcgagcgattttgatgatgaacgtaacggctggccggtggaacaggtgtggaaagaaatgcataaactgctgccgtttagcccggatagcgtggtgacccacggcgattttagcctggataacctgattttcgatgaaggcaaactgattggctgcattgatgtgggccgtgtgggcattgcggatcgttatcaggatctggccattctgtggaactgcctgggcgaatttagcccgagcctgcaaaaacgtctgtttcagaaatatggcattgataatccggatatgaacaaactgcaatttcatctgatgctggatgaatttttctaataattaattggaccgttgtccttttccgctgcataaccctgcttcggggtcattatagcgattttttcggtatatccatcctttttcgcacgatatacaggattttgccaaagggttcgtgtagactttccttggtgtatccaacggcgtcagccgggcaggataggtgaagtaggcccacccgcgagcgggtgttccttcttcactgtccct

SEQ ID NO: 38 - DNA, 6781 bp, synthetic construct
  source 1..6781: mol_type = other DNA
tattcgcacctggcggtgctcaacgggaatcctgctctgcgaggctggccgtaggccggcctcagatccttccgtatttagccagtatgttctctagtgtggttcgttgtttttgcgtgagccatgagaacgaaccattgagatcatacttactttgcatgtcactcaaaaattttgcctcaaaactggtgagctgaatttttgcagttaaagcatcgtgtagtgtttttcttagtccgttatgtaggtaggaatctgatgtaatggttgttggtattttgtcaccattcatttttatctggttgttctcaagttcggttacgagatccatttgtctatctagttcaacttggaaaatcaacgtatcagtcgggcggcctcgcttatcaaccaccaatttcatattgctgtaagtgtttaaatctttacttattggtttcaaaacccattggttaagccttttaaactcatggtagttattttcaagcattaacatgaacttaaattcatcaaggctaatctctatatttgccttgtgagttttcttttgtgttagttcttttaataaccactcataaatcctcatagagtatttgttttcaaaagacttaacatgttccagattatattttatgaatttttttaactggaaaagataaggcaatatctcttcactaaaaactaattctaatttttcgcttgagaacttggcatagtttgtccactggaaaatatcaaagcctttaaccaaaggattcctgatttccacagttctcgtcatcagctctctggttgctttagctaatacaccataagcattttccctactgatgttcatcatctgagcgtattggttataagtgaacgataccgtccgttctttccttgtagggttttcaatcgtggggttgagtagtgccacacagcataaaattagcttggtttcatgctccgttaagtcatagcgactaatcgctagttcatttgctttgaaaacaactaattcagacatacatctcaattggtctaggtgattttaatcactataccaattgagatgggctagtcaatgataattacatgtccttttcctttgagttgtgggtatctgtaaattctgctagacctttgctggaaaacttgtaaattctgctagaccctctgtaaattccgctagacctttgtgtgttttttttgtttatattcaagtggttataatttatagaataaagaaagaataaaaaaagataaaaagaatagatcccagccctgtgtataactcactactttagtcagttccgcagtattacaaaaggatgtcgcaaacgctgtttgctcctctacaaaacagaccttaaaaccctaaaggcttaagtagcaccctcgcaagctcgggcaaatcgctgaatattccttttgtctccgaccatcaggcacctgagtcgctgtctttttcgtgacattcagttcgctgcgctcacggctctggcagtgaatgggggtaaatggcactacaggcgcggcgcgcccagctgtctagggcggcggatttgtcctactcaggagagcgttcaccgacaaacaacagataaaacgaaaggcccagtctttcgactgagcctttcgttttatttgatgcctttaattaagcggccgcggcgcgcccgtcgacgcgcgcgcggctgaggatacctcagcataggcctttgacagctagctcagtcctaggtataatgctagctcttaatcatgctaaggaggattggttttatgagccaaaatggccgtccggtagtcctcatcgccgataagcttgcgcagtccactgttgacgcgcttggagatgcagtagaagtccgttgggttgacggacctaaccgcccagaactgcttgatgcagttaaggaagcggacgcactgctcgtgcgttctgctaccactgtcgatgctgaagtcatcgccgctgcccctaacttgaagatcgtcggtcgtgccggcgtgggcttggacaacgttgacatccctgctgccactgaagctggcgtcatggttgctaacgcaccgacctctaatattcactccgcttgtgagcacgcaatttctttgctgctgtctactgctcgccagatccctgctgctgatgcgacgctgcgtgagggcgagtggaagcggtcttctttcaacggtgtggaaattttcggaaaaactgtcggtatcgtcggttttggccacattggtcagttgtttgctcagcgtcttgctgcgtttgagaccaccattgttgcttacgatccttacgctaaccctgctcgtgcggctcagctgaacgttgagttggttgagttggatgagctgatgagccgttctgactttgtcaccattcaccttcctaagaccaaggaaactgctggcatgtttgatgcgcagctccttgctaagtccaagaagggccagatcatcatcaacgctgctcgtggtggccttgttgatgagcaggctttggctgatgcgattgagtccggtcacattcgtggcgctggtttcgatgtgtactccaccgagccttgcactgattctcctttgttcaagttgcctcaggttgttgtgactcctcacttgggtgggtctactgaagaggctcaggatcgtgcgggtactgacgttgctgattctgtgctcaaggcgctggctggcgagttcgtggcggatgctgtgaacgtttccggtggtcgcgtgggcgaagaggttgctgtgtggatggatctggctcgcaagcttggtcttcttgctggcaagcttgtcgacgccgccccagtctccattgaggttgaggctcgaggcgagctttcttccgagcaggtcgatgcacttggtttgtccgctgttcgtggtttgttctccggaattatcgaagagtccgttactttcgtcaacgctcctcgcattgctgaagagcgtggcctggacatctccgtgaagaccaactctgagtctgttactcaccgttccgtcctgcaggtcaaggtcattactggcagcggcgcgagcgcaactgttgttggtgccctgactggtcttgagcgcgttgagaagatcacccgcatcaatggccgtggcctggatctgcgcgcagagggtctgaacctcttcctgcaggccactgacgctcctggtgcactgggtaccgttggtaccaagctgggtgctgctggcatcaacatcgaggctgctgcgttgactcaggctgagaagggtgacggcgctgtcctgatcctgcgtgttgagtccgctgtctctgaagagctggaagctgaaatcaacgctgagttgggtgctacttccttccaggttgatcttgactaataaagcttggttgataaaagaaggagacttccacatggcccaaatcttcaattttagttctggtccggcaatgctaccggcagaggtgcttaaacaggctcaacaggaactgcgcgactggaacggtcttggtacgtcggtgatggaagtgagtcaccgtggcaaagagttcattcaggttgcagaggaagccgagaaggattttcgcgatcttcttaatgtcccctccaactacaaggtattattctgccatggcggtggtcgcggtcagtttgctgcggtaccgctgaatattctcggtgataaaaccaccgcagattatgttgatgccggttactgggcggcaagtgccattaaagaagcgaaaaaatactgcacgcctaatgtctttgacgccaaagtgactgttgatggtctgcgcgcggttaagccaatgcgtgaatggcaactctctgataatgctgcttatatgcattattgcccgaatgaaaccatcgatggtatcgccatcgacgaaacgccagacttcggcgcagatgtggtggtcgccgctgacttctcttcaaccattctttcccgtccgattgacgtcagccgttatggtgtaatttacgctggcgcgcagaaaaatatcggcccggctggcctgacaatcgtcatcgttcgtgaagatttgctgggcaaagcgaatatcgcgtgtccgtcgattctggattattccatcctcaacgataacggctccatgtttaacacgccgccgacatttgcctggtatctatctggtctggtctttaaatggctgaaagcgaacggcggtgtagctgaaatggataaaatcaatcagcaaaaagcagaactgctatatggggtgattgataacagcgatttctaccgcaatgacgtggcgaaagctaaccgttcgcggatgaacgtgccgttccagttggcggacagtgcgcttgacaaattgttccttgaagagtcttttgctgctggccttcatgcactgaaaggtcaccgtgtggtcggcggaatgcgcgcttctatttataacgccatgccgctggaaggcgttaaagcgctgacagacttcatggttgagttcgaacgccgtcacggttgataaaagaaggagaccagtttatgcctaacattacctggtgcgacctgcctgaagatgtctctttatggccgggtctgcctctttcattaagtggtgatgaagtgatgccactggattaccacgcaggtcgtagcggctggctgctgtatggtcgtgggctggataaacaacgtctgacccaataccagagcaaactgggtgcggcgatggtgattgttgccgcctggtgcgtggaagattatcaggtgattcgtctggcaggttcactcaccgcacgggctacacgcctggcccacgaagcgcagctggatgtcgccccgctggggaaaatcccgcacctgcgcacgccgggtttgctggtgatggatatggactccaccgccatccagattgaatgtattgatgaaattgccaaactggccggaacgggcgagatggtggcggaagtaaccgaacgggcgatgcgcggcgaactcgattttaccgccagcctgcgcagccgtgtggcgacgctgaaaggcgctgacgccaatattctgcaacaggtgcgtgaaaatctgccgctgatgccaggcttaacgcaactggtgctcaagctggaaacgctgggctggaaagtggcgattgcctccggcggctttactttctttgctgaatacctgcgcgacaagctgcgcctgaccgccgtggtagccaatgaactggagatcatggacggtaaatttaccggcaatgtgatcggcgacatcgtagacgcgcagtacaaagcgaaaactctgactcgcctcgcgcaggagtatgaaatcccgctggcgcagaccgtggcgattggcgatggagccaatgacctgccgatgatcaaagcggcagggctggggattgcctaccatgccaagccaaaagtgaatgaaaaggcggaagtcaccatccgtcacgctgacctgatgggggtattctgcatcctctcaggcagcctgaatcagaagtaaagctgaggtcgcctcagcggccggcccctgcaggcgccggcgactagtcttggactcctgttgatagatccagtaatgacctcagaactccatctggatttgttcagaacgctcggttgccgccgggcgttttttattggtgagaatccaggggtccccaataattacgatttaaatttgtgtctcaaaatctctgatgttacattgcacaagataaaaatatatcatcatgaacaataaaactgtctgcttacataaacagtaatacaaggggtgttatgagccatattcagcgtgaaacgagctgtagccgtccgcgtctgaacagcaacatggatgcggatttgtatggctataaatgggcgcgtgataacgtgggtcagagcggcgcgaccatttatcgtctgtatggcaaaccggatgcgccggaactgtttctgaaacatggcaaaggcagcgtggcgaacgatgtgaccgatgaaatggtgcgtctgaactggctgaccgaatttatgccgctgccgaccattaaacattttattcgcaccccggatgatgcgtggctgctgaccaccgcgattccgggcaaaaccgcgtttcaggtgctggaagaatatccggatagcggcgaaaacattgtggatgcgctggccgtgtttctgcgtcgtctgcatagcattccggtgtgcaactgcccgtttaacagcgatcgtgtgtttcgtctggcccaggcgcagagccgtatgaacaacggcctggtggatgcgagcgattttgatgatgaacgtaacggctggccggtggaacaggtgtggaaagaaatgcataaactgctgccgtttagcccggatagcgtggtgacccacggcgattttagcctggataacctgattttcgatgaaggcaaactgattggctgcattgatgtgggccgtgtgggcattgcggatcgttatcaggatctggccattctgtggaactgcctgggcgaatttagcccgagcctgcaaaaacgtctgtttcagaaatatggcattgataatccggatatgaacaaactgcaatttcatctgatgctggatgaatttttctaataattaattggaccgtgtccttttccgctgcataaccctgcttcggggtcattatagcgattttttcggtatatccatcctttttcgcacgatatacaggattttgccaaagggttcgtgtagactttccttggtgtatccaacggcgtcagccgggcaggataggtgaagtaggcccacccgcgagcgggtgttccttcttcactgtccct

SEQ ID NO: 39 - DNA, 6781 bp, synthetic construct
  source 1..6781: mol_type = other DNA
tattcgcacctggcggtgctcaacgggaatcttgctctgcgaggctggccgtaggccggcctcagatccttccgtatttagccagtatgttctctagtgtggttcgttgtttttgcgtgagccatgagaacgaaccattgagatcatacttactttgcatgtcactcaaaaattttgcctcaaaactggtgagctgaatttttgcagttaaagcatcgtgtagtgtttttcttagtccgttatgtaggtaggaatctgatgtaatggttgttggtattttgtcaccattcatttttatctggttgttctcaagttcggttacgagatccatttgtctatctagttcaacttggaaaatcaacgtatcagtcgggcggcctcgcttatcaaccaccaatttcatattgctgtaagtgtttaaatctttacttattggtttcaaaacccattggttaagccttttaaactcatggtagttattttcaagcattaacatgaacttaaattcatcaaggctaatctctatatttgccttgtgagttttcttttgtgttagttcttttaataaccactcataaatcctcatagagtatttgttttcaaaagacttaacatgttccagattatattttatgaatttttttaactggaaaagataaggcaatatctcttcactaaaaactaattctaatttttcgcttgagaacttggcatagtttgtccactggaaaatatcaaagcctttaaccaaaggattcctgatttccacagttctcgtcatcagctctctggttgctttagctaatacaccataagcattttccctactgatgttcatcatctgagcgtattggttataagtgaacgataccgtccgttctttccttgtagggttttcaatcgtggggttgagtagtgccacacagcataaaattagcttggtttcatgctccgttaagtcatagcgactaatcgctagttcatttgctttgaaaacaactaattcagacatacatctcaattggtctaggtgattttaatcactataccaattgagatgggctagtcaatgataattacatgtccttttcctttgagttgtgggtatctgtaaattctgctagacctttgctggaaaacttgtaaattctgctagaccctctgtaaattccgctagacctttgtgtgttttttttgtttatattcaagtggttataatttatagaataaagaaagaataaaaaaagataaaaagaatagatcccagccctgtgtataactcactactttagtcagttccgcagtattacaaaaggatgtcgcaaacgctgtttgctcctctacaaaacagaccttaaaaccctaaaggcttaagtagcaccctcgcaagctcgggcaaatcgctgaatattccttttgtctccgaccatcaggcacctgagtcgctgtctttttcgtgacattcagttcgctgcgctcacggctctggcagtgaatgggggtaaatggcactacaggcgcggcgcgcccagctgtctagggcggcggatttgtcctactcaggagagcgttcaccgacaaacaacagataaaacgaaaggcccagtctttcgactgagcctttcgttttatttgatgcctttaattaagcggccgcggcgcgcccgtcgacgcgcgcgcggctgaggatacctcagcataggcctttgacagctagctcagtcctaggtataatgctagctcttaatcatgctaaggaggattcgccttatgtctcagaatggccgtccggtagtcctcatcgccgataagcttgcgcagtccactgttgacgcgcttggagatgcagtagaagtccgttgggttgacggacctaaccgcccagaactgcttgatgcagttaaggaagcggacgcactgctcgtgcgttctgctaccactgtcgatgctgaagtcatcgccgctgcccctaacttgaagatcgtcggtcgtgccggcgtgggcttggacaacgttgacatccctgctgccactgaagctggcgtcatggttgctaacgcaccgacctctaatattcactccgcttgtgagcacgcaatttctttgctgctgtctactgctcgccagatccctgctgctgatgcgacgctgcgtgagggcgagtggaagcggtcttctttcaacggtgtggaaattttcggaaaaactgtcggtatcgtcggttttggccacattggtcagttgtttgctcagcgtcttgctgcgtttgagaccaccattgttgcttacgatccttacgctaaccctgctcgtgcggctcagctgaacgttgagttggttgagttggatgagctgatgagccgttctgactttgtcaccattcaccttcctaagaccaaggaaactgctggcatgtttgatgcgcagctccttgctaagtccaagaagggccagatcatcatcaacgctgctcgtggtggccttgttgatgagcaggctttggctgatgcgattgagtccggtcacattcgtggcgctggtttcgatgtgtactccaccgagccttgcactgattctcctttgttcaagttgcctcaggttgttgtgactcctcacttgggtgggtctactgaagaggctcaggatcgtgcgggtactgacgttgctgattctgtgctcaaggcgctggctggcgagttcgtggcggatgctgtgaacgtttccggtggtcgcgtgggcgaagaggttgctgtgtggatggatctggctcgcaagcttggtcttcttgctggcaagcttgtcgacgccgccccagtctccattgaggttgaggctcgaggcgagctttcttccgagcaggtcgatgcacttggtttgtccgctgttcgtggtttgttctccggaattatcgaagagtccgttactttcgtcaacgctcctcgcattgctgaagagcgtggcctggacatctccgtgaagaccaactctgagtctgttactcaccgttccgtcctgcaggtcaaggtcattactggcagcggcgcgagcgcaactgttgttggtgccctgactggtcttgagcgcgttgagaagatcacccgcatcaatggccgtggcctggatctgcgcgcagagggtctgaacctcttcctgcaggccactgacgctcctggtgcactgggtaccgttggtaccaagctgggtgctgctggcatcaacatcgaggctgctgcgttgactcaggctgagaagggtgacggcgctgtcctgatcctgcgtgttgagtccgctgtctctgaagagctggaagctgaaatcaacgctgagttgggtgctacttccttccaggttgatcttgactaataaagcttggttgataaaagaaggagactacactatggctcagatcttcaattttagttctggtccggcaatgctaccggcagaggtgcttaaacaggctcaacaggaactgcgcgactggaacggtcttggtacgtcggtgatggaagtgagtcaccgtggcaaagagttcattcaggttgcagaggaagccgagaaggattttcgcgatcttcttaatgtcccctccaactacaaggtattattctgccatggcggtggtcgcggtcagtttgctgcggtaccgctgaatattctcggtgataaaaccaccgcagattatgttgatgccggttactgggcggcaagtgccattaaagaagcgaaaaaatactgcacgcctaatgtctttgacgccaaagtgactgttgatggtctgcgcgcggttaagccaatgcgtgaatggcaactctctgataatgctgcttatatgcattattgcccgaatgaaaccatcgatggtatcgccatcgacgaaacgccagacttcggcgcagatgtggtggtcgccgctgacttctcttcaaccattctttcccgtccgattgacgtcagccgttatggtgtaatttacgctggcgcgcagaaaaatatcggcccggctggcctgacaatcgtcatcgttcgtgaagatttgctgggcaaagcgaatatcgcgtgtccgtcgattctggattattccatcctcaacgataacggctccatgtttaacacgccgccgacatttgcctggtatctatctggtctggtctttaaatggctgaaagcgaacggcggtgtagctgaaatggataaaatcaatcagcaaaaagcagaactgctatatggggtgattgataacagcgatttctaccgcaatgacgtggcgaaagctaaccgttcgcggatgaacgtgccgttccagttggcggacagtgcgcttgacaaattgttccttgaagagtcttttgctgctggccttcatgcactgaaaggtcaccgtgtggtcggcggaatgcgcgcttctatttataacgccatgccgctggaaggcgttaaagcgctgacagacttcatggttgagttcgaacgccgtcacggttgataaaagaaggagaccagtttatgcctaacattacctggtgcgacctgcctgaagatgtctctttatggccgggtctgcctctttcattaagtggtgatgaagtgatgccactggattaccacgcaggtcgtagcggctggctgctgtatggtcgtgggctggataaacaacgtctgacccaataccagagcaaactgggtgcggcgatggtgattgttgccgcctggtgcgtggaagattatcaggtgattcgtctggcaggttcactcaccgcacgggctacacgcctggcccacgaagcgcagctggatgtcgccccgctggggaaaatcccgcacctgcgcacgccgggtttgctggtgatggatatggactccaccgccatccagattgaatgtattgatgaaattgccaaactggccggaacgggcgagatggtggcggaagtaaccgaacgggcgatgcgcggcgaactcgattttaccgccagcctgcgcagccgtgtggcgacgctgaaaggcgctgacgccaatattctgcaacaggtgcgtgaaaatctgccgctgatgccaggcttaacgcaactggtgctcaagctggaaacgctgggctggaaagtggcgattgcctccggcggctttactttctttgctgaatacctgcgcgacaagctgcgcctgaccgccgtggtagccaatgaactggagatcatggacggtaaatttaccggcaatgtgatcggcgacatcgtagacgcgcagtacaaagcgaaaactctgactcgcctcgcgcaggagtatgaaatcccgctggcgcagaccgtggcgattggcgatggagccaatgacctgccgatgatcaaagcggcagggctggggattgcctaccatgccaagccaaaagtgaatgaaaaggcggaagtcaccatccgtcacgctgacctgatgggggtattctgcatcctctcaggcagcctgaatcagaagtaaagctgaggtcgcctcagcggccggcccctgcaggcgccggcgactagtcttggactcctgttgatagatccagtaatgacctcagaactccatctggatttgttcagaacgctcggttgccgccgggcgttttttattggtgagaatccaggggtccccaataattacgatttaaatttgtgtctcaaaatctctgatgttacattgcacaagataaaaatatatcatcatgaacaataaaactgtctgcttacataaacagtaatacaaggggtgttatgagccatattcagcgtgaaacgagctgtagccgtccgcgtctgaacagcaacatggatgcggatttgtatggctataaatgggcgcgtgataacgtgggtcagagcggcgcgaccatttatcgtctgtatggcaaaccggatgcgccggaactgtttctgaaacatggcaaaggcagcgtggcgaacgatgtgaccgatgaaatggtgcgtctgaactggctgaccgaatttatgccgctgccgaccattaaacattttattcgcaccccggatgatgcgtggctgctgaccaccgcgattccgggcaaaaccgcgtttcaggtgctggaagaatatccggatagcggcgaaaacattgtggatgcgctggccgtgtttctgcgtcgtctgcatagcattccggtgtgcaactgcccgtttaacagcgatcgtgtgtttcgtctggcccaggcgcagagccgtatgaacaacggcctggtggatgcgagcgattttgatgatgaacgtaacggctggccggtggaacaggtgtggaaagaaatgcataaactgctgccgtttagcccggatagcgtggtgacccacggcgattttagcctggataacctgattttcgatgaaggcaaactgattggctgcattgatgtgggccgtgtgggcattgcggatcgttatcaggatctggccattctgtggaactgcctgggcgaatttagcccgagcctgcaaaaacgtctgtttcagaaatatggcattgataatccggatatgaacaaactgcaatttcatctgatgctggatgaatttttctaataattaattggaccgtgtccttttccgctgcataaccctgcttcggggtcattatagcgattttttcggtatatccatcctttttcgcacgatatacaggattttgccaaagggttcgtgtagactttccttggtgtatccaacggcgtcagccgggcaggataggtgaagtaggcccacccgcgagcgggtgttccttcttcactgtccct

SEQ ID NO: 40 - DNA, 6783 bp, synthetic construct
  source 1..6783: mol_type = other DNA
tattcgcacctggcggtgctcaacgggaatcctgctctgcgaggctggccgtaggccggcctcagatccttccgtatttagccagtatgttctctagtgtggttcgttgtttttgcgtgagccatgagaacgaaccattgagatcatacttactttgcatgtcactcaaaaattttgcctcaaaactggtgagctgaatttttgcagttaaagcatcgtgtagtgtttttcttagtccgttatgtaggtaggaatctgatgtaatggttgttggtattttgtcaccattcatttttatctggttgttctcaagttcggttacgagatccatttgtctatctagttcaacttggaaaatcaacgtatcagtcgggcggcctcgcttatcaaccaccaatttcatattgctgtaagtgtttaaatctttacttattggtttcaaaacccattggttaagccttttaaactcatggtagttattttcaagcattaacatgaacttaaattcatcaaggctaatctctatatttgccttgtgagttttcttttgtgttagttcttttaataaccactcataaatcctcatagagtatttgttttcaaaagacttaacatgttccagattatattttatgaatttttttaactggaaaagataaggcaatatctcttcactaaaaactaattctaatttttcgcttgagaacttggcatagtttgtccactggaaaatctcaaagcctttaaccaaaggattcctgatttccacagttctcgtcatcagctctctggttgctttagctaatacaccataagcattttccctactgatgttcatcatctgagcgtattggttataagtgaacgataccgtccgttctttccttgtagggttttcaatcgtggggttgagtagtgccacacagcataaaattagcttggtttcatgctccgttaagtcatagcgactaatcgctagttcatttgctttgaaaacaactaattcagacatacatctcaattggtctaggtgattttaatcactataccaattgagatgggctagtcaatgataattacatgtccttttcctttgagttgtgggtatctgtaaattctgctagacctttgctggaaaacttgtaaattctgctagaccctctgtaaattccgctagacctttgtgtgttttttttgtttatattcaagtggttataatttatagaataaagaaagaataaaaaaagataaaaagaatagatcccagccctgtgtataactcactactttagtcagttccgcagtattacaaaaggatgtcgcaaacgctgtttgctcctctacaaaacagaccttaaaaccctaaaggcttaagtagcaccctcgcaagctcgggcaaatcgctgaatattccttttgtctccgaccatcaggcacctgagtcgctgtctttttcgtgacattcagttcgctgcgctcacggctctggcagtgaatgggggtaaatggcactacaggcgcggcgcgcccagctgtctagggcggcggatttgtcctactcaggagagcgttcaccgacaaacaacagataaaacgaaaggcccagtctttcgactgagcctttcgttttatttgatgcctttaattaagcggccgcggcgcgcccgtcgacgcgcgcgcggctgaggatacctcagcataggcctttgacagctagctcagtcctaggtataatgctagctcttaatcatgctaaggaggattttcgaaatgtcgcaaaatggccgtccggtagtcctcatcgccgataagcttgcgcagtccactgttgacgcgcttggagatgcagtagaagtccgttgggttgacggacctaaccgcccagaactgcttgatgcagttaaggaagcggacgcactgctcgtgcgttctgctaccactgtcgatgctgaagtcatcgccgctgcccctaacttgaagatcgtcggtcgtgccggcgtgggcttggacaacgttgacatccctgctgccactgaagctggcgtcatggttgctaacgcaccgacctctaatattcactccgcttgtgagcacgcaatttctttgctgctgtctactgctcgccagatccctgctgctgatgcgacgctgcgtgagggcgagtggaagcggtcttctttcaacggtgtggaaattttcggaaaaactgtcggtatcgtcggttttggccacattggtcagttgtttgctcagcgtcttgctgcgtttgagaccaccattgttgcttacgatccttacgctaaccctgctcgtgcggctcagctgaacgttgagttggttgagttggatgagctgatgagccgttctgactttgtcaccattcaccttcctaagaccaaggaaactgctggcatgtttgatgcgcagctccttgctaagtccaagaagggccagatcatcatcaacgctgctcgtggtggccttgttgatgagcaggctttggctgatgcgattgagtccggtcacattcgtggcgctggtttcgatgtgtactccaccgagccttgcactgattctcctttgttcaagttgcctcaggttgttgtgactcctcacttgggtgggtctactgaagaggctcaggatcgtgcgggtactgacgttgctgattctgtgctcaaggcgctggctggcgagttcgtggcggatgctgtgaacgtttccggtggtcgcgtgggcgaagaggttgctgtgtggatggatctggctcgcaagcttggtcttcttgctggcaagcttgtcgacgccgccccagtctccattgaggttgaggctcgaggcgagctttcttccgagcaggtcgatgcacttggtttgtccgctgttcgtggtttgttctccggaattatcgaagagtccgttactttcgtcaacgctcctcgcattgctgaagagcgtggcctggacatctccgtgaagaccaactctgagtctgttactcaccgttccgtcctgcaggtcaaggtcattactggcagcggcgcgagcgcaactgttgttggtgccctgactggtcttgagcgcgttgagaagatcacccgcatcaatggccgtggcctggatctgcgcgcagagggtctgaacctcttcctgcaggccactgacgctcctggtgcactgggtaccgttggtaccaagctgggtgctgctggcatcaacatcgaggctgctgcgttgactcaggctgagaagggtgacggcgctgtcctgatcctgcgtgttgagtccgctgtctctgaagagctggaagctgaaatcaacgctgagttgggtgctacttccttccaggttgatcttgactaataaagcttggttgataaaagaaggagactaccctatggcacagtcttcaattttagttctggtccggcaatgctaccggcagaggtgcttaaacaggctcaacaggaactgcgcgactggaacggtcttggtacgtcggtgatggaagtgagtcaccgtggcaaagagttcattcaggttgcagaggaagccgagaaggattttcgcgatcttcttaatgtcccctccaactacaaggtattattctgccatggcggtggtcgcggtcagtttgctgcggtaccgctgaatattctcggtgataaaaccaccgcagattatgttgatgccggttactgggcggcaagtgccattaaagaagcgaaaaaatactgcacgcctaatgtctttgacgccaaagtgactgttgatggtctgcgcgcggttaagccaatgcgtgaatggcaactctctgataatgctgcttatatgcattattgcccgaatgaaaccatcgatggtatcgccatcgacgaaacgccagacttcggcgcagatgtggtggtcgccgctgacttctcttcaaccattctttcccgtccgattgacgtcagccgttatggtgtaatttacgctggcgcgcagaaaaatatcggcccggctggcctgacaatcgtcatcgttcgtgaagatttgctgggcaaagcgaatatcgcgtgtccgtcgattctggattattccatcctcaacgataacggctccatgtttaacacgccgccgacatttgcctggtatctatctggtctggtctttaaatggctgaaagcgaacggcggtgtagctgaaatggataaaatcaatcagcaaaaagcagaactgctatatggggtgattgataacagcgatttctaccgcaatgacgtggcgaaagctaaccgttcgcggatgaacgtgccgttccagttggcggacagtgcgcttgacaaattgttccttgaagagtcttttgctgctggccttcatgcactgaaaggtcaccgtgtggtcggcggaatgcgcgcttctatttataacgccatgccgctggaaggcgttaaagcgctgacagacttcatggttgagttcgaacgccgtcacggttgataaaagaaggagaccagtttatgcctaacattacctggtgcgacctgcctgaagatgtctctttatggccgggtctgcctctttcattaagtggtgatgaagtgatgccactggattaccacgcaggtcgtagcggctggctgctgtatggtcgtgggctggataaacaacgtctgacccaataccagagcaaactgggtgcggcgatggtgattgttgccgcctggtgcgtggaagattatcaggtgattcgtctggcaggttcactcaccgcacgggctacacgcctggcccacgaagcgcagctggatgtcgccccgctggggaaaatcccgcacctgcgcacgccgggtttgctggtgatggatatggactccaccgccatccagattgaatgtattgatgaaattgccaaactggccggaacgggcgagatggtggcggaagtaaccgaacgggcgatgcgcggcgaactcgattttaccgccagcctgcgcagccgtgtggcgacgctgaaaggcgctgacgccaatattctgcaacaggtgcgtgaaaatctgccgctgatgccaggcttaacgcaactggtgctcaagctggaaacgctgggctggaaagtggcgattgcctccggcggctttactttctttgctgaatacctgcgcgacaagctgcgcctgaccgccgtggtagccaatgaactggagatcatggacggtaaatttaccggcaatgtgatcggcgacatcgtagacgcgcagtacaaagcgaaaactctgactcgcctcgcgcaggagtatgaaatcccgctggcgcagaccgtggcgattggcgatggagccaatgacctgccgatgatcaaagcggcagggctggggattgcctaccatgccaagccaaaagtgaatgaaaaggcggaagtcaccatccgtcacgctgacctgatgggggtattctgcatcctctcaggcagcctgaatcagaagtgataagctgaggtcgcctcagcggccggcccctgcaggcgccggcgactagtcttggactcctgttgatagatccagtaatgacctcagaactccatctggatttgttcagaacgctcggttgccgccgggcgttttttattggtgagaatccaggggtccccaataattacgatttaaatttgtgtctcaaaatctctgatgttacattgcacaagataaaaatatatcatcatgaacaataaaactgtctgcttacataaacagtaatacaaggggtgttatgagccatattcagcgtgaaacgagctgtagccgtccgcgtctgaacagcaacatggatgcggatctgtatggctataaatgggcgcgtgataacgtgggtcagagcggcgcgaccatttatcgtctgtatggcaaaccggatgcgccggaactgtttctgaaacatggcaaaggcagcgtggcgaacgatgtgaccgatgaaatggtgcgtctgaactggctgaccgaatttatgccgctgccgaccattaaacattttattcgcaccccggatgatgcgtggctgctgaccaccgcgattccgggcaaaaccgcgtttcaggtgctggaagaatatccggatagcggcgaaaacattgtggatgcgctggccgtgtttctgcgtcgtctgcatagcattccggtgtgcaactgcccgtttaacagcgatcgtgtgtttcgtctggcccaggcgcagagccgtatgaacaacggcctggtggatgcgagcgattttgatgatgaacgtaacggctggccggtggaacaggtgtggaaagaaatgcataaactgctgccgtttagcccggatagcgtggtgacccacggcgattttagcctggataacctgattttcgatgaaggcaaactgattggctgcattgatgtgggccgtgtgggcattgcggatcgttatcaggatctggccattctgtggaactgcctgggcgaatttagcccgagcctgcaaaaacgtctgtttcagaaatatggcattgataatccggatatgaacaaactgcaatttcatctgatgctggatgaatttttctaataattaattggaccgttgtccttttccgctgcataaccctgcttcggggtcattatagcgattttttcggtatatccatcctttttcgcacgatatacaggattttgccaaagggttcgtgtagactttccttggtgtatccaacggcgtcagccgggcaggataggtgaagtaggcccacccgcgagcgggtgttccttcttcactgtccct

SEQ ID NO: 41 - protein, 410 aa, Escherichia coli
MAKVSLEKDKIKFLLVEGVHQKALESLRAAGYTNIEFHKGALDDEQLKESIRDAHFIGLRSRTHLTEDVINAAEKLVAIGCFCIGTNQVDLDAAAKRGIPVFNAPFSNTRSVAELVIGELLLLLRGVPEANAKAHRGVWNKLAAGSFEARGKKLGIIGYGHIGTQLGILAESLGMYVYFYDIENKLPLGNATQVQHLSDLLNMSDVVSLHVPENPSTKNMMGAKEISLMKPGSLLINASRGTVVDIPALCDALASKHLAGAAIDVFPTEPATNSDPFTSPLCEFDNVLLTPHIGGSTQEAQENIGLEVAGKLIKYSDNGSTLSAVNFPEVSLPLHGGRRLMHIHENRPGVLTALNKIFAEQGVNIAAQYLQTSAQMGYVVIDIEADEDVAEKALQAMKAIPGTIRARLLY

SEQ ID NO: 42 - protein, 410 aa, Haemophilus influenzae
MTNKVSLDKSKIKFVLFEGVHQSALDTLHSAGYSNIDYYKKALDGDELKEAIKDAHFIGLRSRTHLTAEMIEAAPKLIAVGCFCIGTNQVDLNAAKARGIPVFNAPFSNTRSVAELVLGEILLLMRNVPQANAEVHRGVWNKSATGSYEVRGKKLGIIGYGHIGSQLSIIAESLGMDVYFYDIENKLPLGNAKQVRSLEELLSSCDVISLHVPELPSTKNLMNATRIAQLKQGAILINAARGTIVDIDALAQALKDGKIHGAAIDVFPVEPASINEEFVSPLREFDNVILTPHIGGSTAEAQENIGFEVAGKFVKYSDNGSTLSSVNFPEVSLPEHEGTKRLLHIHENRPGILNKLNQIFSEAHLNIAAQYLQTDPKIGYVVVDVETDDTSLLLTKLKEVDGTIRARVLY

SEQ ID NO: 43 - protein, 469 aa, Saccharomyces cerevisiae
MSYSAADNLQDSFQRAMNFSGSPGAVSTSPTQSFMNTLPRRVSITKQPKALKPFSTGDMNILLLENVNATAIKIFKDQGYQVEFHKSSLPEDELIEKIKDVHAIGIRSKTRLTEKILQHARNLVCIGCFCIGTNQVDLKYAASKGIAVFNSPFSNSRSVAELVIGEIISLARQLGDRSIELHTGTWNKVAARCWEVRGKTLGIIGYGHIGSQLSVLAEAMGLHVLYYDIVTIMALGTARQVSTLDELLNKSDFVTLHVPATPETEKMLSAPQFAAMKDGAYVINASRGTVVDIPSLIQAVKANKIAGAALDVYPHEPAKNGEGSFNDELNSWTSELVSLPNIILTPHIGGSTEEAQSSIGIEVATALSKYINEGNSVGSVNFPEVSLKSLDYDQENTVRVLYIHRNVPGVLKTVNDILSDHNIEKQFSDSHGEIAYLMADISSVNQSEIKDIYEKLNQTSAKVSIRLLY

SEQ ID NO: 44 - protein, 466 aa, Schizosaccharomyces pombe
MDIKGGRRGNVEDSLNKLSLSPPDNNSSFLSNHFQVRKSYSQAPARTLKPFASEDIKILLLENVNQSALSNLKDEGYQVEFLKTSMSEDDLVEKIKGVHAIGIRSKTRLTRRVLEAADSLIVIGCFCIGTNQVDLDFAAERGIAVFNSPYANSRSVAELVIGYIISLARQVGDRSLELHRGEWNKVSSGCWEIRGKTLGIIGYGHIGSQLSVLAEAMGLHVVYYDILPIMPLGSAKQLSSLPELLHRADFVSLHVPASPETKNMISSKEFAAMKEGSYLINASRGTVVDIPALVDASKSGKIAGAAIDVYPSEPAGNGKDKFVDSLNSWTSELTHCKNIILTPHIGGSTEEAQYNIGIEVSEALTRYINEGNSIGAVNFPEVSLRSLTEADRNAARVLFVHRNVPGVLRQVNELFIDHNIKSQFSDSRGDIAYLVADISDCTPGSLEALHQKLESLPCKINTRLLY

SEQ ID NO: 45 - protein, 466 aa, Neurospora crassa
MTVPREIAQPTGDKTAAQFSVSPSTFQSPISSSSFMASALAHRSAPKQLKPFNTEDVKILLLENVNQTGQDILRAQGYQVEFLKTSLPEDQLIEKIKDVHVIGIRSKTKLTANVLREAKNLLVIGCFCIGTNQVDLDYAAQHGIAVFNSPFANSRSVAELVIAEIITLARQLGDRSNEMHRGTWNKVSAKCWEIRGKTLGIVGYGHIGSQLSVLAEAMGMTVIYYDVVTLMAIGTARQVPTLEDLLAEADFVTLHVPETPETKNMISNDQFEKMKTGSYLINASRGTVVDIPALIKASRSGKIAGAALDVFPNEPAANGDYFTNDLNQWGEDLRGLNNIILTPHIGGSTEEAQRAIGVEVADALVRYINQGVTTGSVNVPEVTMRSLTLDEPNHARVIYIHRNVPGVLRKVNEILAEHNVDKQISDSKGDLAYLMADVSDVKQDDIKNIRDSLDSLSSRILTRILY

SEQ ID NO: 46 - protein, 299 aa, Entamoeba histolytica [sequence omitted]

SEQ ID NO: 47 - protein, 533 aa, Homo sapiens
MAFANLRKVLISDSLDPCCRKILQEGGLQVVEKQNLSKEELIAELQDCEGLIVRSATKVTADVINAAEKLQVVGRAGTGVDNVDLEAATRKGILVMNTPNGNSLSAAELTCGMIMCLARQIPQATASMKDGKWERKKFMGTELNGKTLGILGLGRIGREVATRMQSFGMKTIGYDPIISPEVSASFGVQQLPLEEIWPLCDFITVHTPLLPSTTGLLNDNTFAQCKKGVRVVNCARGGIVDEGALLRALQSGQCAGAALDVFTEEPPRDRALVDHENVISCPHLGASTKEAQSRCGEEIAVQFVDMVKGKSLTGVVNAQALTSAFSPHTKPWIGLAEALGTLMRAWAGSPKGTIQVITQGTSLKNAGNCLSPAVIVGLLKEASKQADVNLVNAKLLVKEAGLNVTTSHSPAAPGEQGFGECLLAVALAGAPYQAVGLVQGTTPVLQGLNGAVFRPEVPLRRDLPLLLFRTQTSDPAMLPTMIGLLAEAGVRLLSYQTSLVSDGETWHVMGISSLLPSLEAWKQHVTEAFQFHF

SEQ ID NO: 48 - protein, 533 aa, Rattus norvegicus
MAFANLRKILISDSLDPCCRKILQDGGLQVVEKQNLSKEELIAELQDCEGLIVRSATKVTADVINAAEKLQVVGRAGTGVDNVDLEAATRKGVLVMNTPNGNSLSAAELTCGMLMCLARQIPQATASMKDGKWDRKKFMGTELNGKTLGILGLGRIGREVAARMQAFGMKTVGYDPIISPEVAASFGVQQLPLEEIWPLCDFITVHTPLLPSTTGLLNDSTFAQCKKGVRVVNCARGGIVDEGALLRALQSGQCAGAALDVFTEEPPRDRALVDHENVISCPHLGASTKEAQSRCGEEIAVQFVDMVKGKSLTGVVNAQALTSAFSPHTKPWIGLAEALGTLMHAWAGSPKGTIQVVTQGTSLKNAGTCLSPAVIVGLLREASKQADVNLVNAKLLVKEAGLNVTTSHSPGVPGEQGIGECLLTVALAGAPYQAVGLVQGTTPMLQMLNGAVFRPEVPLRRGQPLLLFRAQPSDPVMLPTMIGLLAEAGVQLLSYQTSKVSDGDTWHVMGLSSLLPSLDAWKQHVSEAFQFCF

SEQ ID NO: 49 - protein, 533 aa, Mus musculus
MAFANLRKVLISDSLDPCCRKILQDGGLQVVEKQNLSKEELIAELQDCEGLIVRSATKVTADVINAAEKLQVVGRAGTGVDNVDLEAATRKGILVMNTPNGNSLSAAELTCGMIMCLARQIPQATASMKDGKWDRKKFMGTELNGKTLGILGLGRIGREVATRMQSFGMKTVGYDPIISPEVAASFGVQQLPLEEIWPLCDFITVHTPLLPSTTGLLNDSTFAQCKKGVRVVNCARGGIVDEGALLRALQSGQCAGAALDVFTEEPPRDRALVDHENVISCPHLGASTKEAQSRCGEEIAVQFVDMVKGKSLTGVVNAQALTSAFSPHTKPWIGLAEAMGTLMHAWAGSPKGTIQVVTQGTSLKNAGTCLSPAVIVGLLREASKQADVNLVNAKLLVKEAGLNVTTSHNPGVPGEQGSGECLLTVALAGAPYQAVGLVQGTTPMLQMLNGAVFRPEVPLRRGQPLLVFRAQPSDPGMLPTMIGLLAEAGVQLLSYQTSMVSDGEPWHVMGLSSLLPSLETWKQHVLEAFQFCF

SEQ ID NO: 50 - protein, 528 aa, Mycobacterium tuberculosis
MSLPVVLIADKLAPSTVAALGDQVEVRWVDGPDRDKLLAAVPEADALLVRSATTVDAEVLAAAPKLKIVARAGVGLDNVDVDAATARGVLVVNAPTSNIHSAAEHALALLLAASRQIPAADASLREHTWKRSSFSGTEIFGKTVGVVGLGRIGQLVAQRIAAFGAYVVAYDPYVSPARAAQLGIELLSLDDLLARADFISVHLPKTPETAGLIDKEALAKTKPGVIIVNAARGGLVDEAALADAITGGHVRAAGLDVFATEPCTDSPLFELAQVVVTPHLGASTAEAQDRAGTDVAESVRLALAGEFVPDAVNVGGGVVNEEVAPWLDLVRKLGVLAGVLSDELPVSLSVQVRGELAAEEVEVLRLSALRGLFSAVIEDAVTFVNAPALAAERGVTAEICKASESPNHRSVVDVRAVGADGSVVTVSGTLYGPQLSQKIVQINGRHFDLRAQGINLIIHYVDRPGALGKIGTLLGTAGVNIQAAQLSEDAEGPGATILLRLDQDVPDDVRTAIAAAVDAYKLEVVDLS

SEQ ID NO: 51 - protein, 525 aa, Bacillus subtilis
MFRVLVSDKMSNDGLQPLIESDFIEIVQKNVADAEDELHTFDALLVRSATKVTEDLFNKMTSLKIVGRAGVGVDNIDIDEATKHGVIVINAPNGNTISTAEHTFAMISSLMRHIPQANISVKSREWNRTAYVGSELYGKTLGIVGLGRIGSEIAQRARAFGMTVHVFDPFLTEERAKKIGVNSRTFEEVLESADIITVHTPLTKETKGLLNKETIAKTKKGVRLINCARGGIIDEAALLEALENGHVAGAALDVFEVEPPVDNKLVDHPLVIATPHLGASTKEAQLNVAAQVSEEVLQFAKGLPVMSAINLPAMTKDEFAKIKPYHQIAGKIGSLVSQCMKEPVQDVAIQYEGTIAKLETSFITKALLSGFLKPRVDSTVNEVNAGGVAKERGISFSEKISSSESGYDNCISVKVTGDRSTFTVTATYIPHFGERIVEINGFNIDFYPTGHLVYIQHQDTTGVIGRVGRILGDNDINIATMQVGRKEKGGEAIMMLSFDRHLEDKIVKELTNVPDIVSVKLIDLP

SEQ ID NO: 52 - protein, 523 aa, Methanobacterium sp.
MKVIIADSINEKGISDLKEVAEVTVATSITPEELVEVIKEYDAIVVRSRTKVTREVIEAGSKLKVIARAGVGVDNVDVQAATEKGIMVINAPESTSITVAEHSMGLMMSLARKISIADKSVKSGQWEKSKFMGIELNNKTLGIVGMGRIGSQVVIRAKAFNMEILVYDPYISKEAGAEMGVSVVDLETLLKESDVITIHVPLTPETRHLISTREMEIMKNTAFIINCARGGIVDEDALYYALKNDIIGGAALDVFESEPPQESPLLELDNLIATPHIGASTAEAQRDAALIVANEIITVFQGGSPRNVLNMPVMDSKNFKIMKPYLDLSEKMGSFMEQATSGNIKNMDVTYCGELSEMPQQDILTRTMLQGILNPILTEPVNLVNAPSIAQNRGIIVTEGKRCESEGYKCIIKLEIKTDKDEFSLDGTYVDEPKIIKINNYWVDVKPEGTMVIAKYQDLPGTIGAIGTKLGEHEINIATMQVGRKEVGGEAIMVLKVDQSVPQSVIDEVKKMDHVEDAVALEF

SEQ ID NO: 53 - protein, 624 aa, Arabidopsis thaliana
MAFSSSCSSVKAVNSRWTSPSPSPSSRFAVLPAFLHRRYATSVKLTAISAALKTVEQTTLTEDNRFSTVGSDSDEYNPTLPKPRILVTEKLGEAGVNLLREFGDVDCSYDLSPEDLKKKVAESDALIVRSGTKVTREVFEAAKGRLKVVGRAGVGIDNVDLQAATEHGCLVVNAPTANTVAAAEHGIALLASMARNVAQADASIKAGKWERSKYVGVSLVGKTLAVMGFGKVGTEVARRAKGLGMTVISHDPYAPADRARALGVDLVSFDQAISTADFVSLHMPLTPATKKVFNDETFSKMKKGVRLINVARGGVIDEDALVRALDAGIVAQAALDVFCEEPPSKDSRLIQHENVTVTPHLGASTKEAQEGVAIEIAEAVAGALKGELSATAVNAPMVAPEVLSELTPYIVLAEKLGRLAVQLASGGKGVQSIRVVYRSARDRDDLDTRLLRAMITKGIIEPISDSYVNLVNADFIAKQKGLRISEERMVVDSSPEYPVDSIQVQILNVESNFAGAVSDAGDISIEGKVKYGVPHLTCVGSFGVDVSLEGNLILCRQVDQPGMIGQVGNILGEQNVNVNFMSVGRTVLRKQAIMAIGVDEEPDNKTLERIGGVSAIEEFVFLKL

SEQ ID NO: 54 - protein, 530 aa, Corynebacterium glutamicum
MSQNGRPVVLIADKLAQSTVDALGDAVEVRWVDGPNRPELLDAVKEADALLVRSATTVDAEVIAAAPNLKIVGRAGVGLDNVDIPAATEAGVMVANAPTSNIHSACEHAISLLLSTARQIPAADATLREGEWKRSSFNGVEIFGKTVGIVGFGHIGQLFAQRLAAFETTIVAYDPYANPARAAQLNVELVELDELMSRSDFVTIHLPKTKETAGMFDAQLLAKSKKGQIIINAARGGLVDEQALADAIESGHIRGAGFDVYSTEPCTDSPLFKLPQVVVTPHLGASTEEAQDRAGTDVADSVLKALAGEFVADAVNVSGGRVGEEVAVWMDLARKLGLLAGKLVDAAPVSIEVEARGELSSEQVDALGLSAVRGLFSGIIEESVTFVNAPRIAEERGLDISVKTNSESVTHRSVLQVKVITGSGASATVVGALTGLERVEKITRINGRGLDLRAEGLNLFLQYTDAPGALGTVGTKLGAAGIAIEAAALTQAEKGDGAVLILRVESAVSEELEAEINAELGATSFQVDLD

SEQ ID NO: 55 - protein, 529 aa, Streptomyces sp.
MSSKPVVLIAEELSPATVDALGPDFEIRYCNGADRAELLPAIADVDAILIRSATKVDAEAIAAANRLKVVARAGVGLDNVDVPAATKAGVMVVNAPTSNIVTAAELACGLILSTARNIPQANAALKSGEWKRSKYTGVELAEKTLGVVGLGRIGALVAQRMSAFGMRIVAYDPYVQPARAAQMGVRMLSLDELLQVSDFITVHLPKTPETIGLIGEEALRKVKPSVRIINAARGGIVDEEALYSALKEGRVAGAGLDVYAKEPCTDSPLFEFDQVICTPHLGASTDEAQEKAGIAVAKSVRLALAGELVPDAVNVQGGVIAEDVKPGLPLAERLGRIFTALAGEVAVRLDVEVYGEITQHDVKVLELSALKGVFEDVVDETVSYVNAPLFAQERGVEVRLTTSSEATDHRNVVTVRGTLANGEEVSVSGTLSGPKHVQKIVAVGEYDVDLALADHMIVLRYEDRPGVVGTVGRILGEAGINIAGMQVARATAGGEALAVLTVDDTVSAAVLNELATEIGATSARSVNLV

SEQ ID NO: 56 - protein, 317 aa, Escherichia coli
MAKVSLEKDKIKFLLVEGVHQKALESLRAAGYTNIEFHKGALDDEQLKESIRDAHFIGLRSRTHLTEDVINAAEKLVAIGCFCIGTNQVDLDAAAKRGIPVFNAPFSNTRSVAELVIGELLLLLRGVPEANAKAHRGVWNKLAAGSFEARGKKLGIIGYGHIGTQLGILAESLGMYVYFYDIENKLPLGNATQVQHLSDLLNMSDVVSLHVPENPSTKNMMGAKEISLMKPGSLLINASRGTVVDIPALCDALASKHLAGAAIDVFPTEPATNSDPFTSPLCEFDNVLLTPHIGGSTQEAQENIGLEVAGKLIKYSD

SEQ ID NO: 57 - protein, 410 aa, Escherichia coli
MAKVSLEKDKIKFLLVEGVHQKALESLRAAGYTNIEFHKGALDDEQLKESIRDAHFIGLRSRTHLTEDVINAAEKLVAIGCFCIGTNQVDLDAAAKRGIPVFNAPFSNTRSVAELVIGELLLLLRGVPEANAKAHRGVWNKLAAGSFEARGKKLGIIGYGHIGTQLGILAESLGMYVYFYDIENKLPLGNATQVQHLSDLLNMSDVVSLHVPENPSTKNMMGAKEISLMKPGSLLINASRGTVVDIPALCDALASKHLAGAAIDVFPTEPATNSDPFTSPLCEFDNVLLTPHIGGSTQEAQENIGLEVAGKLIKYSDNGSTLSAVNFPEVSLPLHGGRRLMHIAEARPGVLTALNKIFAEQGVAIAAQYLQTSAQMGYVVIDIEADEDVAEKALQAMKAIPGTIRARLLY

SEQ ID NO: 58 - protein, 317 aa, Escherichia coli
MAKVSLEKDKIKFLLVEGVHQKALESLRAAGYTNIEFHKGALDDEQLKESIRDAHFIGLRSRTHLTEDVINAAEKLVAIGCFCIGTNQVDLDAAAKRGIPVFNAPFSNTRSVAELVIGELLLLLRGVPEANAKAHRGVWNKLAARSFEARGKKLGIIGYGHIGTQLGILAESLGMYVYFYDIENKLPLGNATQVQHLSDLLNMSDVVSLHVPENPSTKNMMGAKEISLMKPGSLLINASRGTVVDIPALCDALASKHLAGAAIDVFPTEPATNSDPFTSPLCEFDNVLLTPHIGGSTQEAQENIGLEVAGKLIKYSD

SEQ ID NO: 59 - protein, 337 aa, Corynebacterium glutamicum
MSQNGRPVVLIADKLAQSTVDALGDAVEVRWVDGPNRPELLDAVKEADALLVRSATTVDAEVIAAAPNLKIVGRAGVGLDNVDIPAATEAGVMVANAPTSNIHSACEHAISLLLSTARQIPAADATLREGEWKRSSFNGVEIFGKTVGIVGFGHIGQLFAQRLAAFETTIVAYDPYANPARAAQLNVELVELDELMSRSDFVTIHLPKTKETAGMFDAQLLAKSKKGQIIINAARGGLVDEQALADAIESGHIRGAGFDVYSTEPCTDSPLFKLPQVVVTPHLGASTEEAQDRAGTDVADSVLKALAGEFVADAVNVSGGRVGEEVAVWMDLARKLG

SEQ ID NO: 60 - protein, 530 aa, Corynebacterium glutamicum
MSQNGRPVVLIADKLAQSTVDALGDAVEVRWVDGPNRPELLDAVKEADALLVRSATTVDAEVIAAAPNLKIVGRAGVGLDNVDIPAATEAGVMVANAPTSNIHSACEHAISLLLSTARQIPAADATLREGEWKRSSFNGVEIFGKTVGIVGFGHIGQLFAQRLAAFETTIVAYDPYANPARAAQLNVELVELDELMSRSDFVTIHLPKTKETAGMFDAQLLAKSKKGQIIINAARGGLVDEQALADAIESGHIRGAGFDVYSTEPCTDSPLFKLPQVVVTPHLGGSTEEAQDRAGTDVADSVLKALAGEFVADAVNVSGGRVGEEVAVWMDLARKLGLLAGKLVDAAPVSIEVEARGELSSEQVDALGLSAVRGLFSGIIEESVTFVNAPRIAEERGLDISVKTNSESVTHRSVLQVKVITGSGASATVVGALTGLERVEKITRINGRGLDLRAEGLNLFLQATDAPGALGTVGTKLGAAGINIEAAALTQAEKGDGAVLILRVESAVSEELEAEINAELGATSFQVDLD

SEQ ID NO: 61 - protein, 530 aa, Corynebacterium glutamicum
MSQNGRPVVLIADKLAQSTVDALGDAVEVRWVDGPNRPELLDAVKEADALLVRSATTVDAEVIAAAPNLKIVGRAGVGLDNVDIPAATEAGVMVANAPTSNIHSACEHAISLLLSTARQIPAADATLREGEWKRSSFNGVEIFGKTVGIVGFGHIGQLFAQRLAAFETTIVAYDPYANPARAAQLNVELVELDELMSRSDFVTIHLPKTKETAGMFDAQLLAKSKKGQIIINAARGGLVDEQALADAIESGHIRGAGFDVYSTEPCTDSPLFKLPQVVVTPHLGASTEEAQDRAGTDVADSVLKALAGEFVADAVNVSGGRVGEEVAVWMDLARKLGLLAGKLVDAAPVSIEVEARGELSSEQVDALGLSAVRGLFSGIIEESVTFVNAPRIAEERGLDISVKTNSESVTHRSVLQVKVITGSGASATVVGALTGLERVEKITRINGRGLDLRAEGLNLFLQYTDAPGALGTVGTKLGAAGINIEAAALTQAEKGDGAVLILRVESAVSEELEAEINAELGATSFQVDLD

SEQ ID NO: 62 - protein, 528 aa, Mycobacterium tuberculosis
MSLPVVLIADKLAPSTVAALGDQVEVRWVDGPDRDKLLAAVPEADALLVRSATTVDAEVLAAAPKLKIVARAGVGLDNVDVDAATARGVLVVNAPTSNIHSAAEHALALLLAASRQIPAADASLREHTWKRSSFSGTEIFGKTVGVVGLGRIGQLVAQRIAAFGAYVVAYDPYVSPARAAQLGIELLSLDDLLARADFISVHLPKTPETAGLIDKEALAKTKPGVIIVNAARGGLVDEAALADAITGGHVRAAGLDVFATEPCTDSPLFELAQVVVTPHLGASTAEAQDRAGTDVAESVRLALAGEFVPDAVNVGGGVVNEEVAPWLDLVRKLGVLAGVLSDELPVSLSVQVRGELAAEEVEVLRLSALRGLFSAVIEDAVTFVNAPALAAERGVTAEICKASESPNHRSVVDVRAVGADGSVVTVSGTLYGPQLSQKIVQINGRHFDLRAQGINLIIHYVDRPGALGKIGTLLGTAGVAIQAAQLSEDAEGPGATILLRLDQDVPDDVRTAIAAAVDAYKLEVVDLS

SEQ ID NO: 63 - protein, 1011 aa, synthetic construct
ATGGCGTTCGCAAACCTTCGAAAGATTTTAATAAGCGATTCACTGGATCCATGCTGTCGAAAGATACTGCAAGATGGCGGGTTACAGGTAGTAGAGAAGCAAAACCTGTCGAAAGAGGAGTTAATTGCCGAGTTGCAAGACTGCGAGGGTCTCATTGTGCGTTCCGCAACAAAGGTGACCGCAGACGTCATCAATGCGGCGGAGAAGTTACAAGTTGTCGGACGCGCCGGAACCGGCGTGGATAATGTGGACCTCGAGGCGGCAACTAGAAAGGGCGTTCTGGTAATGAACACACCCAATGGAAACTCCCTGTCAGCAGCGGAGCTGACCTGCGGCATGTTGATGTGCCTTGCGCGCCAAATACCACAAGCCACGGCATCAATGAAGGACGGCAAGTGGGACCGCAAGAAGTTTATGGGGACAGAACTGAATGGTAAGACACTTGGTATTCTGGGTTTAGGTCGGATAGGCCGCGAAGTCGCGGCACGGATGCAGGCTTTCGGGATGAAAACAGTGGGTTATGACCCGATAATCAGCCCCGAGGTCGCAGCCTCATTTGGGGTCCAACAATTGCCGTTGGAAGAAATTTGGCCCCTGTGTGACTTCATAACCGTGCATACGCCGCTGCTGCCTTCTACCACAGGTCTCCTCAATGACTCTACTTTTGCCCAATGTAAGAAGGGTGTCCGGGTGGTCAACTGTGCACGCGGCGGAATAGTTGACGAGGGTGCGCTGCTGCGGGCGCTTCAAAGTGGCCAGTGTGCTGGTGCGGCCTTGGATGTATTCACAGAAGAACCCCCGCGCGACCGCGCACTTGTGGATCACGAGAACGTAATTAGCTGCCCTCACTTAGGAGCATCTACAAAGGAAGCCCAATCGCGTTGTGGGGAAGAAATTGCCGTCCAATTCGTTGACATGGTGAAGGGTAAATCATTAACGGGAGTAGTTAATGCACAGGCCCTTACGAGTGCCTTCTCTCCACATACCAAGCCTTGGATTGGATTAGCTGAA

SEQ ID NO: 64 - protein, 334 aa, Clostridium acetobutylicum
MAKIAINGFGRIGRLALRRILEVPGLEVVAINDLTDAKMLAHLFKYDSSQGRFNGEIEVKEGAFVVNGKEVKVFAEADPEKLPWGDLGIDVVLECTGFFTKKEKAEAHVRAGAKKVVISAPAGNDLKTIVFNVNNEDLDGTETVISGASCTTNCLAPMAKVLNDKFGIEKGFMTTIHAFTNDQNTLDGPHRKGDLRRARAAAVSIIPNSTGAAKAISQVIPDLAGKLDGNAQRVPVPTGSITELVSVLKKKVTVEEINAAMKEAADESFGYTEDPIVSADVVGINYGSLFDATLTKIVDVNGSQLVKTAAWYDNEMSYTSQLVRTLAYFAKIAK

SEQ ID NO: 65 - protein, 340 aa, Bacillus subtilis
MKVKVAINGFGRIGRMVFRKAMLDDQIQVVAINASYSAETLAHLIKYDTIHGRYDKEVVAGEDSLIVNGKKVLLLNSRDPKQLPWREYDIDIVVEATGKFNAKDKAMGHIEAGAKKVILTAPGKNEDVTIVMGVNEDQFDAERHVIISNASCTTNCLAPVVKVLDEEFGIESGLMTTVHAYTNDQKNIDNPHKDLRRARACGESIIPTTTGAAKALSLVLPHLKGKLHGLALRVPVPNVSLVDLVVDLKTDVTAEEVNEAFKRAAKTSMYGVLDYSDEPLVSTDYNTNPHSAVIDGLTTMVMEDRKVKVLAWYDNEWGYSCRVVDLIRHVAARMKHPSAV

SEQ ID NO: 66 - protein, 463 aa, Corynebacterium glutamicum
MVPLIGRLHRNNNVVVSVFGRLLVNVSDIDIIKSHRYARHIISKELPLESSLDILRELVDMNLGTASIDLGQLAYSFEESERTDLRAFLEDALAPVIGAETDINPTDIVLYGFGRIGRLLARILVSREALYDGARLRAIVVRKNGEEDLVKRASLLRRDSVHGGFDGTITTDYDNNIIWANGTPIKVIYSNDPATIDYTEYGINDAVVVDNTGRWRDREGLSQHLKSKGVAKVVLTAPGKGDLKNIVYGINHTDITADDQIVSAASCTTNAITPVLKVINDRYGVEFGHVETVHSFTNDQNLIDNFHKGSRRGRAAGLNMVLTETGAAKAVSKALPELEGKLTGNAIRVPTPDVSMAVLNLTLKTEVDRDEVNEFLRRVSLHSDLRQQIDWIRSPEVVSTDFVGTTHAGIVDGLATIATGRHLVLYVWYDNEFGYSNQVIRIVEEIAGVRPRVYPERKQPAVL

SEQ ID NO: 67 - protein, 396 aa, Arabidopsis thaliana
MASVTFSVPKGFTEFSGLRSSSASLPFGKKLSSDEFVSIVSFQTSAMGSSGGYRKGVTEAKLKVAINGFGRIGRNFLRCWHGRKDSPLDIIAINDTGGVKQASHLLKYDSTLGIFDADVKPSGETAISVDGKIIQVVSNRNPSLLPWKELGIDIVIEGTGVFVDREGAGKHIEAGAKKVIITAPGKGDIPTYVVGVNADAYSHDEPIISNASCTTNCLAPFVKVLDQKFGIIKGTMTTTHSYTGDQRLLDASHRDLRRARAAALNIVPTSTGAAKAVALVLPNLKGKLNGIALRVPTPNVSVVDLVVQVSKKTFAEEVNAAFRDSAEKELKGILDVCDEPLVSVDFRCSDFSTTIDSSLTMVMGDDMVKVIAWYDNEWGYSQRVVDLADIVANNWK

SEQ ID NO: 68 - protein, 374 aa, Chlamydomonas reinhardtii
MAAMMQKSAFTGSAVSSKSGVRAKAARAVVDVRAEKKIRVAINGFGRIGRNFLRCWHGRQNTLLDVVAINDSGGVKQASHLLKYDSTLGTFAADVKIVDDSHISVDGKQIKIVSSRDPLQLPWKEMNIDLVIEGTGVFIDKVGAGKHIQAGASKVLITAPAKDKDIPTFVVGVNEGDYKHEYPIISNASCTTNCLAPFVKVLEQKFGIVKGTMTTTHSYTGDQRLLDASHRDLRRARAAALNIVPTTTGAAKAVSLVLPSLKGKLNGIALRVPTPTVSVVDLVVQVEKKTFAEEVNAAFREAANGPMKGVLHVEDAPLVSIDFKCTDQSTSIDASLTMVMGDDMVKVVAWYDNEWGYSQRVVDLAEVTAKKWVA

SEQ ID NO: 69 - protein, 335 aa, Paracoccus yeei
MTVKVAINGFGRIGRLALRSIVELRREDVEVVAINDLGPVATLAHLLRYDSVHGPFRGSIDLGEDWIDVGSGKIRVSSERDPVNLPHDELGVDVALECTGFFTSREKAESHIRAGAKRVLVSAPSDGADKTIVFKVNHDTLTADDVVVSNGSCTTNVLAPIAKVLNDLCGIERGYMTTVHAYTGDQPTQDTVHKDLYRARAAALSMIPTSTGAANAIGRVLPELKGKLHGSSIRVPTPNVSVIDLAVSTSREVSIDEVNDAIRQTAAGAMSGVLAFTTEPLVSVDLNHRTESSIVALPQTDVVDGRMVRVLAWYDNEWSFATRMADTAVAMAKLI

SEQ ID NO: 70 - protein, 333 aa, Celeribacter marinus
MTIKLGINGFGRIGRCTLAHIAEAGLNEVEVVKINATGPIETNAHLLKYDSVHGRFGGPVAVNGNTMDLGRGPIQVMSTYEPDELDWEGVDVVLECTGKFNDGHRADVHMRRGAKKVLISAPAKNVDRTVVFGVNHRDLRDDERMVSNGSCTTNCLAPLAKVLNDAVGIESGIMTTIHSYTGDQPTLDRRHPDLYRARAAALAMIPTSTGAAKALGEVLPELSGKLDGTSMRVPTPNVSAVDLTFQAGKDVSVADINEIVREAAMGHMGMVLGYDPEPKVSIDFNHTTESCIFAPEQTKVIGRTVRVLAWYDNEWGFSARMADVAAAMGRLSH

SEQ ID NO: 71 - protein, 335 aa, Bradyrhizobiaceae bacterium
MAVRVAINGFGRIGRNVLRAIYESKRTDIEVVAINDLGPVETNAHLLRFDSVHGRFPGEVTVEGDSIDIGNGKIKVTAVRDPATLPWKDLGIDIALECTGIFSAKAKASAHLTAGAKRVLVSAPSDGADATIVYGVNHDKLTKDHLVVSNGSCTTNCLAPIAKVLNDTVGIETGFMTTIHAYTGDQPTLDTMHSDLYRGRAAALSMIPTSTGAAKAIGLVLPELQGKLDGVAIRVPTPNVSVVDLKIVAKKTTTKEEINDAMKRAASQELKGILGTTSHPNVSIDFNHDAHSSTFAFDQTKVQGGTLVRVLSWYDNEWGFSNRMADTAVAMSKLI

SEQ ID NO: 72 - protein, 512 aa, Pseudomonas furukawaii
MSGLLLIAGDCVRRHNVAPFFIPYMWKVLPVTQKPDQCLGEWIDREALAEAMIPMIGQLYRNNNVVTSIYGRGLINRSVIAILKAHRFARHRLVDEAELSVHETFPILKAMSELKLGAASVDLGKMVAKFKAEGNGRSVEQFTRDELADVVGKQNGAAREGTDVVLYGFGRIGRLLARILIEKTGGGDGLRLRAIVVRKGAENDLVKRASLLRRDSVHGPFDGTIVIDEANNTLIANGNLIQVIYSNDPSSIDYTAYGIKNALLVDNTGKWRDAEGLSQHLKCPGIDRVVLTAPGKGALKNIVHGINHGDISADDKIISAASCTTNAIVPVLKAVNDQYGIVNGHVETVHSYTNDQNLIDNFHKGSRRGRSAPLNMVITETGAATAAAKALPVLKGRLTGNAIRVPTPNVSMAILNLNLEKATSREEINEYLRQMAMHSDLHKQIDYVSSQEVVSTDFVGSRHAGVVDAEATICNDNRVVLYVWYDNEFGYSCQVVRVMEDMAGVNPPAFPH

SEQ ID NO: 73 - protein, 444 aa, Bigelowiel lanatans
MALVGAICFSLSGASNVAAPAMRTAPRVASMSRTMPMSMAGQRVSVRPKMIQRREMKAEALSYTVDDIRGMLGDDVANQILAKNTPTGPERNVVLYGFGRIGRLLARIITTIPTNLKLKGIVVRQPKKPDLEKRLELIKRDSVHGPFRGTISMDEADNALIMNGQKVRLIYANQPEEVDYTKYGINDAIVIDNTGVWRDDEGLAKHLSSKGAAQVILTAPGKGVKNIVAGVNSDVIEGSDKILSAASCTTNAVVPALSVLHKKFGIVSGHIETVHSFTNDQNLIDNYHKADRRGRAGPLNMVISETGAGKAVAVALPELAGKLTASAIRVPTPDVSIAVMILDLEKSTTAEEINAAFKSEATGTLDDNLGYSDSKEAVSLDFIGSTHAGEVDALATKCTGNSCIVYVWYDNENGYSNQVVRVVEQWAAKQEAAGLKFEAAEAMA

SEQ ID NO: 74 - protein, 521 aa, Pseudomonas chlororaphis
MIFPDGVWLRSARQARIATQGTRLHNVAPFFSPYMWKVPVTQKPDQCLGEWIDREALAEAMIPLIGQLYRNNNVVSSIYGRSLINQSVIAILKAHRFARHRSSDDSELSVHETFPLLKAMSELKLGAASVDLGKLAFKFRNEGNGRTAEQFVREELADVVGQQNASPRKGTDVVLYGFGRIGRLLARILIEKTGGGDGLRLRAIVVRKGAENDLTKRASLLRRDSVHGSFNGTITIDEANNTITANGNLIQVIYAKNPTEVDYTQYGIKDALLVDNTGVWRDADGLGQHLACPGIDRVVLTAPGKGKLKNIVHGINHADITADDKIVSAASCTTNAIVPVLKAVNDKFGIVNGHVETVHSYTNDQNLIDNFHKGDRRGRSAALNMVITETGAATAAAKALPELAGKLTGNAIRVPTPNVSMAILNLNLEKAATREEMNEYLRYMALHSDLHKQIDFVNSQEVVSTDFVGSRHAGVVDAEATITQDNRVVLYVWYDNEFGYSCQVVRVMEDMAGVNPPAFPR

SEQ ID NO: 75 - protein, 340 aa, Saccharolobus solfataricus
MINVAVNGYGTIGKRVADAIIKQPDMKLVGVAKTSPNYEAFIAHRRGIRIYVPQQSIKKFEESGIPVAGTVEDLIKTSDIVVDTTPNGVGAQYKPIYLQLQRNAIFQGGEKAEVADISFSALCNYNEALGKKYIRVVSCNTTALLRTICTVNKVSKVEKVRATIVRRAADQKEVKKGPINSLVPDPATVPSHHAKDVNSVIRNLDIATMAVIAPTTLMHMHFINITLKDKVEKKDILSVLENTPRIVLISSKYDAEATAELVEVARDLKRDRNDIPEVMIFSDSIYVKDDEVMLMYAVHQESIVVPENIDAIRASMKLMSAEDSMRITNESLGILKGYLI

SEQ ID NO: 76 - protein, 158 aa, Pseudomonas viridiflava
ARKVIISAPASGADATIVYGVNHDTLRQSHQIISSASCTTNCLAPVAQVLHRELGIESGLMTTIHAYTNDQNLIDVYHTDPYRARSATQSMIPSKTGAAEAVGLVLPELAGKLTGMAVRVPVINVSLVDLTVTLKRETTAEEVNALMKEATQHSKVVG

SEQ ID NO: 77 - protein, 356 aa, Kluyveromyces lactis
MPDMTNESSSKPAQINIGINGFGRIGRLVLRAALTHPEVKVRLINNPSTTPEYAAYLFKYDSTHGKYRGEVEFDDERIIIQNDHVSAHIPLSHFREPERIPWASYNVDYVIDSTGVFKEVDTASRHKGVKKVIITAPSKTAPMYVYGVNHVKYNPLTDHVVSNASCTTNCLAPLVKALDDEFGIEEALMTTIHATTASQKTVDGTSSGGKDWRGGRSCQGNIIPSSTGAAKAVGKILPELNGKITGMSIRVPTINISLVDLTFRTAKKTSYDDIMKALEQRSRSDMKGVLGVTKDAVVSSDFTSDSRSSIVDAKAGIELNDHFFKVLSWYDNEYGYSSRVVDLSIFMAQKDFEAGV

SEQ ID NO: 78 - protein, 68 aa, Geobacillus stearothermophilus
MALRVPTPNVSLVDLVVDVKRDVTVEEVNEALLRAANGPLKGILDFTMEPLVSIDFNTNPHEPAFGDH

SEQ ID NO: 79 - protein, 234 aa, Streptococcus pyogenes
LAISPFNYPVNLAGSKIAPALIAGNVVALKPPTQGSISGLLLAEAFAEAGIPAGVFNTITGRGSVIGDYIVEHEAVNFINFTGSTPIGEGIGKLAGMRPIMLELGGKDSAIVLEDADLVLAAKNIVAGAFGYSGQRCTAVKRVLVMDKVADQLAAEIKTLVEKLSVGMPEDDADITPLIDTSAADFVEGLIKDATDKGATALTAFNREGNLISPVLFDHVTTDMRLAWEEPFGP

SEQ ID NO: 80 - protein, 501 aa, Thermoproteus tenax
MRAGLLEGVIKEKGGVPVYPSYLAGEWGGSGQEIEVKSPIDLATIAKVISPSREEVERTLDVLFKRGRWSARDMPGTERLAVLRKAADIIERNLDVFAEVLVMNAGKPKSAAVGEVKAAVDRLRLAELDLKKIGGDYIPGDWTYDTLETEGLVRREPLGVVAAITPFNYPLFDAVNKITYSFIYGNAVVVKPSISDPLPAAMAVKALLDAGFPPDAIALLNLPGKEAEKIVADDRVAAVSFTGSTEVGERVVKVGGVKQYVMELGGGDPAIVLEDADLDLAADKIARGIYSYAGQRCDAIKLVLAERPVYGKLVEEVAKRLSSLRVGDPRDPTVDVGPLISPSAVDEMMAAIEDAVEKGGRVLAGGRRLGPTYVQPTLVEAPADRVKDMVLYKREVFAPVALAVEVKDLDQAIELANGRPYGLDAAVFGRDVVKIRRAVRLLEVGAIYINDMPRHGIGYYPFGGRKKSGVFREGIGYAVEAVTAYKTIVFNYKGKGVWKYE

SEQ ID NO: 81 - protein, 475 aa, Streptococcus mutans
MTKQYKNYVNGEWKLSENEIKIYEPASGAELGSVPAMSTEEVDYVYASAKKAQPAWRSLSYIERAAYLHKVADILMRDKEKIGAVLSKEVAKGYKSAVSEVVRTAEIINYAAEEGLRMEGEVLEGGSFEAASKKKIAVVRREPVGLVLAISPFNYPVNLAGSKIAPALIAGNVIAFKPPTQGSISGLLLAEAFAEAGLPAGVFNTITGRGSEIGDYIVEHQAVNFINFTGSTGIGERIGKMAGMRPIMLELGGKDSAIVLEDADLELTAKNIIAGAFGYSGQRCTAVKRVLVMESVADELVEKIREKVLALTIGNPEDDADITPLIDTKSADYVEGLINDANDKGAAALTEIKREGNLICPILFDKVTTDMRLAWEEPFGPVLPIIRVTSVEEAIEISNKSEYGLQASIFTNDFPRAFGIAEQLEVGTVHINNKTQRGTDNFPFLGAKKSGAGIQGVKYSIEAMTTVKSVVFDIK

SEQ ID NO: 82 - protein, 481 aa, Alkalihalobacillus halodurans
MALQTEQFNANILRNGEWVESRTGERISISAPASGVALGSIPALSQEEVNDAIQGAKDAQKIWKIRPIHERVDLLYAWADLLEERKEIIGELIMHEVAKPKKSAIGEVSRTADIIRHTADEALRLNGETLKGDQFKGGSSKKIALVEREPLGVVLAISPFNYPVNLAAAKIAPALVTGNTVVFKPATQGSLSGIKMVEALADAGAPEGIIQVVTGRGSVIGDHLVEHPGIDMITFTGGTTTGERISEKAKMIPVVLELGGKDPAIVLDDADLKLTASQIVSGAFSYSGQRCTAIKRVFVQDSVADQLVANIKELVEQLTVGSPEDDADITPVIDEKSAAFIQGLIDDALENGATLLSGNKRQGNLLSPTLLDDVTPAMRVAWEEPFGPVLPIIRVKDANEAISLSNQSDYGLQASIFTKDTDRAINIGKHLEVGTVHINAKTERGPDHFPFLGVKKSGLGVQGIKPSLLSMTRERVTVLNL

SEQ ID NO: 83 - protein, 470 aa, Saccharolobus solfataricus
MMSQEVIEVRSPSNLNVIGTVKRMHKDEVRGEIEEAYKGFEIISKMPLYKRTAILRKVSEILEREQERLAKLLAMEAGKPIRDSRVEVLRASRLFRHAAEEVGMVLEGKNYRVDAYEYPPGNENRIVVSTREPIGVVTAILPFNFPINSFAHKVAPALAVGNSVVVKPSINTPLAAIEMKKILVEAGLPDSAVRVVTGYSSEIGDEIITHPLVGLITLTGSTQTGLKIASKAVSLGKRIIMELGGSDPIIILEDANIERASSIAVRARFEYAGQNCNAGKRIIVREEIYDKFVKAFNDKARALKVGDPLDETTDVGPVINKESVENLNSVLADAKAKGGKVEILNKGPESGSFFPLTMVTNPSLDMLVLKSEVFGPIVPIVSVKSDEEAIRIANSTEYGLQSAIFTNDVNRALKLSRELKFGAVIINDSTRLRWDSLAFGGFKKSSIGREGVRETMLEMTENKLIAITLL

SEQ ID NO: 84 - protein, 234 aa, Clostridium acetobutylicum
LAISPFNYPVNLSGSKVAPALIAGNSVVLKPSTTGAISALHLAEIFNAAGLPAGVLNTVTGKGSEIGDYLITHEEVNFINFTGSSAVGKHISKIAGMIPMVLELGGKDAAIVLEDANLETTAKSIVSGAYGYSGQRCTAVKRVLVMDKVADELVELVTKKVKELKVGNPFDDVTITPLIDNKAADYVQTLIDDAIEKGATLIVGNKRKENLMYPTLFDNVTADMRIAWEEPFGP

SEQ ID NO: 85 - protein, 234 aa, Bacillus cereus
LAIAPFNYPVNLFAAKLAPALIMGNAVIFKPATQGAISGIKMVEALHKAGLPKGLVNVATGRGSVIGDYLVEHEGINMVSFTGGTNTGKHLAKKASMIPLVLELGGKDPGIVREDADLQDAANHIVSGAFSYSGQRCTAIKRVLVHENVADELVGLLKEQVAKLSVGSPEQDSTIVPLIDDKSADFVQGLVDDAVEKGATIVIGNKRERNLIYPTLIDHVTTDMRLAWEEPFAP

SEQ ID NO: 86 - protein, 509 aa, Saccharolobus solfataricus
MEKTSVLIKSKELMEIYELKDGVPYFKTYLSGQWISGDEWQDVISPIDLNIIGKIPKLNWNQIDDTLEHIYRKGRWSIRDTPGEKRLDIYKKMASLLDKFKEDFVNVLMINNGKTKSAAEGEVKAAIERLLRADLDVKETRGDYVPGDWSSETLETEAVVRKEPVGVVLSIVPFNYPLFDTVNKIVYTTVIGNAIIIKPPSSTPLPILMLAKVMELASFPKDSFAIITIPGRDMNKVVGDKRIQAISLTGSTETGEEVVRNAGIKQFIMELGGGDPAIVLSDADLAWAAQRIAAGIISYTGQRCDSVKLVLVEEEVYDTLKDLLIKELTKSVKVGDPRDPLTTVGPVIDVKTVDEWEKAIKDAVEKGGKILFGGKRLGPTYIEPVLIEAPKETLKDMYFYNKEVFASAALLIKVKNIDEALEISNSRKYGLDAAIFGKDINKIRKLQRFLEVGAIYINDYPRHGIGYFPFGGRKDSGIGREGIGYTIQYVTAYKSIVYNYKGKGIWEYL

SEQ ID NO: 87 - protein, 506 aa, Thermococcus sibiricus
MDKLVHNKIFDGIYRPGEDGIPEFKAYVAGQWVFGESFSEVKSPIDGRIIARVSRLSRDQVEEALARVYEKGREEIRNYPGEKRVQSFLKAAGLMREAFEDFVNVLILDAGKPKSNAVGETKATIERLEKTTFESRRMLGDYVPGDWSEETLESEGIVKREPYGLILAISPFNYPLFISAAKVVPALLSGNTVLLKPASADPLAAIMFVRVLELAGFPKESFALLTIPGSFMDDVVKDRRIRAITFTGSTEVGEHIIRTGGIKAYHLELGGKDPAIVLDDANLELASEKIVKGMVSFSGQRCDAIRLILAQEKIYEDLKARILEKLKGMEPRNPLEDENAVMGPLIDESSAEYIEEVYKDAVEKGARPLTEFRRKGNYVWPILLEVSKEKIKDLRAFNEDVFGSMALLIKVKDEDEAIEIAKSSRFGLDASVFSECERRARKVARKLEVGSVFINEYPRHGIGYYPFGGMKDSGVGREGIGYSVEQFTTTKTIVHNFKGYGVWEYL

SEQ ID NO: 88 - protein, 491 aa, Escherichia coli
MAVTQTAQACDLVIFGAKGDLARRKLLPSLYQLEKAGQLNPDTRIIGVGRADWDKAAYTKVVREALETFMKETIDEGLWDTLSARLDFCNLDVNDTAAFSRLGAMLDQKNRITINYFAMPPSTFGAICKGLGEAKLNAKPARVVMEKPLGTSLATSQEINDQVGEYFEECQVYRIDHYLGKETVLNLLALRFANSLFVNNWDNRTIDHVEITVAEEVGIEGRWGYFDKAGQMRDMIQNHLLQILCMIAMSPPSDLSADSIRDEKVKVLKSLRRIDRSNVREKTVRGQYTAGFAQGKKVPGYLEEEGANKSSNTETFVAIRVDIDNWRWAGVPFYLRTGKRLPTKCSEVVVYFKTPELNLFKESWQDLPQNKLTIRLQPDEGVDIQVLNKVPGLDHKHNLQITKLDLSYSETFNQTHLADAYERLLLETMRGIQALFVRRDEVEEAWKWVDSITEAWAMDNDAPKPYQAGTWGPVASVAMITRDGRSWNEFE

SEQ ID NO: 89 - protein, 468 aa, Escherichia coli
MSKQQIGVVGMAVMGRNLALNIESRGYTVSIFNRSREKTEEVIAENPGKKLVPYYTVKEFVESLETPRRILLMVKAGAGTDAAIDSLKPYLDKGDIIIDGGNTFFQDTIRRNRELSAEGFNFIGTGVSGGEEGALKGPSIMPGGQKEAYELVAPILTKIAAVAEDGEPCVTYIGADGAGHYVKMVHNGIEYGDMQLIAEAYSLLKGGLNLTNEELAQTFTEWNNGELSSYLIDITKDIFTKKDEDGNYLVDVILDEAANKGTGKWTSQSALDLGEPLSLITESVFARYISSLKDQRVAASKVLSGPQAQPAGDKAEFIEKVRRALYLGKIVSYAQGFSQLRAASEEYNWDLNYGEIAKIFRAGCIIRAQFLQKITDAYAENPQIANLLLAPYFKQIADDYQQALRDVVAYAVQNGIPVPTFSAAVAYYDSYRAAVLPANLIQAQRDYFGAHTYKRIDKEGVFHTEWLD

SEQ ID NO: 90 - protein, 464 aa, Lactobacillus brevis
MKIISIKFVLGGNIMKVTVVGCTHAGTFAIKQILAEHPDAEVTVYERNDVISFLSCGIALYLGGKVADPQGLFYSSPEELQKLGANVQMNHNVLAIDPDQKTVTVEDLTSHAQTTESYDKLVMTSGSWPIVPKIPGIDSDRVKLCKNWAHAQALIEDAKEAKRITVIGAGYIGAELAEAYSTTGHDVTLIDAMDRVMPKYFDADFTDVIEQDYRDHGVQLALSETVESFTDSATGLTIKTDKNSYETDLAILCIGFRPNTDLLKGKVDMAPNGAIITDDYMRSSNPDIFAAGDSAAVHYNPTHQNAYIPLATNAVRQGILVGKNLVKPTVKYMGTQSSSGLALYDRTIVSTGLTLAAAKQQGVNAEQVIVEDNYRPEFMPSTEPVLMSLVFDPDTHRILGGALMSKYDVSQSANTLSVCIQNENTIDDLAMVDMLFQPNFDRPFNYLNILAQAAQAKVAQSVNA

SEQ ID NO: 91 - protein, 450 aa, Levilactobacillus brevis
MKVTVVGCTHAGTFAIKQILAEHPDAEVTVYERNDVISFLSCGIALYLGGKVADPQGLFYSSPEELQKLGANVQMNHNVLAIDPDQKTVTVEDLTSHAQTTESYDKLVMTSGSWPIVPKIPGIDSDRVKLCKNWAHAQALIEDAKEAKRITVIGAGYIGAELAEAYSTTGHDVTLIDAMDRVMPKYFDADFTDVIEQDYRDHGVQLALSETVESFTDSATGLTIKTDKNSYETDLAILCIGFRPNTDLLKGKVDMAPNGAIITDDYMRSSNPDIFAAGDSAAVHYNPTHQNAYIPLATNAVRQGILVGKNLVKPTVKYMGTQSSSGLALYDRTIVSTGLTLAAAKQQGVNAEQVIVEDNYRPEFMPSTEPVLMSLVFDPDTHRILGGALMSKYDVSQSANTLSVCIQNENTIDDLAMVDMLFQPNFDRPFNYLNILAQAAQAKVAQSVNA

SEQ ID NO: 92 - protein, 449 aa, Secundilactobacillus silagincola
MKVAVIGCTHAGTFATKQILAENPDAEVTVYEKNDVISFLSCGIALYLGGQVKDPQGLFYSNPDELSKLGATVLMRHNVTAIDNQAHTITVEDLATHEVTTSSYDKLVMTSGSWPIIPPIPGIDSDKVLLCKNWAHAQTLFQKAENAKRIAVIGAGYIGAELAEAYSLKGHDVTLIDAQDRVMPKYFDSAFTDKIEDEYRAHNVQLALSQKVQGFETTADGVTITTDKEAIDVDLAVLCIGFRPNTDLLAGKVDMAKNGAILTNDYMQTSDPDIFAAGDSAAVHYNPTGKNAYIPLATNAVRQGILVGKNIVKPTVKYMGTQSSSGLALYGTSLCSTGLTYEAAKAQGINAEQVIITDNYRPEFMPTTLPVTMSLVFNPDTREILGGALMSKYDISQSANLLSVCIQNHNTIDDLAMVDMLFQPNFDRPFNYLNILGQAAQEKLTTVKA

SEQ ID NO: 93 - protein, 450 aa, Secundilactobacillus folii
MKVAVIGCTHAGTFATKQILAENPDAEVTVYERNDVISFLSCGIALYLGGEVKDPQGLFYSSPDELSGLGAKVLMRHDVKSIDNQAHTITVEDLDSHETTTTSYDKLVMTTGSWPVIPSIPGIKSDRVLLCKNWAHAQALFNRAKDSKRIAVIGAGYIGAELAEAYSLKNHDVTLIDAQDRVMPKYFDAAFTDKVEDEYTKHGVALALSQKVQSFETTDDAVTIHTDKESVTVDLAILCIGFKPNTILLEGKVDMAANGAILTNDYMQSSDPDIFAAGDSAAVHYNPTGKNAYIPLATNAVRQGILVGKNLVKPTVKYMGTQSTSGLSLYGISLCSTGLTYEAAQEQGINAQQVIITDNYRPEFMPTTLPVTMSLVFNPETREILGGALMSKYDISQSANLLSVCIQNHNTIDDLAMVDMLFQPNFDRPFNYLNILGQAAQQKLAEAVKA

SEQ ID NO: 94 - protein, 451 aa, Lactobacillus kimchicus
MKVVIIGCTHAGTFATKQILTEHPDAEVTVYERNDVISFLSCGIALYLGGQVKDPQGLFYSNPQELAELGATIKMRHDVKSVDNVAHTVVVEDLNTHETTTVLYDKLVMTTGSWPVIPPIPGIDSDRVKLCKNWVHAQTLFKEAPTAKRIAVIGAGYIGAELAEAYSLKGHEVTLIDGEDRVMPKYFDQTFTTKIEANYQNHGVRLALNQRVQSFETTTDAVTIHTDKDAITADLAILCIGFRPNTELVKGKVDMAQNGAILTNDYMQSSDPDIFAAGDAAAVHYNPTGKNAYIPLATNAVRQGILVGKNIAQPTVKYMGTQSSSGLALYGVSICSTGLTYEAAKAQGLAAEQVIVEDNYRPEFMPTTTPVLMSLVFDPNTRQILGGALMSDYDISQSANLLSVCIQNQNTIDDLAMVDMLFQPNFDRPFNYLNILAQAAQEKVAKATAEA

SEQ ID NO: 95 - protein, 445 aa, Lentilactobacillus curieae
MKIAVIGCTHAGTFAIKTVLAEHPDAEVTVYEKNDNISFLSCGIALYLGGEVKDPQGLFYSSPEELSKLGATVKMQHSVESVDPDKKELTVKNLEDNTEFTDTYDKLVVTSGSWPVIPPIPGVDNKNVYLCKNYGHAKALFEKAKDAKRIIVIGAGYIGAELAEAYSKSGHDVTLLDGADRVMPKYFDSEFTDVIEQDFRDHGVTLGLGEKVQEISGDDVATVKTDKNSYEADLVVLCVGFRPNNDLVKGKLDMTDNGALITNDYMQTSNPDIYAAGDSVAVHYNPTHGLAYIPLATNAVRQGILVGKNIETPTVKYIGTQSSSGLKLYDQIMVSTGLTLDSAKRAGINADRVVVKDNYRPEFMPTTAEVLMSLVYDKDSRKILGGSLMSTYDISQSANTLSVCIQDGDTIDELAMVDMLFQPQFDRPFNYLNILAQAAQAKADK

SEQ ID NO: 96 - protein, 452 aa, Lentilactobacillus parakefiri
MKVAVIGCTHAGTFAIKTILAEHPDAEVTVYEKNDNISFLSCGIALYLGGHVKDPQGLFYSSPDELKKLGANVKMNHEVTNVDPASKTIEVSDLKNDQQFEDTYDKLVVTSGSWPVIPPIKGVDNKNVYLCKNWNHAKELFETAPEKKRITIVGAGYIGAELAEAYNTKGHDVTLLDGADRIMSKYFDKEFTDVVEKDFTDHGVTLGLDQQVTEISGEDTVTIKTTKGSYETDLVVLCVGFRPNTGLFKGKLAMTDNGALITNEYMQTSDPDIYGAGDSVAVHYNPTHGLAYIPLATNAVRQGILVGKNIEKPTVKYMGTQSSSGLKLYDKTIVSTGLTMAAAKAQNINASEVIITDNYRPEFMPTTEPVLMSLVYDPDSRRILGGSLLSTYDVSQSANTLSVCIQNENTIDDLAMVDMLFQPQFDRPFNYLNILGQAAQEQADKLTKAASK

SEQ ID NO: 97 - protein, 452 aa, Lactobacillus farraginis
MKIAVIGCTHAGTFAVKTILSEHPDAQVTVYEKNDNISFLSCGIALYLGQQVKDPQGLFYSNPEELKTLGANVKMNHEVTDVDPEAKTITVTNLTEGKQFTDTYDKLVATTGSWPIMPPIQGIDNKNVYLCKNWNHAQELFKTAPAKKRITVVGAGYIGAELAEAYSTTGHDVTLIDGADRVMSKYFDRQFTDVVEQDYKDHGVTLALGQQVTGISGDDTVTITTTKGSYETDLVIMCVGFKPNTSLFKGKLEMLKNGALITNAYMQTSDPDIYAAGDSVAVHYNPTNSPAYIPLATNAVRQGILVGKNIEQPTVKYMGTQSSSGLKLYDRTIVSTGLTMAAANQQGINAAVVTITDNYRPEFMPTTEPVLMSLVYNPENRQILGGTLMSTYDVSQSANTLSVCIQNQNTIDDLAMVDMLFQPQFDRPFNYLNILGQAAQQQLAQQADSVKA

SEQ ID NO: 98 - protein, 414 aa, Staphylococcus aureus
MTENNNLVTSTQGIIKEALHKLGFDEGMYDLIKEPLRMLQVRIPVRMDDGTVKTFTGYRAQHNDAVGPTKGGVRFHPDVDEEEVKALSMWMTLKCGIVNLPYGGGKGGIVCDPRQMSIHEVERLSRGYVRAISQFVGPNKDIPAPDVFTNSQIMAWMMDEYSALDKFNSPGFITGKPIVLGGSHGRDRSTALGVVIAIEQAAKRRNMQIEGAKVVIQGFGNAGSFLAKFLYDLGAKIVGISDAYGALHDPNGLDIDYLLDRRDSFGTVTNLFEETISNKELFELDCDILVPAAISNQITEDNAHDIKASIVVEAANGPTTPEATRILTERGILLVPDVLASAGGVTVSYFEWVQNNQGYYWSEEEVNEKLREKLEAAFDTIYELSQNRKIDMRLAAYIIGIKRTAEAARYRGWA

SEQ ID NO: 99 - protein, 424 aa, Bacillus subtilis
MSAKQVSKDEEKEALNLFLSTQTIIKEALRKLGYPGDMYELMKEPQRMLTVRIPVKMDNGSVKVFTGYRSQHNDAVGPTKGGVRFHPEVNEEEVKALSIWMTLKCGIANLPYGGGKGGIICDPRTMSFGELERLSRGYVRAISQIVGPTKDIPAPDVYTNSQIMAWMMDEYSRLREFDSPGFITGKPLVLGGSQGRETATAQGVTICIEEAVKKKGIKLQNARIIIQGFGNAGSFLAKFMHDAGAKVIGISDANGGLYNPDGLDIPYLLDKRDSFGMVTNLFTDVITNEELLEKDCDILVPAAISNQITAKNAHNIQASIVVEAANGPTTIDATKILNERGVLLVPDILASAGGVTVSYFEWVQNNQGYYWSEEEVAEKLRSVMVSSFETIYQTAATHKVDMRLAAYMTGIRKSAEASRFRGWV

SEQ ID NO: 100 - protein, 1620 aa, Pseudomonas aeruginosa
MAFFTAASKADFQHQLQTALAQHLGDKALPQVTLFAEQFFSLISLDELTQRRLSDLVGCTLSAWRLLERFDRDQPEVRVYNPDYEKHGWQSTHTAVEVLHPDLPFLVDSVRMELNRRGYSIHTLQTNVLSVRRSAKGELKEILPKGSQGKDVSQESLMYLEIDRCAHAGELRALEKAILEVLGEVRVTVADFEPMKAKARELLTWLGKAKLKVPAEELKEVRSYLEWLLDNHFTFLGYEEFSVADEADGGRMVYDEKSFLGLTRLLRAGLSKDDLHIEDYAVAYLREPVLLSFAKAAHPSRVHRPAYPDYVSIRELDGKGRVIRECRFMGLFTSSVYNESVNDIPFIRGKVAEVMRRSGFDTKAHLGKELAQVLEVLPRDDLFQTPVDELFSTALAIVRIQERNKIRVFLRKDPYGRFCYCLAYVPRDVYSTETRLKIQQVLMERLQASDCEFWTFFSESVLARVQFILRVDPKSRIDIDPARLEEEVIQACRSWQDDYSSLVVENLGEAKGTNVLADFPKGFPAGYRERFAPHFAVVDLQHLLSLSEQRPLVMSFYQPLAQGEQQLHCKLYHADTPLALSDVLPILENLGLRVLGEFPYRLRHQNGREYWIHDFAFTYAEGLDVDIQQLNEILQDAFVHIVSGDAENDAFNRLVLTANLPWRDVALLRAYARYLKQIRLGFDLGYIASALNAHTDIARELVRLFKTRFYLARKLTAEDLEDKQQKLEQAILGALDEVQVLNEDRILRRYLDLIKATLRTNFYQPDGNGQNKSYFSFKFNPKAIPELPRPVPKYEIFVYSPRVEGVHLRGGKVARGGLRWSDREEDFRTEVLGLVKAQQVKNAVIVPVGAKGGFVPRRLPLGGSRDEIQAEAIACYRIFISGLLDITDNLKEGEVVPPANVVRHDEDDPYLVVAADKGTATFSDIANGIAAEYGFWLGDAFASGGSAGYDHKGMGITAKGAWVSVQRHFRERGIDVQKDNISVIGIGDMAGDVFGNGLLMSDKLQLVAAFNHMHIFIDPNPDAASSFVERQRLFNLPRSSWADYDAKLISAGGGIFLRSAKSIAITPEMKARFDIQADRLAPTELIHALLKAPVDLLWNGGIGTYVKSSKETHADVGDKANDGLRVDGRELRAKVVGEGGNLGMTQLARVEFGLHGGANNTDFIDNAGGVDCSDHEVNIKILLNEVVQAGDMTEKQRNALLVKMTDAVGALVLGNNYKQTQALSLAQRRARERIAEYKRLMGDLEARGKLDRALEFLPSDEELAERISAGQGLTRAELSVLISYSKIDLKESLLKSLVPDDDYLTRDMETAFPALLAEKFGDAMRRHRLKREIVSTQIANDLVNHMGITFVQRLKESTGMSAANVAGAYVIVRDVFHLPHWFRQIENLDYQVPADIQLTLMDELMRLGRRATRWFLRSRRNELDAARDVAHFGPRIAALGLKLNELLEGPTRELWQARYQTYVDAGVPELLARMVAGTSHLYTLLPIIEASDVTGQDTAEVAKAYFAVGSALDLTWYLQQITNLPVENNWQALAREAFRDDLDWQQRAITVSVLQMQDGPKEVEARVGLWLEQHLPLVERWRAMLVELRAASGTDYAMYAVANRELMDLAQSSQHGVCIP

SEQ ID NO: 101 - protein, 450 aa, Clostridium symbiosum
MSKYVDRVIAEVEKKYADEPEFVQTVEEVLSSLGPVVDAHPEYEEVALLERMVIPERVIEFRVPWEDDNGKVHVNTGYRVQFNGAIGPYKGGLRFAPSVNLSIMKFLGFEQAFKDSLTTLPMGGAKGGSDFDPNGKSDREVMRFCQAFMTELYRHIGPDIDVPAGDLGVGAREIGYMYGQYRKIVGGFYNGVLTGKARSFGGSLVRPEATGYGSVYYVEAVMKHENDTLVGKTVALAGFGNVAWGAAKKLAELGAKAVTLSGPDGYIYDPEGITTEEKINYMLEMRASGRNKVQDYADKFGVQFFPGEKPWGQKVDIIMPCATQNDVDLEQAKKIVANNVKYYIEVANMPTTNEALRFLMQQPNMVVAPSKAVNAGGVLVSGFEMSQNSERLSWTAEEVDSKLHQVMTDIHDGSAAAAERYGLGYNLVAGANIVGFQKIADAMMAQGIAW

SEQ ID NO: 102 - protein, 1092 aa, Saccharomyces cerevisiae
MLFDNKNRGALNSLNTPDIASLSISSMSDYHVFDFPGKDLQREEVIDLLDQQGFIPDDLIEQEVDWFYNSLGIDDLFFSRESPQLISNIIHSLYASKLDFFAKSKFNGIQPRLFSIKNKIITNDNHAIFMESNTGVSISDSQQKNFKFASDAVGNDTLEHGKDTIKKNRIEMDDSCPPYELDSEIDDLFLDNKSQKNCRLVSFWAPESELKLTFVYESVYPNDDPAGVDISSQDLLKGDIESISDKTMYKVSSNENKKLYGLLLKLVKEREGPVIKTTRSVENKDEIRLLVAYKRFTTKRYYSALNSLFHYYKLKPSKFYLESFNVKDDDIIIFSVYLNENQQLEDVLLHDVEAALKQVEREASLLYAIPNNSFHEVYQRRQFSPKEAIYAHIGAIFINHFVNRLGSDYQNLLSQITIKRNDTTLLEIVENLKRKLRNETLTQQTIINIMSKHYTIISKLYKNFAQIHYYHNSTKDMEKTLSFQRLEKVEPFKNDQEFEAYLNKFIPNDSPDLLILKTLNIFNKSILKTNFFITRKVAISFRLDPSLVMTKFEYPETPYGIFFVVGNTFKGFHIRFRDIARGGIRIVCSRNQDIYDLNSKNVIDENYQLASTQQRKNKDIPEGGSKGVILLNPGLVEHDQTFVAFSQYVDAMIDILINDPLKENYVNLLPKEEILFFGPDEGTAGFVDWATNHARVRNCPWWKSFLTGKSPSLGGIPHDEYGMTSLGVRAYVNKIYETLNLTNSTVYKFQTGGPDGDLGSNEILLSSPNECYLAILDGSGVLCDPKGLDKDELCRLAHERKMISDFDTSKLSNNGFFVSVDAMDIMLPNGTIVANGTTFRNTFHTQIFKFVDHVDIFVPCGGRPNSITLNNLHYFVDEKTGKCKIPYIVEGANLFITQPAKNALEEHGCILFKDASANKGGVTSSSMEVLASLALNDNDFVHKFIGDVSGERSALYKSYVVEVQSRIQKNAELEFGQLWNLNQLNGTHISEISNQLSFTINKLNDDLVASQELWLNDLKLRNYLLLDKIIPKILIDVAGPQSVLENIPESYLKVLLSSYLSSTFVYQNGIDVNIGKFLEFIGGLKREAEASA

SEQ ID NO: 103 - protein, 420 aa, Pyrococcus furiosus
MVEQDPYEIVIKQLERAAQYMEISEEALEFLKRPQRIVEVTIPVEMDDGSVKVFTGFRVQHNWARGPTKGGIRWHPEETLSTVKALAAWMTWKTAVMDLPYGGGKGGIIVDPKKLSDREKERLARGYIRAIYDVISPYEDIPAPDVYTNPQIMAWMMDEYETISRRKTPAFGIITGKPLSIGGSLGRIEATARGASYTIREAAKVLGWDTLKGKTIAIQGYGNAGYYLAKIMSEDFGMKVVAVSDSKGGIYNPDGLNADEVLKWKNEHGSVKDFPGATNITNEELLELEVDVLAPAAIEEVITKKNADNIKAKIVAEVANGPVTPEADEILFEKGILQIPDFLCNAGGVTVSYFEWVQNITGYYWTIEEVRERLDKKMTKAFYDVYNIAKEKNIHMRDAAYVVAVQRVYQAMLDRGWVKH

SEQ ID NO: 104 - protein, 421 aa, Thermococcus kodakarensis
MVEIDPFEMAVQQLERAAQFMDISEEALEWLKRPMRIVEVSVPVEMDDGSVKVFTGFRVQHNWARGPTKGGIRWHPAETLSTVKALATWMTWKVAVVDLPYGGGKGGIIVDPKKLSEREQERLARSYIRAVYDVIGPWTDIPAPDVYTNPKIMAWMMDEYETIMRRKGPAFGVITGKPPGVGGIVARMDATARGAAFTIREAAKALGWDDLKGKTIAIQGYGNAGYYLHKIMSEEFGMKVVAVSDSKGGIYNPDGLPPADEVLKWKKEHGSVKDMPGTQNITNEELLELEVDILAPSAIEGVITKENADNVKAKIVAEVANGPVTPEADEILHEKGILQIPDFLCNAGGVTVSYFEWVQNINGFYWTVEETRKRLDDKMTKAFWDVFNTHKEKNIHMRDAAYVVAVSRVYEAMKHRGWVKK

SEQ ID NO: 105 - protein, 448 aa, Lactobacillus sp.
MSNAKSYIESVKDTIQRRDPNQTEFQEAAFTVLDTLEPVLDKHPEYIKANLLERLVEPERAIQFRVPWQSDDGQFHVNRGFRVQFNSAIGPYKGGLRLHPSVSLDVVKFLGFEQVLKNSLTGLPIGGAKGGSDFNPKGKSDSEVMRFCQSFMTELQRHIGPDLDVPAGDIGVGGREIGFLFGAYKRLNGYQNGVLTGKGLTFGGSLARPEATGFGLLYYTHAMLKALGDTLTNKKIKVSGAGNVATYAIQKATEYGATVITCSDSDGYVYDPNGIDFKLVKQIKEVERGRIKEYAQRVETAEYHDGSVWDFDINYDIALPCATQNEISKDQAKLIAKDRVKYVCEGANMPSVPDAIATYRDNNIYYGPAKAANAGGVAVSALEMSQNSERLSWSFETVDNRLHDIMDNIFEISEAADKEYQLNQDYQAGANIAGFEKVAQTMMAQGLV

SEQ ID NO: 106 - protein, 1646 aa, Streptomyces sp.
MQTKLDEAKAELLERAARVAENSPVGGHLPTGTADEGTPDRESVLAFLQRYYLHTAPEDLTDRDPVDVFGAALSHYRLAENRPQGTANVRVLTPTVEENGWACSHSIVEVVTDDMPFLVDSVTNELTRQGRGIHVVIHPQVVVRRDLTGQLIEVLPQRPSGDRSALPHDAHTESWIHVEIDRETDRADLKQITADLLRVLSDVREAVEDWEKMREAALRIAEDLPAEPTASDLPEQEVEEARELLRWLAADHFTFLGYREYQLREDDSLAAVPGTGLGILRSDPHHASEDSHPVSPSFERLPADARAKAREHRLLVLTKANSRATVHRPSYLDYIGVKKFDADGNVVGERRFLGLFSSAAYTESVRRVPVIRRKVAEVLQRAGFSPNSHDGRDLLQILETYPRDELFQTPADELQSIVTSVLYLQERRRLRLYLRQDEYGRYYSALVYLPRDRYTTGVRLRIIDILKEELGGISVDFTAWNTESILSRLHFVVRVPQGTELPELSDSDKERIEARLVEAARSWADGFAEALTGELGEERAAELLRRYGNAFPEGYKADHTPRAAVADLCHLEQLTEDSNFALSLYEPVGAAPEERRFKIYRKGEAVSLSAVLPVLSRLGVEVTDERPYELRCADRTASWIYDFGLRMPKAQNGAGDYLGDDGRERFQEAFAATWTGKAENDGFNALVLSAGLTWRQAMVLRAYAKYLRQAGSTFSQDYMEDTLRNNVHTTRLLVSLFEARMSPDRQRAGHEIVDALLEEVDAALDQVASLDEDRILRSFLTVIKATLRTNFFQEALGGQPHDYVSMKFDPQAIPDLPAPRPAFEIWVYSPRVEGVHLRFGKVARGGLRWSDRREDFRTEILGLVKAQMVKNTVIVPVGAKGGFVAKQLPDPGVDREAWLAEGIASYKVFISALLDITDNMVAGEVVPPADVVRHDEDDTYLVVAADKGTATFSDIANGVAESYNFWLGDAFASGGSAGYDHKGMGITARGAWESVKRHFRELDVDTQTEDFTVVGIGDMSGDVFGNGMLLSEHIRLVAAFDHRHIFIDPTPDAATSYAERRRVFELPRSSWADYNTELISAGGGVFPRSAKAIQLNAHIREALGIEGKVSKMTPADLMKAILKAPVDLLWNGGIGTYVKSSAESHGDVGDKANDPIRVDGADLRVKVVGEGGNLGLTQLGRIEFALHGGKINTDAIDNSAGVDTSDHEVNIKILLNGLVTEGDMTVKQRNKLLAEMTDEVGHLVLRNNYAQNTAIANALAQSKDMLHAQQRFMRHLVREGHLDRALEFLPTDRQIRERLTNGQGLTGPETAVLLAYTKITVSDELLHTSLPDDPYLRTLLDAYFPSALRERFPEQMHGHPLAREIITTVLVNDTVNTGGTTYLHRLREETGASLEEIVRAQTAARAIFRSAAVWDGVESLDNRVEAAVQTRIRLHSRRLVERGTRWLLNNRPQPLQLAETVEFFGERVEQVWSQLPKLLKGADLEWYQQIYDELSGAGVPDELATRVAGFSSAFPTLDIVSVADRNGKEPLDVAEVYYDLADRLHITQLMDRIIELPRADRWQSMARASIREDLYAAHAAVTADVLAVGNGTSTPEQRFKAWEEKNAAILGRARSTLEEIQGSETFDLANLSVAMRTMRTLLRTHS

SEQ ID NO: 107 - protein, 1626 aa, Brevibacterium sp.
MTQVSISDVAEEWRKLRGQGAPENFLDAYYPRFETGASDPEAYAAAAARHFAVGTEYDGQTPAIAIYNPAVDSPEFRDNHTVVALVLADMPHLVSSIVSDLAAAGRAIRRVHHPIITVSGSGSDLSIVSPAEAPSVTADTASLPQVSAAPDAQSSDDPQQQSWIRLEIDRIPEDDFAELEQRLREVLAYVAAAARDAQAMASKAKDIAAELSAHAPRPELASEAEAAAALLNWLDGHFTFLGYREYDYTHDAEHSSLEPIEDTSMGISALRPLVKSPLSRAVAEKALEPHVLVLTKANSRSRVIRSSFMDYIGVKTFDSSGEIVGERRFVGVFKPEFYNDSVLNIPVIDRKVSRILSASGFPAGSHSANELLGVLETYPREDLLHEDTEEIFDVVMEIVDMQERRESRVFVRADPYQRFVSVILYLPRDLYNTDARVRVQEVLREFYNADSVDFDVLLSESALARIHFVARMARDEQLPQISAEDVERRIVGAVRSWSEDVHAFLIPAEHGDSGTTNARADLWSKAFPPSYGEHHTPAEAVADVGRFEALDAGHGSAVRLYRPERSADASVRLVLYRYERVGLSEVLPFLTAFGATVIDERPHELDLADGSHRYIYDFGLSFSEELGDDDCERISDAFMAGWEGKKEAGVFDRLIVTGLSWQHVTIIRALGKYLRQAGFTYSDAYVGEVYSDHPEISKLLVDYFAAKFDPAADDESREGAMAEIDDAIEAALSEVASLDADRVLRSSLELLRATLRTNYYIDESGELPTALVLKIRPTELSFVPKPKPALEMWVYSPQVEGAHLRFGAVARGGLRWSDRRDDFRTEVLGLVKAQMVKNALIVPTGAKGGFFPKQLPPMSDRDAWMAAGQAAYEVFIESMLEVSDDLTYGADDSSVVVHPDRVVRHDGDDYYLVVAADKGTARFSDVANAIAERRGFWLGDAFASGGSVGYDHKKMAITSRGAWKSVERHFRELGLNTAADDFTVVGIGDMSGDVFGNGMLRSEHIRLVAAFDHRDIFLDPNPDAARSFVERQRLFDLPRSSWQDYDRELISAGGGVFSRSAKSIDLSAEAASVLGVDPGRRSPADLMSEILKAPVDLVYNGGIGTYIKASTESHAEVGDKSNDSIRIDGADVRARVIGEGGNLGVTQLGRVEAALNGVEINTDAVDNSAGVDSSDHEVNIKLLLRTLVHKGAFAAEEREQVLHSFTDQVADRVLSNNYSQNVVLGEARAQTEAMSGTYGRLLNYLEKHADLDRAVEFLPNADELAKRRFGYYVSPELAVLLAYVKMHAADEILDSVVPDEMWMRRELVSYFPESLQEKYGELIPEHPLHREIATAKLVNRLVDRGGLTYIYRMLEETPASVPQIARVFVVVSEIFGLDDYFEAVCALDNEVPTEVQVKLQHDYVRLLDRSSRWLVQQAPDTLDVDSGIEMYGKVVEALRSRVPELVDGYDAESMQAKAQEYIDDGVPSDLAWRAAALLDEFVLLDITQLAARANESAEDVAEVYYAVNEHFAGSQVLTLIGGLDRSDRWSALARGSMRDDFYSAILSVAETVLAATDSPISGTPDERAKQRVAEWLERNETVVSRVIETTETILGLDSVTQAPLSVLLRSLRSMVRSSTWESEHNS

SEQ ID NO: 108 - protein, 362 aa, Escherichia coli
MAQIFNFSSGPAMLPAEVLKQAQQELRDWNGLGTSVMEVSHRGKEFIQVAEEAEKDFRDLLNVPSNYKVLFCHGGGRGQFAAVPLNILGDKTTADYVDAGYWAASAIKEAKKYCTPNVFDAKVTVDGLRAVKPMREWQLSDNAAYMHYCPNETIDGIAIDETPDFGADVVVAADFSSTILSRPIDVSRYGVIYAGAQKNIGPAGLTIVIVREDLLGKANIACPSILDYSILNDNGSMFNTPPTFAWYLSGLVFKWLKANGGVAEMDKINQQKAELLYGVIDNSDFYRNDVAKANRSRMNVPFQLADSALDKLFLEESFAAGLHALKGHRVVGGMRASIYNAMPLEGVKALTDFMVEFERRHG

SEQ ID NO: 109 - protein, 322 aa, Escherichia coli [sequence omitted]

SEQ ID NO: 110 - protein, 387 aa, Escherichia coli
MSVIKMTDLDLAGKRVFIRADLNVPVKDGKVTSDARIRASLPTIELALKQGAKVMVTSHLGRPTEGEYNEEFSLLPVVNYLKDKLSNPVRLVKDYLDGVDVAEGELVVLENVRFNKGEKKDDETLSKKYAALCDVFVMDAFGTAHRAQASTHGIGKFADVACAGPLLAAELDALGKALKEPARPMVAIVGGSKVSTKLTVLDSLSKIADQLIVGGGIANTFIAAQGHDVGKSLYEADLVDEAKRLLTTCNIPVPSDVRVATEFSETAPATLKSVNDVKADEQILDIGDASAQELAEILKNAKTILWNGPVGVFEFPNFRKGTEIVANAIADSEAFSIAGGGDTLAAIDLFGIADKISYISTGGGAFLEFVEGKVLPAVAMLEERAKK

SEQ ID NO: 111 - DNA, 97 bp, synthetic construct
  source 1..97: mol_type = other DNA
  modified_base 8: mod_base = OTHER; note = Uracil
ataggcctttgacagctagctcagtcctaggtataatgctagctcttaatcatgctaaggaggattaactttatgagccagaatggccgtccggtag

SEQ ID NO: 112 - DNA, 109 bp, synthetic construct
  source 1..109: mol_type = other DNA
  modified_base 8: mod_base = OTHER; note = Uracil
ataggcctaaaaagagtattgacttaaagtctaacctataggtataatgtgtggatcttaatcatgctaaggaggattaactttatgagccagaatggccgtccggtag

SEQ ID NO: 113 - DNA, 109 bp, synthetic construct
  source 1..109: mol_type = other DNA
  modified_base 8: mod_base = OTHER; note = Uracil
ataggcctaaaaaatttatttgctttcgcatctttttgtacctataatgtgtggatcttaatcatgctaaggaggattaactttatgagccagaatggccgtccggtag

SEQ ID NO: 114 - DNA, 108 bp, synthetic construct
  source 1..108: mol_type = other DNA
  modified_base 8: mod_base = OTHER; note = Uracil
ataggcctaaaaagagtattgacttcgcatctttttgtacctataatgtgtggatcttaatcatgctaaggaggattaactttatgagccagaatggccgtccggtag

SEQ ID NO: 115 - DNA, 97 bp, synthetic construct
  source 1..97: mol_type = other DNA
  modified_base 8: mod_base = OTHER; note = Uracil
ataggcctttgacagctagctcagtcctaggtactgtgctagctcttaatcatgctaaggaggattaactttatgagccagaatggccgtccggtag

SEQ ID NO: 116 - DNA, 98 bp, synthetic construct
  source 1..98: mol_type = other DNA
  modified_base 8: mod_base = OTHER; note = Uracil
ataggcctttgacaattaatcatccggctcgtaatttatgtggatcttaatcatgctaaggaggattaactttatgagccagaatggccgtccggtag

SEQ ID NO: 117 - DNA, 98 bp, synthetic construct
  source 1..98: mol_type = other DNA
  modified_base 8: mod_base = OTHER; note = Uracil
ataggcctttgacaattaatcatccggctcgtaatgtttgtggatcttaatcatgctaaggaggattaactttatgagccagaatggccgtccggtag

SEQ ID NO: 118 - DNA, 98 bp, synthetic construct
  source 1..98: mol_type = other DNA
  modified_base 8: mod_base = OTHER; note = Uracil
ataggcctttgacaattaatcatccggctcgtataatgtgtggatcttaatcatgctaaggaggattaactttatgagccagaatggccgtccggtag

SEQ ID NO: 119 - DNA, 98 bp, synthetic construct
  source 1..98: mol_type = other DNA
  modified_base 8: mod_base = OTHER; note = Uracil
ataggcctttgacaattaatcatccggctcttagtgtttgtggatcttaatcatgctaaggaggattaactttatgagccagaatggccgtccggtag

SEQ ID NO: 120 - DNA, 97 bp, synthetic construct
  source 1..97: mol_type = other DNA
  modified_base 8: mod_base = OTHER; note = Uracil
ataggcctttgcctcttaatcatcggctcgtataatgtgtggatcttaatcatgctaaggaggattaactttatgagccagaatggccgtccggtag

SEQ ID NO: 121 - DNA, 97 bp, synthetic construct
  source 1..97: mol_type = other DNA
  modified_base 8: mod_base = OTHER; note = Uracil
ataggcctctgacagctagctcagtcctaggtataatgctagctcttaatcatgctaaggaggattaactttatgagccagaatggccgtccggtag

SEQ ID NO: 122 - DNA, 97 bp, synthetic construct
  source 1..97: mol_type = other DNA
  modified_base 8: mod_base = OTHER; note = Uracil
ataggcctttgacagctagctcagtcctaggtattgtgctagctcttaatcatgctaaggaggattaactttatgagccagaatggccgtccggtag

SEQ ID NO: 123 - DNA, 97 bp, synthetic construct
  source 1..97: mol_type = other DNA
  modified_base 8: mod_base = OTHER; note = Uracil
ataggccttttacggctagctcagtcctaggtatagtgctagctcttaatcatgctaaggaggattaactttatgagccagaatggccgtccggtag

SEQ ID NO: 124 - DNA, 97 bp, synthetic construct
  source 1..97: mol_type = other DNA
  modified_base 8: mod_base = OTHER; note = Uracil
ataggccttttatagctagctcagcccttggtacaatgctagctcttaatcatgctaaggaggattaactttatgagccagaatggccgtccggtag

SEQ ID NO: 125 - DNA, 97 bp, synthetic construct
  source 1..97: mol_type = other DNA
  modified_base 8: mod_base = OTHER; note = Uracil
ataggccttttacggctagctcagccctaggtattatgctagctcttaatcatgctaaggaggattaactttatgagccagaatggccgtccggtag

SEQ ID NO: 126 - DNA, 97 bp, synthetic construct
  source 1..97: mol_type = other DNA
  modified_base 8: mod_base = OTHER; note = Uracil
ataggcctttgacagctagctcagtcctagggactatgctagctcttaatcatgctaaggaggattaactttatgagccagaatggccgtccggtag

SEQ ID NO: 127 - DNA, 24 bp, synthetic construct
  source 1..24: mol_type = other DNA
  modified_base 7: mod_base = OTHER; note = Uracil
acgaactcgccagccagcgccttg

SEQ ID NO: 128 - DNA, 29 bp, synthetic construct
  source 1..29: mol_type = other DNA
  modified_base 7: mod_base = OTHER; note = Uracil
agttcgtggcggatgctgtgaacgtttcc

SEQ ID NO: 129 - DNA, 34 bp, synthetic construct
  source 1..34: mol_type = other DNA
  modified_base 8: mod_base = OTHER; note = Uracil
aggcctatgctgaggtatcctcagccgcgcgcgc

SEQ ID NO: 130 - DNA, 18 bp, synthetic construct
  source 1..18: mol_type = other DNA
  modified_base 9: mod_base = OTHER; note = Uracil
agctgaggtcgcctcagc

SEQ ID NO: 131 - DNA, 27 bp, synthetic construct
  source 1..27: mol_type = other DNA
  modified_base 9: mod_base = OTHER; note = Uracil
acctcctatgtcacttctgattcaggc

SEQ ID NO: 132 - DNA, 39 bp, synthetic construct
  source 1..39: mol_type = other DNA
  modified_base 9: mod_base = OTHER; note = Uracil
ataggaggtcctcctatgtcaattcaacatttccgtgtc

SEQ ID NO: 133 - DNA, 28 bp, synthetic construct
  source 1..28: mol_type = other DNA
  modified_base 4: mod_base = OTHER; note = Uracil
  modified_base 9: mod_base = OTHER; note = Uracil
acctcagcttaccaatgcttaatcagtg

SEQ ID NO: 134 - DNA, 40 bp, synthetic construct
  source 1..40: mol_type = other DNA
  modified_base 9: mod_base = OTHER; note = Uracil
aaggaggatnnnnnnatgagycaraatggccgtccggtag

SEQ ID NO: 135 - DNA, 73 bp, synthetic construct
  source 1..73: mol_type = other DNA
  modified_base 12: mod_base = OTHER; note = Uracil
aaaattgaagatytgngccatnnnnnngtctccttcttttatcaaccaagctttattagtcaagatcaacctg

SEQ ID NO: 136 - DNA, 31 bp, synthetic construct
  source 1..31: mol_type = other DNA
  modified_base 12: mod_base = OTHER; note = Uracil
atcttcaattttagttctggtccggcaatgc

SEQ ID NO: 137 - DNA, 28 bp, synthetic construct
  source 1..28: mol_type = other DNA
  modified_base 9: mod_base = OTHER; note = Uracil
atcctccttagcatgattaagagctagc

SEQ ID NO: 138 - DNA, 27 bp, synthetic construct
  source 1..27: mol_type = other DNA
  modified_base 9: mod_base = OTHER; note = Uracil
agctgaggtcgcctcagcggccggccc

SEQ ID NO: 139 - DNA, 32 bp, synthetic construct
  source 1..32: mol_type = other DNA
  modified_base 9: mod_base = OTHER; note = Uracil
acctcagctttacttctgattcaggctgcctg

SEQ ID NO: 140 - DNA, 6783 bp, synthetic construct; identical to SEQ ID NO: 40
  source 1..6783: mol_type = other DNA

SEQ ID NO: 141 - DNA, 6783 bp, synthetic construct
  source 1..6783: mol_type = other DNA
tattcgcacctggcggtgctcaacgggaatcctgctctgcgaggctggccgtaggccggcctcagatccttccgtatttagccagtatgttctctagtgtggttcgttgtttttgcgtgagccatgagaacgaaccattgagatcatacttactttgcatgtcactcaaaaattttgcctcaaaactggtgagctgaatttttgcagttaaagcatcgtgtagtgtttttcttagtccgttatgtaggtaggaatctgatgtaatggttgttggtattttgtcaccattcatttttatctggttgttctcaagttcggttacgagatccatttgtctatctagttcaacttggaaaatcaacgtatcagtcgggcggcctcgcttatcaaccaccaatttcatattgctgtaagtgtttaaatctttacttattggtttcaaaacccattggttaagccttttaaactcatggtagttattttcaagcattaacatgaacttaaattcatcaaggctaatctctatatttgccttgtgagttttcttttgtgttagttcttttaataaccactcataaatcctcatagagtatttgttttcaaaagacttaacatgttccagattatattttatgaatttttttaactggaaaagataaggcaatatctcttcactaaaaactaattctaatttttcgcttgagaacttggcatagtttgtccactggaaaatctcaaagcctttaaccaaaggattcctgatttccacagttctcgtcatcagctctctggttgctttagctaatacaccataagcattttccctactgatgttcatcatctgagcgtattggttataagtgaacgataccgtccgttctttccttgtagggttttcaatcgtggggttgagtagtgccacacagcataaaattagcttggtttcatgctccgttaagtcatagcgactaatcgctagttcatttgctttgaaaacaactaattcagacatacatctcaattggtctaggtgattttaatcactataccaattgagatgggctagtcaatgataattacatgtccttttcctttgagttgtgggtatctgtaaattctgctagacctttgctggaaaacttgtaaattctgctagaccctctgtaaattccgctagacctttgtgtgttttttttgtttatattcaagtggttataatttatagaataaagaaagaataaaaaaagataaaaagaatagatcccagccctgtgtataactcactactttagtcagttccgcagtattacaaaaggatgtcgcaaacgctgtttgctcctctacaaaacagaccttaaaaccctaaaggcttaagtagcaccctcgcaagctcgggcaaatcgctgaatattccttttgtctccgaccatcaggcacctgagtcgctgtctttttcgtgacattcagttcgctgcgctcacggctctggcagtgaatgggggtaaatggcactacaggcgcggcgcgcccagctgtctagggcggcggatttgtcctactcaggagagcgttcaccgacaaacaacagataaaacgaaaggcccagtctttcgactgagcctttcgttttatttgatgcctttaattaagcggccgcggcgcgcccgtcgacgcgcgcgcggctgaggatacctcagcataggcctttgacagctagctcagtcctaggtataatgctagctcttaatcatgctaaggaggatttgtgacatgagtcagaatggccgtccggtagtcctcatcgccgataagcttgcgcagtccactgttgacgcgcttggagatgcagtagaagtccgttgggttgacggacctaaccgcccagaactgcttgatgcagttaaggaagcggacgcactgctcgtgcgttctgctaccactgtcgatgctgaagtcatcgccgctgcccctaacttgaagatcgtcggtcgtgccggcgtgggcttggacaacgttgacatccctgctgccactgaagctggcgtcatggttgctaacgcaccgacctctaatattcactccgcttgtgagcacgcaatttctttgctgctgtctactgctcgccagatccctgctgctgatgcgacgctgcgtgagggcgagtggaagcggtcttctttcaacggtgtggaaattttcggaaaaactgtcggtatcgtcggttttggccacattggtcagttgtttgctcagcgtcttgctgcgtttgagaccaccattgttgcttacgatccttacgctaaccctgctcgtgcggctcagctgaacgttgagttggttgagttggatgagctgatgagccgttctgactttgtcaccattcaccttcctaagaccaaggaaactgctggcatgtttgatgcgcagctccttgctaagtccaagaagggccagatcatcatcaacgctgctcgtggtggccttgttgatgagcaggctttggctgatgcgattgagtccggtcacattcgtggcgctggtttcgatgtgtactccaccgagccttgcactgattctcctttgttcaagttgcctcaggttgttgtgactcctcacttgggtgggtctactgaagaggctcaggatcgtgcgggtactgacgttgctgattctgtgctcaaggcgctggctggcgagttcgtggcggatgctgtgaacgtttccggtggtcgcgtgggcgaagaggttgctgtgtggatggatctggctcgcaagcttggtcttcttgctggcaagcttgtcgacgccgccccagtctccattgaggttgaggctcgaggcgagctttcttccgagcaggtcgatgcacttggtttgtccgctgttcgtggtttgttctccggaattatcgaagagtccgttactttcgtcaacgctcctcgcattgctgaagagcgtggcctggacatctccgtgaagaccaactctgagtctgttactcaccgttccgtcctgcaggtcaaggtcattactggcagcggcgcgagcgcaactgttgttggtgccctgactggtcttgagcgcgttgagaagatcacccgcatcaatggccgtggcctggatctgcgcgcagagggtctgaacctcttcctgcaggccactgacgctcctggtgcactgggtaccgttggtaccaagctgggtgctgctggcatcaacatcgaggctgctgcgttgactcaggctgagaagggtgacggcgctgtcctgatcctgcgtgttgagtccgctgtctctgaagagctggaagctgaaatcaacgctgagttgggtgctacttccttccaggttgatcttgactaataaagcttggttgataaaagaaggagacttgccgatggcgcaatcttcaattttagttctggtccggcaatgctaccggcagaggtgcttaaacaggctcaacaggaactgcgcgactggaacggtcttggtacgtcggtgatggaagtgagtcaccgtggcaaagagttcattcaggttgcagaggaagccgagaaggattttcgcgatcttcttaatgtcccctccaactacaaggtattattctgccatggcggtggtcgcggtcagtttgctgcggtaccgctgaatattctcggtgataaaaccaccgcagattatgttgatgccggttactgggcggcaagtgccattaaagaagcgaaaaaatactgcacgcctaatgtctttgacgccaaagtgactgttgatggtctgcgcgcggttaagccaatgcgtgaatggcaactctctgataatgctgcttatatgcattattgcccgaatgaaaccatcgatggtatcgccatcgacgaaacgccagacttcggcgcagatgtggtggtcgccgctgacttctcttcaaccattctttcccgtccgattgacgtcagccgttatggtgtaatttacgctggcgcgcagaaaaatatcggcccggctggcctgacaatcgtcatcgttcgtgaagatttgctgggcaaagcgaatatcgcgtgtccgtcgattctggattattccatcctcaacgataacggctccatgtttaacacgccgccgacatttgcctggtatctatctggtctggtctttaaatggctgaaagcgaacggcggtgtagctgaaatggataaaatcaatcagcaaaaagcagaactgctatatggggtgattgataacagcgatttctaccgcaatgacgtggcgaaagctaaccgttcgcggatgaacgtgccgttccagttggcggacagtgcgcttgacaaattgttccttgaagagtcttttgctgctggccttcatgcactgaaaggtcaccgtgtggtcggcggaatgcgcgcttctatttataacgccatgccgctggaaggcgttaaagcgctgacagacttcatggttgagttcgaacgccgtcacggttgataaaagaaggagaccagtttatgcctaacattacctggtgcgacctgcctgaagatgtctctttatggccgggtctgcctctttcattaagtggtgatgaagtgatgccactggattaccacgcaggtcgtagcggctggctgctgtatggtcgtgggctggataaacaacgtctgacccaataccagagcaaactgggtgcggcgatggtgattgttgccgcctggtgcgtggaagattatcaggtgattcgtctggcaggttcactcaccgcacgggctacacgcctggcccacgaagcgcagctggatgtcgccccgctggggaaaatcccgcacctgcgcacgccgggtttgctggtgatggatatggactccaccgccatccagattgaatgtattgatgaaattgccaaactggccggaacgggcgagatggtggcggaagtaaccgaacgggcgatgcgcggcgaactcgattttaccgccagcctgcgcagccgtgtggcgacgctgaaaggcgctgacgccaatattctgcaacaggtgcgtgaaaatctgccgctgatgccaggcttaacgcaactggtgctcaagctggaaacgctgggctggaaagtggcgattgcctccggcggctttactttctttgctgaatacctgcgcgacaagctgcgcctgaccgccgtggtagccaatgaactggagatcatggacggtaaatttaccggcaatgtgatcggcgacatcgtagacgcgcagtacaaagcgaaaactctgactcgcctcgcgcaggagtatgaaatcccgctggcgcagaccgtggcgattggcgatggagccaatgacctgccgatgatcaaagcggcagggctggggattgcctaccatgccaagccaaaagtgaatgaaaaggcggaagtcaccatccgtcacgctgacctgatgggggtattctgcatcctctcaggcagcctgaatcagaagtgataagctgaggtcgcctcagcggccggcccctgcaggcgccggcgactagtcttggactcctgttgatagatccagtaatgacctcagaactccatctggatttgttcagaacgctcggttgccgccgggcgttttttattggtgagaatccaggggtccccaataattacgatttaaatttgtgtctcaaaatctctgatgttacattgcacaagataaaaatatatcatcatgaacaataaaactgtctgcttacataaacagtaatacaaggggtgttatgagccatattcagcgtgaaacgagctgtagccgtccgcgtctgaacagcaacatggatgcggatctgtatggctataaatgggcgcgtgataacgtgggtcagagcggcgcgaccatttatcgtctgtatggcaaaccggatgcgccggaactgtttctgaaacatggcaaaggcagcgtggcgaacgatgtgaccgatgaaatggtgcgtctgaactggctgaccgaatttatgccgctgccgaccattaaacattttattcgcaccccggatgatgcgtggctgctgaccaccgcgattccgggcaaaaccgcgtttcaggtgctggaagaatatccggatagcggcgaaaacattgtggatgcgctggccgtgtttctgcgtcgtctgcatagcattccggtgtgcaactgcccgtttaacagcgatcgtgtgtttcgtctggcccaggcgcagagccgtatgaacaacggcctggtggatgcgagcgattttgatgatgaacgtaacggctggccggtggaacaggtgtggaaagaaatgcataaactgctgccgtttagcccggatagcgtggtgacccacggcgattttagcctggataacctgattttcgatgaaggcaaactgattggctgcattgatgtgggccgtgtgggcattgcggatcgttatcaggatctggccattctgtggaactgcctgggcgaatttagcccgagcctgcaaaaacgtctgtttcagaaatatggcattgataatccggatatgaacaaactgcaatttcatctgatgctggatgaatttttctaataattaattggaccgttgtccttttccgctgcataaccctgcttcggggtcattatagcgattttttcggtatatccatcctttttcgcacgatatacaggattttgccaaagggttcgtgtagactttccttggtgtatccaacggcgtcagccgggcaggataggtgaagtaggcccacccgcgagcgggtgttccttcttcactgtccct

SEQ ID NO: 142 - DNA, 6783 bp, synthetic construct
  source 1..6783: mol_type = other DNA
tattcgcacctggcggtgctcaacgggaatcctgctctgcgaggctggccgtaggccggcctcagatccttccgtatttagccagtatgttctctagtgtggttcgttgtttttgcgtgagccatgagaacgaaccattgagatcatacttactttgcatgtcactcaaaaattttgcctcaaaactggtgagctgaatttttgcagttaaagcatcgtgtagtgtttttcttagtccgttatgtaggtaggaatctgatgtaatggttgttggtattttgtcaccattcatttttatctggttgttctcaagttcggttacgagatccatttgtctatctagttcaacttggaaaatcaacgtatcagtcgggcggcctcgcttatcaaccaccaatttcatattgctgtaagtgtttaaatctttacttattggtttcaaaacccattggttaagccttttaaactcatggtagttattttcaagcattaacatgaacttaaattcatcaaggctaatctctatatttgccttgtgagttttcttttgtgttagttcttttaataaccactcataaatcctcatagagtatttgttttcaaaagacttaacatgttccagattatattttatgaatttttttaactggaaaagataaggcaatatctcttcactaaaaactaattctaatttttcgcttgagaacttggcatagtttgtccactggaaaatctcaaagcctttaaccaaaggattcctgatttccacagttctcgtcatcagctctctggttgctttagctaatacaccataagcattttccctactgatgttcatcatctgagcgtattggttataagtgaacgataccgtccgttctttccttgtagggttttcaatcgtggggttgagtagtgccacacagcataaaattagcttggtttcatgctccgttaagtcatagcgactaatcgctagttcatttgctttgaaaacaactaattcagacatacatctcaattggtctaggtgattttaatcactataccaattgagatgggctagtcaatgataattacatgtccttttcctttgagttgtgggtatctgtaaattctgctagacctttgctggaaaacttgtaaattctgctagaccctctgtaaattccgctagacctttgtgtgttttttttgtttatattcaagtggttataatttatagaataaagaaagaataaaaaaagataaaaagaatagatcccagccctgtgtataactcactactttagtcagttccgcagtattacaaaaggatgtcgcaaacgctgtttgctcctctacaaaacagaccttaaaaccctaaaggcttaagtagcaccctcgcaagctcgggcaaatcgctgaatattccttttgtctccgaccatcaggcacctgagtcgctgtctttttcgtgacattcagttcgctgcgctcacggctctggcagtgaatgggggtaaatggcactacaggcgcggcgcgcccagctgtctagggcggcggatttgtcctactcaggagagcgttcaccgacaaacaacagataaaacgaaaggcccagtctttcgactgagcctttcgttttatttgatgcctttaattaagcggccgcggcgcgcccgtcgacgcgcgcgcggctgaggatacctcagcataggcctttgacagctagctcagtcctaggtataatgctagctcttaatcatgctaaggaggattgattcgatgtcgcagaatggccgtccggtagtcctcatcgccgataagcttgcgcagtccactgttgacgcgcttggagatgcagtagaagtccgttgggttgacggacctaaccgcccagaactgcttgatgcagttaaggaagcggacgcactgctcgtgcgttctgctaccactgtcgatgctgaagtcatcgccgctgcccctaacttgaagatcgtcggtcgtgccggcgtgggcttggacaacgttgacatccctgctgccactgaagctggcgtcatggttgctaacgcaccgacctctaatattcactccgcttgtgagcacgcaatttctttgctgctgtctactgctcgccagatccctgctgctgatgcgacgctgcgtgagggcgagtggaagcggtcttctttcaacggtgtggaaattttcggaaaaactgtcggtatcgtcggttttggccacattggtcagttgtttgctcagcgtcttgctgcgtttgagaccaccattgttgcttacgatccttacgctaaccctgctcgtgcggctcagctgaacgttgagttggttgagttggatgagctgatgagccgttctgactttgtcaccattcaccttcctaagaccaaggaaactgctggcatgtttgatgcgcagctccttgctaagtccaagaagggccagatcatcatcaacgctgctcgtggtggccttgttgatgagcaggctttggctgatgcgattgagtccggtcacattcgtggcgctggtttcgatgtgtactccaccgagccttgcactgattctcctttgttcaagttgcctcaggttgttgtgactcctcacttgggtgggtctactgaagaggctcaggatcgtgcgggtactgacgttgctgattctgtgctcaaggcgctggctggcgagttcgtggcggatgctgtgaacgtttccggtggtcgcgtgggcgaagaggttgctgtgtggatggatctggctcgcaagcttggtcttcttgctggcaagcttgtcgacgccgccccagtctccattgaggttgaggctcgaggcgagctttcttccgagcaggtcgatgcacttggtttgtccgctgttcgtggtttgttctccggaattatcgaagagtccgttactttcgtcaacgctcctcgcattgctgaagagcgtggcctggacatctccgtgaagaccaactctgagtctgttactcaccgttccgtcctgcaggtcaaggtcattactggcagcggcgcgagcgcaactgttgttggtgccctgactggtcttgagcgcgttgagaagatcacccgcatcaatggccgtggcctggatctgcgcgcagagggtctgaacctcttcctgcaggccactgacgctcctggtgcactgggtaccgttggtaccaagctgggtgctgctggcatcaacatcgaggctgctgcgttgactcaggctgagaagggtgacggcgctgtcctgatcctgcgtgttgagtccgctgtctctgaagagctggaagctgaaatcaacgctgagttgggtgctacttccttccaggttgatcttgactaataaagcttggttgataaaagaaggagaccccactatggctcaatcttcaattttagttctggtccggcaatgctaccggcagaggtgcttaaacaggctcaacaggaactgcgcgactggaacggtcttggtacgtcggtgatggaagtgagtcaccgtggcaaagagttcattcaggttgcagaggaagccgagaaggattttcgcgatcttcttaatgtcccctccaactacaaggtattattctgccatggcggtggtcgcggtcagtttgctgcggtaccgctgaatattctcggtgataaaaccaccgcagattatgttgatgccggttactgggcggcaagtgccattaaagaagcgaaaaaatactgcacgcctaatgtctttgacgccaaagtgactgttgatggtctgcgcgcggttaagccaatgcgtgaatggcaactctctgataatgctgcttatatgcattattgcccgaatgaaaccatcgatggtatcgccatcgacgaaacgccagacttcggcgcagatgtggtggtcgccgctgacttctcttcaaccattctttcccgtccgattgacgtcagccgttatggtgtaatttacgctggcgcgcagaaaaatatcggcccggctggcctgacaatcgtcatcgttcgtgaagatttgctgggcaaagcgaatatcgcgtgtccgtcgattctggattattccatcctcaacgataacggctccatgtttaacacgccgccgacatttgcctggtatctatctggtctggtctttaaatggctgaaagcgaacggcggtgtagctgaaatggataaaatcaatcagcaaaaagcagaactgctatatggggtgattgataacagcgatttctaccgcaatgacgtggcgaaagctaaccgttcgcggatgaacgtgccgttccagttggcggacagtgcgcttgacaaattgttccttgaagagtcttttgctgctggccttcatgcactgaaaggtcaccgtgtggtcggcggaatgcgcgcttctatttataacgccatgccgctggaaggcgttaaagcgctgacagacttcatggttgagttcgaacgccgtcacggttgataaaagaaggagaccagtttatgcctaacattacctggtgcgacctgcctgaagatgtctctttatggccgggtctgcctctttcattaagtggtgatgaagtgatgccactggattaccacgcaggtcgtagcggctggctgctgtatggtcgtgggctggataaacaacgtctgacccaataccagagcaaactgggtgcggcgatggtgattgttgccgcctggtgcgtggaagattatcaggtgattcgtctggcaggttcactcaccgcacgggctacacgcctggcccacgaagcgcagctggatgtcgccccgctggggaaaatcccgcacctgcgcacgccgggtttgctggtgatggatatggactccaccgccatccagattgaatgtattgatgaaattgccaaactggccggaacgggcgagatggtggcggaagtaaccgaacgggcgatgcgcggcgaactcgattttaccgccagcctgcgcagccgtgtggcgacgctgaaaggcgctgacgccaatattctgcaacaggtgcgtgaaaatctgccgctgatgccaggcttaacgcaactggtgctcaagctggaaacgctgggctggaaagtggcgattgcctccggcggctttactttctttgctgaatacctgcgcgacaagctgcgcctgaccgccgtggtagccaatgaactggagatcatggacggtaaatttaccggcaatgtgatcggcgacatcgtagacgcgcagtacaaagcgaaaactctgactcgcctcgcgcaggagtatgaaatcccgctggcgcagaccgtggcgattggcgatggagccaatgacctgccgatgatcaaagcggcagggctggggattgcctaccatgccaagccaaaagtgaatgaaaaggcggaagtcaccatccgtcacgctgacctgatgggggtattctgcatcctctcaggcagcctgaatcagaagtgataagctgaggtcgcctcagcggccggcccctgcaggcgccggcgactagtcttggactcctgttgatagatccagtaatgacctcagaactccatctggatttgttcagaacgctcggttgccgccgggcgttttttattggtgagaatccaggggtccccaataattacgatttaaatttgtgtctcaaaatctctgatgttacattgcacaagataaaaatatatcatcatgaacaataaaactgtctgcttacataaacagtaatacaaggggtgttatgagccatattcagcgtgaaacgagctgtagccgtccgcgtctgaacagcaacatggatgcggatctgtatggctataaatgggcgcgtgataacgtgggtcagagcggcgcgaccatttatcgtctgtatggcaaaccggatgcgccggaactgtttctgaaacatggcaaaggcagcgtggcgaacgatgtgaccgatgaaatggtgcgtctgaactggctgaccgaatttatgccgctgccgaccattaaacattttattcgcaccccggatgatgcgtggctgctgaccaccgcgattccgggcaaaaccgcgtttcaggtgctggaagaatatccggatagcggcgaaaacattgtggatgcgctggccgtgtttctgcgtcgtctgcatagcattccggtgtgcaactgcccgtttaacagcgatcgtgtgtttcgtctggcccaggcgcagagccgtatgaacaacggcctggtggatgcgagcgattttgatgatgaacgtaacggctggccggtggaacaggtgtggaaagaaatgcataaactgctgccgtttagcccggatagcgtggtgacccacggcgattttagcctggataacctgattttcgatgaaggcaaactgattggctgcattgatgtgggccgtgtgggcattgcggatcgttatcaggatctggccattctgtggaactgcctgggcgaatttagcccgagcctgcaaaaacgtctgtttcagaaatatggcattgataatccggatatgaacaaactgcaatttcatctgatgctggatgaatttttctaataattaattggaccgttgtccttttccgctgcataaccctgcttcggggtcattatagcgattttttcggtatatccatcctttttcgcacgatatacaggattttgccaaagggttcgtgtagactttccttggtgtatccaacggcgtcagccgggcaggataggtgaagtaggcccacccgcgagcgggtgttccttcttcactgtccct

SEQ ID NO: 143 - DNA, 6783 bp, synthetic construct
  source 1..6783: mol_type = other DNA
tattcgcacctggcggtgctcaacgggaatcctgctctgcgaggctggccgtaggccggcctcagatccttccgtatttagccagtatgttctctagtgtggttcgttgtttttgcgtgagccatgagaacgaaccattgagatcatacttactttgcatgtcactcaaaaattttgcctcaaaactggtgagctgaatttttgcagttaaagcatcgtgtagtgtttttcttagtccgttatgtaggtaggaatctgatgtaatggttgttggtattttgtcaccattcatttttatctggttgttctcaagttcggttacgagatccatttgtctatctagttcaacttggaaaatcaacgtatcagtcgggcggcctcgcttatcaaccaccaatttcatattgctgtaagtgtttaaatctttacttattggtttcaaaacccattggttaagccttttaaactcatggtagttattttcaagcattaacatgaacttaaattcatcaaggctaatctctatatttgccttgtgagttttcttttgtgttagttcttttaataaccactcataaatcctcatagagtatttgttttcaaaagacttaacatgttccagattatattttatgaatttttttaactggaaaagataaggcaatatctcttcactaaaaactaattctaatttttcgcttgagaacttggcatagtttgtccactggaaaatctcaaagcctttaaccaaaggattcctgatttccacagttctcgtcatcagctctctggttgctttagctaatacaccataagcattttccctactgatgttcatcatctgagcgtattggttataagtgaacgataccgtccgttctttccttgtagggttttcaatcgtggggttgagtagtgccacacagcataaaattagcttggtttcatgctccgttaagtcatagcgactaatcgctagttcatttgctttgaaaacaactaattcagacatacatctcaattggtctaggtgattttaatcactataccaattgagatgggctagtcaatgataattacatgtccttttcctttgagttgtgggtatctgtaaattctgctagacctttgctggaaaacttgtaaattctgctagaccctctgtaaattccgctagacctttgtgtgttttttttgtttatattcaagtggttataatttatagaataaagaaagaataaaaaaagataaaaagaatagatcccagccctgtgtataactcactactttagtcagttccgcagtattacaaaaggatgtcgcaaacgctgtttgctcctctacaaaacagaccttaaaaccctaaaggcttaagtagcaccctcgcaagctcgggcaaatcgctgaatattccttttgtctccgaccatcaggcacctgagtcgctgtctttttcgtgacattcagttcgctgcgctcacggctctggcagtgaatgggggtaaatggcactacaggcgcggcgcgcccagctgtctagggcggcggatttgtcctactcaggagagcgttcaccgacaaacaacagataaaacgaaaggcccagtctttcgactgagcctttcgttttatttgatgcctttaattaagcggccgcggcgcgcccgtcgacgcgcgcgcggctgaggatacctcagcataggcctttgacagctagctcagtcctaggtataatgctagctcttaatcatgctaaggaggattataattatgagtcagaatggccgtccggtagtcctcatcgccgataagcttgcgcagtccactgttgacgcgcttggagatgcagtagaagtccgttgggttgacggacctaaccgcccagaactgcttgatgcagttaaggaagcggacgcactgctcgtgcgttctgctaccactgtcgatgctgaagtcatcgccgctgcccctaacttgaagatcgtcggtcgtgccggcgtgggcttggacaacgttgacatccctgctgccactgaagctggcgtcatggttgctaacgcaccgacctctaatattcactccgcttgtgagcacgcaatttctttgctgctgtctactgctcgccagatccctgctgctgatgcgacgctgcgtgagggcgagtggaagcggtcttctttcaacggtgtggaaattttcggaaaaactgtcggtatcgtcggttttggccacattggtcagttgtttgctcagcgtcttgctgcgtttgagaccaccattgttgcttacgatccttacgctaaccctgctcgtgcggctcagctgaacgttgagttggttgagttggatgagctgatgagccgttctgactttgtcaccattcaccttcctaagaccaaggaaactgctggcatgtttgatgcgcagctccttgctaagtccaagaagggccagatcatcatcaacgctgctcgtggtggccttgttgatgagcaggctttggctgatgcgattgagtccggtcacattcgtggcgctggtttcgatgtgtactccaccgagccttgcactgattctcctttgttcaagttgcctcaggttgttgtgactcctcacttgggtgggtctactgaagaggctcaggatcgtgcgggtactgacgttgctgattctgtgctcaaggcgctggctggcgagttcgtggcggatgctgtgaacgtttccggtggtcgcgtgggcgaagaggttgctgtgtggatggatctggctcgcaagcttggtcttcttgctggcaagcttgtcgacgccgccccagtctccattgaggttgaggctcgaggcgagctttcttccgagcaggtcgatgcacttggtttgtccgctgttcgtggtttgttctccggaattatcgaagagtccgttactttcgtcaacgctcctcgcattgctgaagagcgtggcctggacatctccgtgaagaccaactctgagtctgttactcaccgttccgtcctgcaggtcaaggtcattactggcagcggcgcgagcgcaactgttgttggtgccctgactggtcttgagcgcgttgagaagatcacccgcatcaatggccgtggcctggatctgcgcgcagagggtctgaacctcttcctgcaggccactgacgctcctggtgcactgggtaccgttggtaccaagctgggtgctgctggcatcaacatcgaggctgctgcgttgactcaggctgagaagggtgacggcgctgtcctgatcctgcgtgttgagtccgctgtctctgaagagctggaagctgaaatcaacgctgagttgggtgctacttccttccaggttgatcttgactaataaagcttggttgataaaagaaggagacacatcaatggctcaatcttcaattttagttctggtccggcaatgctaccggcagaggtgcttaaacaggctcaacaggaactgcgcgactggaacggtcttggtacgtcggtgatggaagtgagtcaccgtggcaaagagttcattcaggttgcagaggaagccgagaaggattttcgcgatcttcttaatgtcccctccaactacaaggtattattctgccatggcggtggtcgcggtcagtttgctgcggtaccgctgaatattctcggtgataaaaccaccgcagattatgttgatgccggttactgggcggcaagtgccattaaagaagcgaaaaaatactgcacgcctaatgtctttgacgccaaagtgactgttgatggtctgcgcgcggttaagccaatgcgtgaatggcaactctctgataatgctgcttatatgcattattgcccgaatgaaaccatcgatggtatcgccatcgacgaaacgccagacttcggcgcagatgtggtggtcgccgctgacttctcttcaaccattctttcccgtccgattgacgtcagccgttatggtgtaatttacgctggcgcgcagaaaaatatcggcccggctggcctgacaatcgtcatcgttcgtgaagatttgctgggcaaagcgaatatcgcgtgtccgtcgattctggattattccatcctcaacgataacggctccatgtttaacacgccgccgacatttgcctggtatctatctggtctggtctttaaatggctgaaagcgaacggcggtgtagctgaaatggataaaatcaatcagcaaaaagcagaactgctatatggggtgattgataacagcgatttctaccgcaatgacgtggcgaaagctaaccgttcgcggatgaacgtgccgttccagttggcggacagtgcgcttgacaaattgttccttgaagagtcttttgctgctggccttcatgcactgaaaggtcaccgtgtggtcggcggaatgcgcgcttctatttataacgccatgccgctggaaggcgttaaagcgctgacagacttcatggttgagttcgaacgccgtcacggttgataaaagaaggagaccagtttatgcctaacattacctggtgcgacctgcctgaagatgtctctttatggccgggtctgcctctttcattaagtggtgatgaagtgatgccactggattaccacgcaggtcgtagcggctggctgctgtatggtcgtgggctggataaacaacgtctgacccaataccagagcaaactgggtgcggcgatggtgattgttgccgcctggtgcgtggaagattatcaggtgattcgtctggcaggttcactcaccgcacgggctacacgcctggcccacgaagcgcagctggatgtcgccccgctggggaaaatcccgcacctgcgcacgccgggtttgctggtgatggatatggactccaccgccatccagattgaatgtattgatgaaattgccaaactggccggaacgggcgagatggtggcggaagtaaccgaacgggcgatgcgcggcgaactcgattttaccgccagcctgcgcagccgtgtggcgacgctgaaaggcgctgacgccaatattctgcaacaggtgcgtgaaaatctgccgctgatgccaggcttaacgcaactggtgctcaagctggaaacgctgggctggaaagtggcgattgcctccggcggctttactttctttgctgaatacctgcgcgacaagctgcgcctgaccgccgtggtagccaatgaactggagatcatggacggtaaatttaccggcaatgtgatcggcgacatcgtagacgcgcagtacaaagcgaaaactctgactcgcctcgcgcaggagtatgaaatcccgctggcgcagaccgtggcgattggcgatggagccaatgacctgccgatgatcaaagcggcagggctggggattgcctaccatgccaagccaaaagtgaatgaaaaggcggaagtcaccatccgtcacgctgacctgatgggggtattctgcatcctctcaggcagcctgaatcagaagtgataagctgaggtcgcctcagcggccggcccctgcaggcgccggcgactagtcttggactcctgttgatagatccagtaatgacctcagaactccatctggatttgttcagaacgctcggttgccgccgggcgttttttattggtgagaatccaggggtccccaataattacgatttaaatttgtgtctcaaaatctctgatgttacattgcacaagataaaaatatatcatcatgaacaataaaactgtctgcttacataaacagtaatacaaggggtgttatgagccatattcagcgtgaaacgagctgtagccgtccgcgtctgaacagcaacatggatgcggatctgtatggctataaatgggcgcgtgataacgtgggtcagagcggcgcgaccatttatcgtctgtatggcaaaccggatgcgccggaactgtttctgaaacatggcaaaggcagcgtggcgaacgatgtgaccgatgaaatggtgcgtctgaactggctgaccgaatttatgccgctgccgaccattaaacattttattcgcaccccggatgatgcgtggctgctgaccaccgcgattccgggcaaaaccgcgtttcaggtgctggaagaatatccggatagcggcgaaaacattgtggatgcgctggccgtgtttctgcgtcgtctgcatagcattccggtgtgcaactgcccgtttaacagcgatcgtgtgtttcgtctggcccaggcgcagagccgtatgaacaacggcctggtggatgcgagcgattttgatgatgaacgtaacggctggccggtggaacaggtgtggaaagaaatgcataaactgctgccgtttagcccggatagcgtggtgacccacggcgattttagcctggataacctgattttcgatgaaggcaaactgattggctgcattgatgtgggccgtgtgggcattgcggatcgttatcaggatctggccattctgtggaactgcctgggcgaatttagcccgagcctgcaaaaacgtctgtttcagaaatatggcattgataatccggatatgaacaaactgcaatttcatctgatgctggatgaatttttctaataattaattggaccgttgtccttttccgctgcataaccctgcttcggggtcattatagcgattttttcggtatatccatcctttttcgcacgatatacaggattttgccaaagggttcgtgtagactttccttggtgtatccaacggcgtcagccgggcaggataggtgaagtaggcccacccgcgagcgggtgttccttcttcactgtccct

SEQ ID NO: 144 - DNA, 6783 bp, synthetic construct
  source 1..6783: mol_type = other DNA
tattcgcacctggcggtgctcaacgggaatcctgctctgcgaggctggccgtaggccggcctcagatccttccgtatttagccagtatgttctctagtgtggttcgttgtttttgcgtgagccatgagaacgaaccattgagatcatacttactttgcatgtcactcaaaaattttgcctcaaaactggtgagctgaatttttgcagttaaagcatcgtgtagtgtttttcttagtccgttatgtaggtaggaatctgatgtaatggttgttggtattttgtcaccattcatttttatctggttgttctcaagttcggttacgagatccatttgtctatctagttcaacttggaaaatcaacgtatcagtcgggcggcctcgcttatcaaccaccaatttcatattgctgtaagtgtttaaatctttacttattggtttcaaaacccattggttaagccttttaaactcatggtagttattttcaagcattaacatgaacttaaattcatcaaggctaatctctatatttgccttgtgagttttcttttgtgttagttcttttaataaccactcataaatcctcatagagtatttgttttcaaaagacttaacatgttccagattatattttatgaatttttttaactggaaaagataaggcaatatctcttcactaaaaactaattctaatttttcgcttgagaacttggcatagtttgtccactggaaaatctcaaagcctttaaccaaaggattcctgatttccacagttctcgtcatcagctctctggttgctttagctaatacaccataagcattttccctactgatgttcatcatctgagcgtattggttataagtgaacgataccgtccgttctttccttgtagggttttcaatcgtggggttgagtagtgccacacagcataaaattagcttggtttcatgctccgttaagtcatagcgactaatcgctagttcatttgctttgaaaacaactaattcagacatacatctcaattggtctaggtgattttaatcactataccaattgagatgggctagtcaatgataattacatgtccttttcctttgagttgtgggtatctgtaaattctgctagacctttgctggaaaacttgtaaattctgctagaccctctgtaaattccgctagacctttgtgtgttttttttgtttatattcaagtggttataatttatagaataaagaaagaataaaaaaagataaaaagaatagatcccagccctgtgtataactcactactttagtcagttccgcagtattacaaaaggatgtcgcaaacgctgtttgctcctctacaaaacagaccttaaaaccctaaaggcttaagtagcaccctcgcaagctcgggcaaatcgctgaatattccttttgtctccgaccatcaggcacctgagtcgctgtctttttcgtgacattcagttcgctgcgctcacggctctggcagtgaatgggggtaaatggcactacaggcgcggcgcgcccagctgtctagggcggcggatttgtcctactcaggagagcgttcaccgacaaacaacagataaaacgaaaggcccagtctttcgactgagcctttcgttttatttgatgcctttaattaagcggccgcggcgcgcccgtcgacgcgcgcgcggctgaggatacctcagcataggcctttgacagctagctcagtcctaggtataatgctagctcttaatcatgctaaggaggattcgccttatgtctcaaaatggccgtccggtagtcctcatcgccgataagcttgcgcagtccactgttgacgcgcttggagatgcagtagaagtccgttgggttgacggacctaaccgcccagaactgcttgatgcagttaaggaagcggacgcactgctcgtgcgttctgctaccactgtcgatgctgaagtcatcgccgctgcccctaacttgaagatcgtcggtcgtgccggcgtgggcttggacaacgttgacatccctgctgccactgaagctggcgtcatggttgctaacgcaccgacctctaatattcactccgcttgtgagcacgcaatttctttgctgctgtctactgctcgccagatccctgctgctgatgcgacgctgcgtgagggcgagtggaagcggtcttctttcaacggtgtggaaattttcggaaaaactgtcggtatcgtcggttttggccacattggtcagttgtttgctcagcgtcttgctgcgtttgagaccaccattgttgcttacgatccttacgctaaccctgctcgtgcggctcagctgaacgttgagttggttgagttggatgagctgatgagccgttctgactttgtcaccattcaccttcctaagaccaaggaaactgctggcatgtttgatgcgcagctccttgctaagtccaagaagggccagatcatcatcaacgctgctcgtggtggccttgttgatgagcaggctttggctgatgcgattgagtccggtcacattcgtggcgctggtttcgatgtgtactccaccgagccttgcactgattctcctttgttcaagttgcctcaggttgttgtgactcctcacttgggtgggtctactgaagaggctcaggatcgtgcgggtactgacgttgctgattctgtgctcaaggcgctggctggcgagttcgtggcggatgctgtgaacgtttccggtggtcgcgtgggcgaagaggttgctgtgtggatggatctggctcgcaagcttggtcttcttgctggcaagcttgtcgacgccgccccagtctccattgaggttgaggctcgaggcgagctttcttccgagcaggtcgatgcacttggtttgtccgctgttcgtggtttgttctccggaattatcgaagagtccgttactttcgtcaacgctcctcgcattgctgaagagcgtggcctggacatctccgtgaagaccaactctgagtctgttactcaccgttccgtcctgcaggtcaaggtcattactggcagcggcgcgagcgcaactgttgttggtgccctgactggtcttgagcgcgttgagaagatcacccgcatcaatggccgtggcctggatctgcgcgcagagggtctgaacctcttcctgcaggccactgacgctcctggtgcactgggtaccgttggtaccaagctgggtgctgctggcatcaacatcgaggctgctgcgttgactcaggctgagaagggtgacggcgctgtcctgatcctgcgtgttgagtccgctgtctctgaagagctggaagctgaaatcaacgctgagttgggtgctacttccttccaggttgatcttgactaataaagcttggttgataaaagaaggagactacactatggctcagtcttcaattttagttctggtccggcaatgctaccggcagaggtgcttaaacaggctcaacaggaactgcgcgactggaacggtcttggtacgtcggtgatggaagtgagtcaccgtggcaaagagttcattcaggttgcagaggaagccgagaaggattttcgcgatcttcttaatgtcccctccaactacaaggtattattctgccatggcggtggtcgcggtcagtttgctgcggtaccgctgaatattctcggtgataaaaccaccgcagattatgttgatgccggttactgggcggcaagtgccattaaagaagcgaaaaaatactgcacgcctaatgtctttgacgccaaagtgactgttgatggtctgcgcgcggttaagccaatgcgtgaatggcaactctctgataatgctgcttatatgcattattgcccgaatgaaaccatcgatggtatcgccatcgacgaaacgccagacttcggcgcagatgtggtggtcgccgctgacttctcttcaaccattctttcccgtccgattgacgtcagccgttatggtgtaatttacgctggcgcgcagaaaaatatcggcccggctggcctgacaatcgtcatcgttcgtgaagatttgctgggcaaagcgaatatcgcgtgtccgtcgattctggattattccatcctcaacgataacggctccatgtttaacacgccgccgacatttgcctggtatctatctggtctggtctttaaatggctgaaagcgaacggcggtgtagctgaaatggataaaatcaatcagcaaaaagcagaactgctatatggggtgattgataacagcgatttctaccgcaatgacgtggcgaaagctaaccgttcgcggatgaacgtgccgttccagttggcggacagtgcgcttgacaaattgttccttgaagagtcttttgctgctggccttcatgcactgaaaggtcaccgtgtggtcggcggaatgcgcgcttctatttataacgccatgccgctggaaggcgttaaagcgctgacagacttcatggttgagttcgaacgccgtcacggttgataaaagaaggagaccagtttatgcctaacattacctggtgcgacctgcctgaagatgtctctttatggccgggtctgcctctttcattaagtggtgatgaagtgatgccactggattaccacgcaggtcgtagcggctggctgctgtatggtcgtgggctggataaacaacgtctgacccaataccagagcaaactgggtgcggcgatggtgattgttgccgcctggtgcgtggaagattatcaggtgattcgtctggcaggttcactcaccgcacgggctacacgcctggcccacgaagcgcagctggatgtcgccccgctggggaaaatcccgcacctgcgcacgccgggtttgctggtgatggatatggactccaccgccatccagattgaatgtattgatgaaattgccaaactggccggaacgggcgagatggtggcggaagtaaccgaacgggcgatgcgcggcgaactcgattttaccgccagcctgcgcagccgtgtggcgacgctgaaaggcgctgacgccaatattctgcaacaggtgcgtgaaaatctgccgctgatgccaggcttaacgcaactggtgctcaagctggaaacgctgggctggaaagtggcgattgcctccggcggctttactttctttgctgaatacctgcgcgacaagctgcgcctgaccgccgtggtagccaatgaactggagatcatggacggtaaatttaccggcaatgtgatcggcgacatcgtagacgcgcagtacaaagcgaaaactctgactcgcctcgcgcaggagtatgaaatcccgctggcgcagaccgtggcgattggcgatggagccaatgacctgccgatgatcaaagcggcagggctggggattgcctaccatgccaagccaaaagtgaatgaaaaggcggaagtcaccatccgtcacgctgacctgatgggggtattctgcatcctctcaggcagcctgaatcagaagtgataagctgaggtcgcctcagcggccggcccctgcaggcgccggcgactagtcttggactcctgttgatagatccagtaatgacctcagaactccatctggatttgttcagaacgctcggttgccgccgggcgttttttattggtgagaatccaggggtccccaataattacgatttaaatttgtgtctcaaaatctctgatgttacattgcacaagataaaaatatatcatcatgaacaataaaactgtctgcttacataaacagtaatacaaggggtgttatgagccatattcagcgtgaaacgagctgtagccgtccgcgtctgaacagcaacatggatgcggatctgtatggctataaatgggcgcgtgataacgtgggtcagagcggcgcgaccatttatcgtctgtatggcaaaccggatgcgccggaactgtttctgaaacatggcaaaggcagcgtggcgaacgatgtgaccgatgaaatggtgcgtctgaactggctgaccgaatttatgccgctgccgaccattaaacattttattcgcaccccggatgatgcgtggctgctgaccaccgcgattccgggcaaaaccgcgtttcaggtgctggaagaatatccggatagcggcgaaaacattgtggatgcgctggccgtgtttctgcgtcgtctgcatagcattccggtgtgcaactgcccgtttaacagcgatcgtgtgtttcgtctggcccaggcgcagagccgtatgaacaacggcctggtggatgcgagcgattttgatgatgaacgtaacggctggccggtggaacaggtgtggaaagaaatgcataaactgctgccgtttagcccggatagcgtggtgacccacggcgattttagcctggataacctgattttcgatgaaggcaaactgattggctgcattgatgtgggccgtgtgggcattgcggatcgttatcaggatctggccattctgtggaactgcctgggcgaatttagcccgagcctgcaaaaacgtctgtttcagaaatatggcattgataatccggatatgaacaaactgcaatttcatctgatgctggatgaatttttctaataattaattggaccgttgtccttttccgctgcataaccctgcttcggggtcattatagcgattttttcggtatatccatcctttttcgcacgatatacaggattttgccaaagggttcgtgtagactttccttggtgtatccaacggcgtcagccgggcaggataggtgaagtaggcccacccgcgagcgggtgttccttcttcactgtccct

SEQ ID NO: 145 - DNA, 15 bp, synthetic construct
  source 1..15: mol_type = other DNA
aactttatgagccag

SEQ ID NO: 146 - DNA, 15 bp, synthetic construct
  source 1..15: mol_type = other DNA
ggatacatgtcccaa

SEQ ID NO: 147 - DNA, 15 bp, synthetic construct
  source 1..15: mol_type = other DNA
catgttatgagtcag

SEQ ID NO: 148 - DNA, 15 bp, synthetic construct
  source 1..15: mol_type = other DNA
ctgttcatgtctcag

SEQ ID NO: 149 - DNA, 15 bp, synthetic construct
  source 1..15: mol_type = other DNA
ggatacatgtcccaa

SEQ ID NO: 150 - DNA, 15 bp, synthetic construct
  source 1..15: mol_type = other DNA
ggttttatgagccaa

SEQ ID NO: 151 - DNA, 15 bp, synthetic construct
  source 1..15: mol_type = other DNA
cgccttatgtctcag

SEQ ID NO: 152 - DNA, 15 bp, synthetic construct
  source 1..15: mol_type = other DNA
ttcgaaatgtcgcaa

SEQ ID NO: 153 - DNA, 15 bp, synthetic construct
  source 1..15: mol_type = other DNA
tgagacatgtctcag

SEQ ID NO: 154 - DNA, 15 bp, synthetic construct
  source 1..15: mol_type = other DNA
tgtgacatgagtcag

SEQ ID NO: 155 - DNA, 15 bp, synthetic construct
  source 1..15: mol_type = other DNA
gattcgatgtcgcag

SEQ ID NO: 156 - DNA, 15 bp, synthetic construct
  source 1..15: mol_type = other DNA
ataattatgagtcag

SEQ ID NO: 157 - DNA, 15 bp, synthetic construct
  source 1..15: mol_type = other DNA
cgccttatgtctcaa

SEQ ID NO: 158 - DNA, 15 bp, synthetic construct
  source 1..15: mol_type = other DNA
cagtttatggctcaa

SEQ ID NO: 159 - DNA, 15 bp, synthetic construct
  source 1..15: mol_type = other DNA
cccggaatggcacaa

SEQ ID NO: 160 - DNA, 15 bp, synthetic construct
  source 1..15: mol_type = other DNA
tttgatatggcgcaa

SEQ ID NO: 161 - DNA, 15 bp, synthetic construct
  source 1..15: mol_type = other DNA
acccaaatggcccaa

SEQ ID NO: 162 - DNA, 15 bp, synthetic construct
  source 1..15: mol_type = other DNA
cccggaatggcacaa

SEQ ID NO: 163 - DNA, 15 bp, synthetic construct
  source 1..15: mol_type = other DNA
ttccacatggcccaa

SEQ ID NO: 164 - DNA, 15 bp, synthetic construct
  source 1..15: mol_type = other DNA
tacactatggctcag

SEQ ID NO: 165 - DNA, 15 bp, synthetic construct
  source 1..15: mol_type = other DNA
taccctatggcacag

SEQ ID NO: 166 - DNA, 15 bp, synthetic construct
  source 1..15: mol_type = other DNA
gacaccatggcacag

SEQ ID NO: 167 - DNA, 15 bp, synthetic construct
  source 1..15: mol_type = other DNA
ttgccgatggcgcaa

SEQ ID NO: 168 - DNA, 15 bp, synthetic construct
  source 1..15: mol_type = other DNA
cccactatggctcaa

SEQ ID NO: 169 - DNA, 15 bp, synthetic construct
  source 1..15: mol_type = other DNA
acatcaatggctcaa

SEQ ID NO: 170 - DNA, 15 bp, synthetic construct
  source 1..15: mol_type = other DNA
tacactatggctcag

SEQ ID NO: 171 - protein, 5 aa, Synthetic construct
GCFCI

SEQ ID NO: 172 - protein, 5 aa, synthetic construct
ARAGV

SEQ ID NO: 173 - DNA, 80 bp, synthetic construct
  source 1..80: mol_type = other DNA
gattnnnnnnatgagycaraatggccgtccggtagtcctcatcgccgataagcttgcgcagtccactgttgacgcgcttg

SEQ ID NO: 174 - DNA, 80 bp, synthetic construct
  source 1..80: mol_type = other DNA
ctaannnnnntactcrgtyttaccggcaggccatcaggagtagcggctattcgaacgcgtcaggtgacaactgcgcgaac

SEQ ID NO: 175 - DNA, 80 bp, synthetic construct
  source 1..80: mol_type = other DNA
taataaagcttggttgataaaagaaggagacnnnnnnatggcncaratcttcaattttagttctggtccggcaatgctac

SEQ ID NO: 176 - DNA, 80 bp, synthetic construct
  source 1..80: mol_type = other DNA
attatttcgaaccaactattttcttcctctgnnnnnntaccgngtytagaagttaaaatcaagaccaggccgttacgatg